European Patent Specification EP 4 063 397 B1, published June 19, 2024. Title: Chimeric antigen receptors based on single-domain antibodies and methods of use thereof. Applicant: Legend Biotech Ireland Limited. Application Not Yet Assigned. The sequence listing filed with the application follows.

SEQUENCE LISTING (277 sequences)

SEQ ID NO: 1 - protein, 5 aa, Artificial Sequence
  CD19 single-domain antibody VHH CDR1
INRMG

SEQ ID NO: 2 - protein, 16 aa, Artificial Sequence
  CD19 single-domain antibody VHH CDR2
SITVRGITNYADSVKG

SEQ ID NO: 3 - protein, 9 aa, Artificial Sequence
  CD19 single-domain antibody VHH CDR3
VSSNRDPDY

SEQ ID NO: 4 - protein, 5 aa, Artificial Sequence
  CD20 single-domain antibody VHH CDR1
IGTMG

SEQ ID NO: 5 - protein, 17 aa, Artificial Sequence
  CD20 single-domain antibody VHH CDR2
AIRWSTGGTRYADSVKG

SEQ ID NO: 6 - protein, 20 aa, Artificial Sequence
  CD20 single-domain antibody VHH CDR3
DRLSLDLSGRYHYNPAVYDY

SEQ ID NO: 7 - protein, 11 aa, Artificial Sequence
  BCMA 269A37346 VHH CDR1
SGFTLDYYAIG

SEQ ID NO: 8 - protein, 11 aa, Artificial Sequence
  BCMA 269A37348 VHH CDR1
SGRTFSTYGMA

SEQ ID NO: 9 - protein, 8 aa, Artificial Sequence
  BCMA 269A37917 VHH CDR1
SGRTFTMG

SEQ ID NO: 10 - protein, 11 aa, Artificial Sequence
  BCMA 269A37355 VHH CDR1
SGGIFVINAMG

SEQ ID NO: 11 - protein, 11 aa, Artificial Sequence
  BCMA 269A37915 VHH CDR1
SGRTFSSIVMG

SEQ ID NO: 12 - protein, 11 aa, Artificial Sequence
  BCMA 269A37936 VHH CDR1
SGFTFDRAVIV

SEQ ID NO: 13 - protein, 11 aa, Artificial Sequence
  BCMA 269A37953 VHH CDR1
STYTVNSDVMG

SEQ ID NO: 14 - protein, 11 aa, Artificial Sequence
  BCMA 269A37965 VHH CDR1
SGATLTNDHMA

SEQ ID NO: 15 - protein, 11 aa, Artificial Sequence
  BCMA 269A37972 VHH CDR1
SGGTLSKNTVA

SEQ ID NO: 16 - protein, 11 aa, Artificial Sequence
  BCMA 269A37353 VHH CDR1
SEHTFSSHVMG

SEQ ID NO: 17 - protein, 11 aa, Artificial Sequence
  BCMA 269A37948 VHH CDR1
SGRAFSTYFMA

SEQ ID NO: 18 - protein, 17 aa, Artificial Sequence
  BCMA 269A37346 VHH CDR2
CISRSDGSTYYADSVKG

SEQ ID NO: 19 - protein, 19 aa, Artificial Sequence
  BCMA 269A37348 VHH CDR2
SKASMNYSGRTYYADSVKG

SEQ ID NO: 20 - protein, 17 aa, Artificial Sequence
  BCMA 269A37917 VHH CDR2
AISLSPTLAYYAESVKG

SEQ ID NO: 21 - protein, 16 aa, Artificial Sequence
  BCMA 269A37355 VHH CDR2
SIRGLGRTNYDDSVKG

SEQ ID NO: 22 - protein, 17 aa, Artificial Sequence
  BCMA 269A37915 VHH CDR2
AIMWNDGITYLQDSVKG

SEQ ID NO: 23 - protein, 17 aa, Artificial Sequence
  BCMA 269A37936 VHH CDR2
FIKPSDGTIYYIDSLKG

SEQ ID NO: 24 - protein, 17 aa, Artificial Sequence
  BCMA 269A37953 VHH CDR2
AIMWNDGITYLQDSVKG

SEQ ID NO: 25 - protein, 17 aa, Artificial Sequence
  BCMA 269A37965 VHH CDR2
AIDWSGRTTNYADPVEG

SEQ ID NO: 26 - protein, 17 aa, Artificial Sequence
  BCMA 269A37972 VHH CDR2
SITWDGRTTYYADSVKG

SEQ ID NO: 27 - protein, 17 aa, Artificial Sequence
  BCMA 269A37353 VHH CDR2
VIGWRDISTSYADSVKG

SEQ ID NO: 28 - protein, 17 aa, Artificial Sequence
  BCMA 269A37948 VHH CDR2
GIAWSGGSTAYADSVKG

SEQ ID NO: 29 - protein, 14 aa, Artificial Sequence
  BCMA 269A37346 VHH CDR3
AGADCSGYLRDYEF

SEQ ID NO: 30 - protein, 18 aa, Artificial Sequence
  BCMA 269A37348 VHH CDR3
AGTGCSTYGCFDAQIIDY

SEQ ID NO: 31 - protein, 13 aa, Artificial Sequence
  BCMA 269A37917 VHH CDR3
ADRKSVMSIRPDY

SEQ ID NO: 32 - protein, 13 aa, Artificial Sequence
  BCMA 269A37355 VHH CDR3
VYVTLLGGVNRDY

SEQ ID NO: 33 - protein, 11 aa, Artificial Sequence
  BCMA 269A37915 VHH CDR3
ASKGRYSEYEY

SEQ ID NO: 34 - protein, 17 aa, Artificial Sequence
  BCMA 269A37936 VHH CDR3
ASPEDWYTDWIDWSIYR

SEQ ID NO: 35 - protein, 11 aa, Artificial Sequence
  BCMA 269A37953 VHH CDR3
ASKGRYSEYEY

SEQ ID NO: 36 - protein, 12 aa, Artificial Sequence
  BCMA 269A37965 VHH CDR3
VLRAWISYDNDY

SEQ ID NO: 37 - protein, 12 aa, Artificial Sequence
  BCMA 269A37972 VHH CDR3
DLGKWPAGPADY

SEQ ID NO: 38 - protein, 11 aa, Artificial Sequence
  BCMA 269A37353 VHH CDR3
ARRIDAADFDS

SEQ ID NO: 39 - protein, 11 aa, Artificial Sequence
  BCMA 269A37948 VHH CDR3
SRGIEVEEFGA

SEQ ID NO: 40 - protein, 11 aa, Artificial Sequence
  CD38 38A37333 VHH CDR1
SGLTFSSYPMM

SEQ ID NO: 41 - protein, 11 aa, Artificial Sequence
  CD38 38A37336 VHH CDR1
SGFTFSSNWMY

SEQ ID NO: 42 - protein, 11 aa, Artificial Sequence
  CD38 38A37699 VHH CDR1
SGRIFSINAMG

SEQ ID NO: 43 - protein, 14 aa, Artificial Sequence
  CD38 38A37331 VHH CDR1
SGSIFKVFRVFAMS

SEQ ID NO: 44 - protein, 11 aa, Artificial Sequence
  CD38 38A37717 VHH CDR1
TGKVFSIYDMG

SEQ ID NO: 45 - protein, 11 aa, Artificial Sequence
  CD38 38A37719 VHH CDR1
SASIFTRLPMG

SEQ ID NO: 46 - protein, 9 aa, Artificial Sequence
  CD38 38A37330 VHH CDR1
SGRAYATMA

SEQ ID NO: 47 - protein, 11 aa, Artificial Sequence
  CD38 38A37334 VHH CDR1
SGLTFSSYIMG

SEQ ID NO: 48 - protein, 11 aa, Artificial Sequence
  CD38 38A37730 VHH CDR1
SQGIFTINAMG

SEQ ID NO: 49 - protein, 11 aa, Artificial Sequence
  CD38 38A37340 VHH CDR1
SGRTFSSYAMA

SEQ ID NO: 50 - protein, 11 aa, Artificial Sequence
  CD38 38A37731 VHH CDR1
SGTIVSISTMG

SEQ ID NO: 51 - protein, 8 aa, Artificial Sequence
  CD38 38A37326 VHH CDR1
SGRTYAMG

SEQ ID NO: 52 - protein, 17 aa, Artificial Sequence
  CD38 38A37333 VHH CDR2
RISDSGGYTNYDDSVKG

SEQ ID NO: 53 - protein, 17 aa, Artificial Sequence
  CD38 38A37336 VHH CDR2
TISTDGRGTYYKDSVKG

SEQ ID NO: 54 - protein, 16 aa, Artificial Sequence
  CD38 38A37699 VHH CDR2
AISTAGSTNYGDSVKG

SEQ ID NO: 55 - protein, 16 aa, Artificial Sequence
  CD38 38A37331 VHH CDR2
SISSGETTTYADSVKG

SEQ ID NO: 56 - protein, 16 aa, Artificial Sequence
  CD38 38A37717 VHH CDR2
EITSSGTTHYDDFVSG

SEQ ID NO: 57 - protein, 16 aa, Artificial Sequence
  CD38 38A37719 VHH CDR2
GIVPSGRINYADSVKG

SEQ ID NO: 58 - protein, 17 aa, Artificial Sequence
  CD38 38A37330 VHH CDR2
HLRVSGDTTYYTDSVKG

SEQ ID NO: 59 - protein, 16 aa, Artificial Sequence
  CD38 38A37334 VHH CDR2
EISSGGMTSYADSVKG

SEQ ID NO: 60 - protein, 16 aa, Artificial Sequence
  CD38 38A37730 VHH CDR2
EVSSGGRTDYADSVKG

SEQ ID NO: 61 - protein, 17 aa, Artificial Sequence
  CD38 38A37340 VHH CDR2
SISTSGGITDYADSVKG

SEQ ID NO: 62 - protein, 16 aa, Artificial Sequence
  CD38 38A37731 VHH CDR2
TITRRGRTNYTDSVKG

SEQ ID NO: 63 - protein, 16 aa, Artificial Sequence
  CD38 38A37326 VHH CDR2
TISGAGNTKYADSVKG

SEQ ID NO: 64 - protein, 6 aa, Artificial Sequence
  CD38 38A37333 VHH CDR3
ILGLPT

SEQ ID NO: 65 - protein, 18 aa, Artificial Sequence
  CD38 38A37336 VHH CDR3
KEPRVLMAYLRNLGDFGS

SEQ ID NO: 66 - protein, 8 aa, Artificial Sequence
  CD38 38A37699 VHH CDR3
LNFPPYVY

SEQ ID NO: 67 - protein, 9 aa, Artificial Sequence
  CD38 38A37331 VHH CDR3
ADHTFTGDF

SEQ ID NO: 68 - protein, 8 aa, Artificial Sequence
  CD38 38A37717 VHH CDR3
NHVFGGSY

SEQ ID NO: 69 - protein, 8 aa, Artificial Sequence
  CD38 38A37719 VHH CDR3
ADTFPLPT

SEQ ID NO: 70 - protein, 19 aa, Artificial Sequence
  CD38 38A37330 VHH CDR3
GPYGILAAARVSNPGNYDY

SEQ ID NO: 71 - protein, 16 aa, Artificial Sequence
  CD38 38A37334 VHH CDR3
APERGSIWYSRYEYKY

SEQ ID NO: 72 - protein, 13 aa, Artificial Sequence
  CD38 38A37730 VHH CDR3
VSGWHVFVGDRIV

SEQ ID NO: 73 - protein, 14 aa, Artificial Sequence
  CD38 38A37340 VHH CDR3
ARTWYLRTSLQYDY

SEQ ID NO: 74 - protein, 14 aa, Artificial Sequence
  CD38 38A37731 VHH CDR3
AEVQLDIWASAYDY

SEQ ID NO: 75 - protein, 11 aa, Artificial Sequence
  CD38 38A37326 VHH CDR3
AGKWFPAANEY

SEQ ID NO: 76 - protein, 117 aa, Artificial Sequence
  CD19 single-domain antibody VHH
QVKLEESGGELVQPGGPLRLSCAASGNIFSINRMGWYRQAPGKQRAFVASITVRGITNYADSVKGRFTISVDKSKNTIYLQMNALKPEDTAVYYCNAVSSNRDPDYWGQGTQVTVSS

SEQ ID NO: 77 - protein, 129 aa, Artificial Sequence
  CD20 single-domain antibody VHH
PVQLVESGGGLVQAGDSLRLSCAASGRTFGIGTMGWFRQPPGKEREFVAAIRWSTGGTRYADSVKGRFTISRDNAKLTVDLQMDSLKPEDTAVYYCAADRLSLDLSGRYHYNPAVYDYWGQGTQVTVSS

SEQ ID NO: 78 - protein, 122 aa, Artificial Sequence
  BCMA 269A37346 VHH
QVQLVESGGGLVQPGGSLRLSCEASGFTLDYYAIGWFRQAPGKEREGVICISRSDGSTYYADSVKGRFTISRDNAKKTVYLQMISLKPEDTAAYYCAAGADCSGYLRDYEFRGQGTQVTVSS

SEQ ID NO: 79 - protein, 128 aa, Artificial Sequence
  BCMA 269A37348 VHH
QVKLEESGGRLVQPRGSLRLSCAGSGRTFSTYGMAWFRQAPGKEREFVASKASMNYSGRTYYADSVKGRFTIARDNAKNMVFLQMNNLKPEDTAVYYCAAGTGCSTYGCFDAQIIDYWGKGTLVTVSS

SEQ ID NO: 80 - protein, 118 aa, Artificial Sequence
  BCMA 269A37917 VHH
EVQLVESGGGLVQAGGSLRLSCAASGRTFTMGWFRQAPGKEREFVAAISLSPTLAYYAESVKGRFTISRDNAKNTVVLQMNSLKPEDTALYYCAADRKSVMSIRPDYWGQGTQVTVSS

SEQ ID NO: 81 - protein, 120 aa, Artificial Sequence
  BCMA 269A37355 VHH
AVQLVDSGGGLVQPGGSLRLSCVASGGIFVINAMGWYRQAPGKQRELVASIRGLGRTNYDDSVKGRFTISRDNANNTVYLQMNSLEPEDTAVYYCTVYVTLLGGVNRDYWGQGTQVTVSS

SEQ ID NO: 82 - protein, 119 aa, Artificial Sequence
  BCMA 269A37915 VHH
EVQLVESGGGLVQAGGSLRLSCAASGRTFSSIVMGWFRQAPGKEREFVGAIMWNDGITYLQDSVKGRFTIFRDNAKNTVYLQMNSLKLEDTAVYYCAASKGRYSEYEYWGQGTQVTVSS

SEQ ID NO: 83 - protein, 128 aa, Artificial Sequence
  BCMA 269A37936 VHH
EVQLVESGGGVVQAGGSLTVSCTASGFTFDRAVIVWFRQAPGKGREGVSFIKPSDGTIYYIDSLKGRFTISSDIAKNTVYLQMKSLESEDSAVYYCAASPEDWYTDWIDWSIYRWQHWGQGTQVTVSS

SEQ ID NO: 84 - protein, 119 aa, Artificial Sequence
  BCMA 269A37953 VHH
EVQLVESGGGMVQAGDSLRLSCVQSTYTVNSDVMGWFRQAPGKEREFVGAIMWNDGITYLQDSVKGRFTIFRDNAKNTVYLQMNSLKLEDTAVYYCAASKGRYSEYEYWGQGTQVTVSS

SEQ ID NO: 85 - protein, 120 aa, Artificial Sequence
  BCMA 269A37965 VHH
AVQLVESGGGLVQAGDSLRLSCTASGATLTNDHMAWFRQAPGKGREFVAAIDWSGRTTNYADPVEGRFTISRNNAKNTVYLEMNSLKLEDTAVYYCAVLRAWISYDNDYWGQGTQVTVSS

SEQ ID NO: 86 - protein, 120 aa, Artificial Sequence
  BCMA 269A37972 VHH
QVQLVESGGGLVQAGGSLRLSCAASGGTLSKNTVAWFRQAPGKERGFVASITWDGRTTYYADSVKGRFTISRDNAKNTVYLQMNSLKPEDTAVYVCADLGKWPAGPADYWGQGTQVTVSS

SEQ ID NO: 87 - protein, 119 aa, Artificial Sequence
  BCMA 269A37353 VHH
QVKLEESGGGLVQAGRSLRLSCAASEHTFSSHVMGWFRQAPGKERESVAVIGWRDISTSYADSVKGRFTISRDNAKKTLYLQMNSLKPEDTAVYYCAARRIDAADFDSWGQGTQVTVSS

SEQ ID NO: 88 - protein, 119 aa, Artificial Sequence
  BCMA 269A37948 VHH
AVQLVESGGGLVQAGDSLRLTCTASGRAFSTYFMAWFRQAPGKEREFVAGIAWSGGSTAYADSVKGRFTISRDNAKNTVYLQMNSLKSEDTAVYYCASRGIEVEEFGAWGQGTQVTVSS

SEQ ID NO: 89 - protein, 114 aa, Artificial Sequence
  CD38 38A37333 VHH
DVQLVESGGGLVQPGGSLRLSCVASGLTFSSYPMMWVRQAPGKGLEWVSRISDSGGYTNYDDSVKGRFTISRDNAKNTLYLQMNSLTPEDTAVYYCRILGLPTTGQGTQVTVSS

SEQ ID NO: 90 - protein, 126 aa, Artificial Sequence
  CD38 38A37336 VHH
EVQLVESGGGLVQPGGSLRLSCAASGFTFSSNWMYWVRQAPGKGLEWVATISTDGRGTYYKDSVKGRFTVSRDNAMSTLLLQMNNLKSEDTAVYYCAKEPRVLMAYLRNLGDFGSWGQGTQVTVSS

SEQ ID NO: 91 - protein, 115 aa, Artificial Sequence
  CD38 38A37699 VHH
QVQLVESGGGLVQAGGSLRLSCAASGRIFSINAMGWYRQAPGKQRELVAAISTAGSTNYGDSVKGRFTISRDNAKNTVYLQMNSLKPEDTAVYYCNLNFPPYVYWGQGTQVTVSS

SEQ ID NO: 92 - protein, 119 aa, Artificial Sequence
  CD38 38A37331 VHH
QVKLEESGGGLVQPGESLRLSCSASGSIFKVFRVFAMSWYRQGPGKQRELVASISSGETTTYADSVKGRFTISRDNAKNTAYLQMDSLKPEDTAVYYCNADHTFTGDFWGQGTQVTVSS

SEQ ID NO: 93 - protein, 116 aa, Artificial Sequence
  CD38 38A37717 VHH
EVQLVESGGGLVQAGGSLRLSCIATGKVFSIYDMGWYRQAPGKQRELVAEITSSGTTHYDDFVSGRFTISRDNAKNTVYLQMNTLKAEDTAVYYCRANHVFGGSYWGQGTQVTVSS

SEQ ID NO: 94 - protein, 115 aa, Artificial Sequence
  CD38 38A37719 VHH
QVKLEESGGGSVQTGGSLRLSCAASASIFTRLPMGWYRQAPGKQRELVVGIVPSGRINYADSVKGRFTISRDNAKNTVYLQMNSLRPEDTAVYYCRADTFPLPTWGQGTQVTVSS

SEQ ID NO: 95 - protein, 126 aa, Artificial Sequence
  CD38 38A37330 VHH
QVQLVESGGGLVQAGDSLRLSCAASGRAYATMAWFRQAPGKEREFVAHLRVSGDTTYYTDSVKGRFTISRDNAKNTAYLQMNMLKPEDTAVYYCAAGPYGILAAARVSNPGNYDYWGQGTQVTVSS

SEQ ID NO: 96 - protein, 123 aa, Artificial Sequence
  CD38 38A37334 VHH
EVQLVESGGGLVQAGGSLRLSCAASGLTFSSYIMGWFRQAPGEERELVAEISSGGMTSYADSVKGRFTISRDNAKKTGYLQMNSLKPEDTAVYYCAAPERGSIWYSRYEYKYWGQGTQVTVSS

SEQ ID NO: 97 - protein, 120 aa, Artificial Sequence
  CD38 38A37730 VHH
AVQLVDSGGGLAQTGGSLRLSCAASQGIFTINAMGWYRQVPGKQRELVAEVSSGGRTDYADSVKGRFTISRDNAKNTVYLQMNSLKPEDTGVYYCRVSGWHVFVGDRIVWGQGTLVTVSS

SEQ ID NO: 98 - protein, 123 aa, Artificial Sequence
  CD38 38A37340 VHH
DVQLVESGGGLVQAGDSLRLSCAASGRTFSSYAMAWFRQAPGKEREIVSSISTSGGITDYADSVKGRFTISKDSAKMNTVYLQMNSLEPEDTAVYYCAARTWYLRTSLQYDYWGQGTQVTVSS

SEQ ID NO: 99 - protein, 121 aa, Artificial Sequence
  CD38 38A37731 VHH
QVKLEESGGGLVQAGGSLRLSCVASGTIVSISTMGWYRQAPGKQRELVATITRRGRTNYTDSVKGRFTISRDNAKNTVYLQMNSLKPEDTAVYYCNAEVQLDIWASAYDYWGQGTQVTVAS

SEQ ID NO: 100 - protein, 115 aa, Artificial Sequence
  CD38 38A37326 VHH
EVQLVESGGGLVQAGGSLRLSCAASGRTYAMGWYRQAPGKQRDLVATISGAGNTKYADSVKGRFTISRDNAKNTMYLQMNSLKPEDTAVYYCAAGKWFPAANEYWGQGTQVTVSS

SEQ ID NO: 101 - DNA, 351 bp, Artificial Sequence
  CD19 single-domain antibody VHH
caggtaaagctggaggagtctgggggagaattggtgcagcctggggggcctctgagactctcctgtgcagcctcgggaaacatcttcagtatcaatcgcatgggctggtaccgccaggctccagggaagcagcgcgcgttcgtcgcatctattactgttcgtggtataacaaactatgcagactccgtgaagggccgattcaccatttctgtagacaagtccaaaaacacgatttatctgcagatgaacgcactcaaacctgaggacacggccgtctattattgtaatgcagtgtcttcaaacagggaccccgactactggggccaggggacccaggtcaccgtctcctca

SEQ ID NO: 102 - DNA, 387 bp, Artificial Sequence
  CD20 single-domain antibody VHH
ccggtgcagctggtggagtctgggggaggcttggtgcaggctggggattctctgagactctcctgtgctgcctctggacgcaccttcggtattggtaccatgggctggttccgccaacctccagggaaggagcgtgaatttgtagcagctattaggtggagtactggtggcactcgctatgcagactccgtgaagggccgattcaccatctcccgagacaacgccaagctcacggtagatctgcaaatggacagcctgaaacctgaagacacggccgtttattactgtgcagcagatagactgtcccttgatttaagtggtcgttaccactacaaccccgccgtgtatgactattggggccaggggacccaggtcaccgtctcctca

SEQ ID NO: 103 - DNA, 366 bp, Artificial Sequence
  BCMA 269A37346 VHH
caggtgcagctggtggagtctgggggaggcttggtgcagcctgggggttctctgaggctctcctgtgaagcctctggattcactttggattattatgccataggctggttccgccaggccccagggaaggagcgcgagggggtcatatgtattagtagaagtgatggtagcacatactatgcagactccgtgaagggccgattcaccatctccagagacaacgccaagaaaacggtgtatctgcaaatgatcagcctgaaacctgaggacacggccgcttattactgtgcagcaggggccgattgttcggggtacctacgagattatgagttccgggggcaggggacccaggtcaccgtctcctca

SEQ ID NO: 104 - DNA, 384 bp, Artificial Sequence
  BCMA 269A37348 VHH
caggtaaagctggaggagtctgggggacgattggtgcagccaaggggctctctgagactctcctgtgcaggctctggacgcactttcagtacctatggtatggcctggttccgccaggctccagggaaggagcgtgagttcgtagcgtctaaagcatcgatgaattacagcggtagaacatactatgcagactccgtgaagggccgattcaccatcgccagagacaacgccaagaacatggtgtttctgcaaatgaacaacctgaagcctgaggacacggccgtttattactgtgcagcgggcactggatgctcaacatatgggtgttttgacgcccagataatagactactggggcaaagggaccctggtcaccgtctcctca

SEQ ID NO: 105 - DNA, 354 bp, Artificial Sequence
  BCMA 269A37917 VHH
gaggtgcagctggtggagtctgggggaggcttggtgcaggctggggggtctctgagactctcctgtgcagcctctggacgcaccttcaccatggggtggttccgtcaggctccagggaaggagcgtgagtttgtagcagctattagtttgagtcctactttagcatattatgcagagtccgtgaagggccgattcaccatcagccgagacaacgccaagaacacggtggttttgcaaatgaacagcctgaaacctgaggacacggccctttattactgtgcagcagaccggaaatcagtaatgtctattcggcccgactactggggccaggggacccaggtcaccgtctcctca

SEQ ID NO: 106 - DNA, 360 bp, Artificial Sequence
  BCMA 269A37355 VHH
gccgtgcagctggtggattctgggggaggcttggtgcagcctggggggtctctgagactctcctgtgtagcctctggaggtatcttcgtcatcaatgccatgggctggtaccgccaggctccaggaaagcagcgcgagttggtcgcatctattcgtggactaggcagaacaaactatgacgactccgtgaagggccgattcaccatctccagagacaacgccaacaacacggtgtatctgcagatgaacagcctggaacctgaggacacggccgtctactactgtacagtctacgttacactacttggtggggttaatagggactactggggccaggggacccaggtcaccgtctcctca

SEQ ID NO: 107 - DNA, 357 bp, Artificial Sequence
  BCMA 269A37915 VHH
gaggtgcagctggtggagtctgggggaggattggtgcaggctgggggctctctgagactctcctgtgcagcctctggacggaccttcagtagcattgtcatgggctggttccgccaggctccagggaaggagcgtgagtttgtaggagcgattatgtggaatgatggtattacatacttgcaagactccgtgaagggccgatttaccatcttcagagacaatgccaagaacacggtgtatctgcaaatgaacagcctgaaacttgaggatacggccgtttattactgtgcagcatccaagggtagatactcggaatatgagtactggggccaggggacccaggtcaccgtctcctca

SEQ ID NO: 108 - DNA, 384 bp, Artificial Sequence
  BCMA 269A37936 VHH
gaggtgcagctggtggagtctgggggaggcgtggtgcaggctggggggtctctgacagtctcctgtacagcctctggattcactttcgaccgtgctgtcatagtctggttccgccaggcccccgggaagggccgtgagggggtctcatttattaaacctagtgatggcaccatatactacattgactccctgaagggccgattcacgatctccagtgacatcgccaagaatacggtatatctgcaaatgaaaagtctggaatcggaggactcggccgtttattactgtgcggcctcgcctgaggactggtacacggattggatcgactggagtatatatcggtggcagcactggggccaggggacccaggtcactgtctcctca

SEQ ID NO: 109 - DNA, 357 bp, Artificial Sequence
  BCMA 269A37953 VHH
gaggtgcagctggtggagtctgggggaggaatggtgcaggctggggactctctgagactatcctgtgtgcagtctacttacaccgtcaatagcgatgtcatgggctggttccgccaggctccagggaaggagcgtgagtttgtaggagcgattatgtggaatgatggtattacatacttgcaagactccgtgaagggccgatttaccatcttcagagacaacgccaagaacacggtgtatctgcaaatgaacagcctgaaacttgaggatacggccgtttattactgtgcagcatccaagggtagatactcggaatatgagtactggggccaggggacccaggtcaccgtctcctca

SEQ ID NO: 110 - DNA, 360 bp, Artificial Sequence
  BCMA 269A37965 VHH
gcggtgcagctggtggagtctgggggaggattggtgcaggctggggactctctgagactctcctgtacagcctctggtgcaaccttgactaacgatcacatggcatggttccgccaggctccagggaaggggcgtgaatttgtagcagctattgactggagtggtcgtaccacaaattacgcagaccccgtagagggccgattcaccatctccagaaacaacgccaagaacacggtgtatctggaaatgaacagcctgaaacttgaggacacggccgtttattactgtgcggtcctccgcgcttggatctcatatgacaatgactactggggccaggggacccaggtcaccgtctcctca

SEQ ID NO: 111 - DNA, 360 bp, Artificial Sequence
  BCMA 269A37972 VHH
caggtgcagctggtggagtctgggggaggattggtgcaggctgggggctctctgagactctcctgtgcagcctctggaggcaccttaagtaaaaataccgtggcttggttccgccaggctccagggaaggagcgtgggtttgtagcgtctattacctgggatggtcgtacgacatactatgcagactccgtgaagggccgattcaccatctccagagacaacgccaagaacacagtgtatctgcaaatgaacagcctgaaacctgaggatacggccgtttatgtctgtgcagacttagggaaatggcctgcgggcccggcggactactggggccaggggacccaggtcaccgtctcctca

SEQ ID NO: 112 - DNA, 357 bp, Artificial Sequence
  BCMA 269A37353 VHH
caggtaaagctggaggagtctgggggaggcttggtgcaggctgggcggtctctgagactctcctgtgcagcctctgaacacaccttcagtagccatgtcatgggctggttccgccaggctccagggaaggagcgtgagtctgttgcagttattggctggagagatattagcacaagctatgcagactccgtgaagggccgattcaccatctccagagacaacgccaagaagacgctgtatctgcaaatgaatagcctgaaacctgaggacacggccgtttactactgtgcagcacgtcggatcgacgcagctgactttgattcctgggggcaggggacccaggtcaccgtctcctcg

SEQ ID NO: 113 - DNA, 357 bp, Artificial Sequence
  BCMA 269A37948 VHH
gcggtgcagctggtggagtctgggggaggattggtgcaggctggggactctctgagactcacctgtacagcctctggacgcgccttcagtacctatttcatggcctggttccgccaggctccagggaaggagcgtgagtttgtagcaggaattgcatggagtggtggtagcacggcgtatgcagactccgtgaagggccgattcaccatctccagagacaacgccaagaacacggtgtatctgcaaatgaacagcctgaaatctgaggacacggccgtttattactgtgccagcagggggattgaggtcgaagagtttggtgcctggggccaggggacccaggtcaccgtctcgtcg

SEQ ID NO: 114 - DNA, 342 bp, Artificial Sequence
  CD38 38A37333 VHH
gatgtgcagctggtggagtctgggggaggcttggtgcagcctggggggtctctgagactctcctgtgtagcctctggattgaccttcagtagctaccccatgatgtgggtccgccaggctccaggaaaggggctcgagtgggtctcacgtattagcgatagtggtggttacacaaactatgacgactccgtgaagggccgattcaccatctccagagacaacgccaagaacacgctgtatctgcaaatgaacagcctgacacctgaggacacggccgtgtattactgtagaatcctggggttgcccaccacgggccaggggacccaggtcaccgtctcctca

SEQ ID NO: 115 - DNA, 378 bp, Artificial Sequence
  CD38 38A37336 VHH
gaggtgcagctggtggagtctgggggaggcctggtgcagcctggggggtctctgagactctcctgtgcagcctctggattcaccttcagtagcaactggatgtattgggtccgtcaggctccagggaaggggctcgagtgggtcgcaactattagtactgatggtcgtggaacatactataaagactctgtgaagggccgattcaccgtctccagagacaacgccatgagtacgctgcttctgcaaatgaacaatctgaaatctgaagatacggccgtgtattattgtgcaaaagagccgagggtgttgatggcttacctgcggaacctgggtgactttggttcctggggccaggggacccaggtcaccgtctcctcg

SEQ ID NO: 116 - DNA, 345 bp, Artificial Sequence
  CD38 38A37699 VHH
caggtgcagctggtggagtctgggggaggcttggtgcaggctggggggtctctgagactctcctgtgcagcctctggaaggatcttcagtatcaatgccatgggctggtaccgccaggctccagggaagcagcgcgagttggtcgccgctattagtacggctggtagcacaaactatggagactccgtgaagggccgattcaccatctccagagacaacgccaagaacacggtgtatctgcaaatgaacagcctgaaacctgaggacacagctgtttattactgtaatttaaattttcccccgtatgtgtactggggccaggggacccaggtcaccgtctcctca

SEQ ID NO: 117 - DNA, 357 bp, Artificial Sequence
  CD38 38A37331 VHH
caggtaaagctggaggagtctgggggaggtctggtgcagcctggggagtctctgagactctcctgttcagcctctggaagcatcttcaaagttttcagagtctttgccatgagctggtaccgccagggtcccgggaaacagcgcgagttggtcgcatccattagtagtggcgagaccacaacctatgcagactccgtgaagggccgattcaccatctccagagacaacgccaagaatacggcgtatctgcaaatggacagcctgaaacctgaggacacggccgtctattactgtaatgcggatcacacctttacaggagacttctggggccaggggacccaggtcaccgtctcctca

SEQ ID NO: 118 - DNA, 348 bp, Artificial Sequence
  CD38 38A37717 VHH
gaggtgcagctggtggaaagcggggggggactggtgcaggcaggcgggtcactgagactgtcatgtatcgcaactgggaaggtgtttagcatctacgacatgggctggtataggcaggcaccaggaaagcagagggagctggtggccgagatcaccagctccggcaccacacactacgacgatttcgtgtctggccggtttaccatcagcagagacaacgccaagaatacagtgtatctgcagatgaacaccctgaaggccgaggatacagccgtgtactattgccgggctaatcacgtcttcggcggctcctactgggggcagggaactcaggtcactgtgtcatcc

SEQ ID NO: 119 - DNA, 345 bp, Artificial Sequence
  CD38 38A37719 VHH
caggtaaagctggaggagtctgggggaggctcggtgcagactggggggtctctgagactctcctgtgcagcctctgcaagcatcttcactaggctgcccatgggctggtaccgccaggctccagggaagcagcgcgagttggtcgtaggcattgttcctagtggtaggataaactatgcagactccgtgaagggccgattcaccatctccagagacaacgccaagaacacggtgtatctgcaaatgaacagcctgcgccctgaggacacagccgtctattactgccgcgccgataccttccccttgcccacctggggccaggggacccaggtcaccgtctcctca

SEQ ID NO: 120 - DNA, 378 bp, Artificial Sequence
  CD38 38A37330 VHH
caggtgcagctggtggagtctgggggaggattggtgcaggctggggactctctgagactctcctgtgcagcctctggacgcgcctacgctacgatggcctggttccgccaggctccagggaaggagcgtgagtttgtagcacatctgcgcgtgagtggtgataccacttactatacagactccgtgaagggccgattcaccatctccagagacaacgccaagaacacggcgtatctgcaaatgaacatgttgaaacctgaggacacggccgtttattactgtgcagcgggaccgtatggcattcttgccgctgccagggtcagtaatccaggaaattatgattattggggccaggggacccaggtcaccgtctcctca

SEQ ID NO: 121 - DNA, 369 bp, Artificial Sequence
  CD38 38A37334 VHH
gaggtgcagctggtggagtctgggggaggattggtgcaggctgggggctctctgagactctcctgtgcagcctctggactcaccttcagtagttatattatgggctggttccgccaggctccaggcgaggagcgcgagttggtcgcggaaattagtagcggtggtatgacatcgtatgcagactccgtgaagggccgattcaccatctccagagacaacgccaagaagacggggtatctgcaaatgaacagcctgaaacctgaggacacggccgtttactattgtgcagcccctgagaggggtagtatctggtacagccgctacgaatataagtactggggccaggggacccaggtcaccgtctcctca

SEQ ID NO: 122 - DNA, 360 bp, Artificial Sequence
  CD38 38A37730 VHH
gccgtgcagctggtggattctgggggaggcttggcgcagactggggggtctctgagactctcctgtgcagcctctcaagggatcttcactatcaatgccatgggctggtaccgccaggttccagggaagcagcgggagttggtcgcagaagttagtagtggtggccgcacagactatgcagactccgtgaagggccgattcaccatctccagagacaacgccaagaacacggtgtacctgcaaatgaacagcctgaaacctgaggacacaggcgtctattattgtcgagtttctggatggcatgtgtttgtcggtgaccgcatagtttggggccagggcaccctggtcactgtctcctca

SEQ ID NO: 123 - DNA, 369 bp, Artificial Sequence
  CD38 38A37340 VHH
gatgtgcagctggtggagtctgggggaggattggtgcaggctggggactctctgagactctcctgtgcagcctctggacgcaccttcagtagctatgccatggcctggttccgccaggctccagggaaggagcgtgagattgtttcgtctatcagtaccagtggtggtatcacagactatgcagactccgtgaagggccgattcaccatctccaaagacagcgcgaagatgaacacggtgtatctgcaaatgaatagcctagaacctgaggacacggccgtttactactgtgcggcccgtacatggtaccttcgtacttctctccaatatgactattggggccaggggacccaggtcaccgtctcctca

SEQ ID NO: 124 - DNA, 363 bp, Artificial Sequence
  CD38 38A37731 VHH
caggtaaagctggaggagtctgggggaggcttggtgcaggctggggggtctctgagactctcctgtgtagcctctggaaccatcgtcagtatcagtaccatgggctggtaccgccaggctccagggaagcagcgcgagttggtcgcgactataaccaggcgtggacgcacgaactatacagactccgtgaagggccgattcaccatctccagagacaacgccaaaaacacggtgtatctgcaaatgaacagcctgaaacctgaggacacagccgtctattactgtaatgcagaggtgcaactggatatatgggcatctgcgtatgactactggggccaggggacccaggtcaccgtcgcctca

SEQ ID NO: 125 - DNA, 345 bp, Artificial Sequence
  CD38 38A37326 VHH
gaggtgcagctggtggagtctgggggaggattggtgcaggctgggggctctctgagactctcctgtgcagcctctggacgcacctatgccatgggctggtatcgccaggctccagggaagcagcgcgacttggtcgcaactattagtggtgcgggtaacacaaagtatgcagactccgtgaagggccgattcaccatctccagagacaacgccaagaacacaatgtatctgcaaatgaacagcctgaaacctgaggacacggccgtttattactgtgccgcgggtaaatggttccctgctgcgaatgagtactggggccaggggacccaggtcaccgtctcctca

SEQ ID NO: 126 - DNA, 9 bp, Artificial Sequence
  Kozak nucleic acid sequence
gccgccacc

SEQ ID NO: 127 - protein, 21 aa, Artificial Sequence
  CD8alpha signal peptide
MALPVTALLLPLALLLHAARP

SEQ ID NO: 128 - DNA, 63 bp, Artificial Sequence
  CD8alpha signal peptide nucleic acid sequence 1
atggccttaccagtgaccgccttgctcctgccgctggccttgctgctccacgccgccaggccg

SEQ ID NO: 129 - DNA, 63 bp, Artificial Sequence
  CD8alpha signal peptide nucleic acid sequence 2
atggctctgcccgtcactgctctgctgctgcccctggctctgctgctgcacgccgcaagaccc

SEQ ID NO: 130 - protein, 45 aa, Artificial Sequence
  CD8alpha hinge
TTTPAPRPPTPAPTIASQPLSLRPEACRPAAGGAVHTRGLDFACD

SEQ ID NO: 131 - DNA, 135 bp, Artificial Sequence
  CD8alpha hinge
accacgacgccagcgccgcgaccaccaacaccggcgcccaccatcgcgtcgcagcccctgtccctgcgcccagaggcgtgccggccagcggcggggggcgcagtgcacacgagggggctggacttcgcctgtgat

SEQ ID NO: 132 - protein, 24 aa, Artificial Sequence
  CD8alpha transmembrane
IYIWAPLAGTCGVLLLSLVITLYC

SEQ ID NO: 133 - protein, 27 aa, Artificial Sequence
  CD28 transmembrane
FWVLVVVGGVLACYSLLVTVAFIIFWV

SEQ ID NO: 134 - DNA, 72 bp, Artificial Sequence
  CD8alpha transmembrane
atctacatctgggcgcccttggccgggacttgtggggtccttctcctgtcactggttatcaccctttactgc

SEQ ID NO: 135 - DNA, 81 bp, Artificial Sequence
  CD28 transmembrane
ttttgggtgctggtggtggttggtggagtcctggcttgctatagcttgctagtaacagtggcctttattattttctgggtg

SEQ ID NO: 136 - protein, 41 aa, Artificial Sequence
  CD28 cytoplasmic aa sequence
RSKRSRLLHSDYMNMTPRRPGPTRKHYQPYAPPRDFAAYRS

SEQ ID NO: 137 - protein, 42 aa, Artificial Sequence
  CD137 cytoplasmic domain
KRGRKKLLYIFKQPFMRPVQTTQEEDGCSCRFPEEEEGGCEL

SEQ ID NO: 138 - DNA, 123 bp, Artificial Sequence
  CD28 cytoplasmic na sequence
aggagtaagaggagcaggctcctgcacagtgactacatgaacatgactccccgccgccccgggcccacccgcaagcattaccagccctatgccccaccacgcgacttcgcagcctatcgctcc

SEQ ID NO: 139 - DNA, 126 bp, Artificial Sequence
  CD137 cytoplasmic domain
aaacggggcagaaagaaactcctgtatatattcaaacaaccatttatgagaccagtacaaactactcaagaggaagatggctgtagctgccgatttccagaagaagaagaaggaggatgtgaactg

SEQ ID NO: 140 - protein, 113 aa, Artificial Sequence
  wt CD3z cytoplasmic domain
RVKFSRSADAPAYQQGQNQLYNELNLGRREEYDVLDKRRGRDPEMGGKPQRRKNPQEGLYNELQKDKMAEAYSEIGMKGERRRGKGHDGLYQGLSTATKDTYDALHMQALPPR

SEQ ID NO: 141 - protein, 113 aa, Artificial Sequence
  Q65K CD3z cytoplasmic domain
RVKFSRSADAPAYKQGQNQLYNELNLGRREEYDVLDKRRGRDPEMGGKPQRRKNPQEGLYNELQKDKMAEAYSEIGMKGERRRGKGHDGLYQGLSTATKDTYDALHMQALPPR

SEQ ID NO: 142 - DNA, 336 bp, Artificial Sequence
  wt CD3z cytoplasmic domain
agagtgaagttcagcaggagcgcagacgcccccgcgtaccagcagggccagaaccagctctataacgagctcaatctaggacgaagagaggagtacgatgttttggacaagagacgtggccgggaccctgagatggggggaaagccgagaaggaagaaccctcaggaaggcctgtacaatgaactgcagaaagataagatggcggaggcctacagtgagattgggatgaaaggcgagcgccggaggggcaaggggcacgatggcctttaccagggtctcagtacagccaccaaggacacctacgacgcccttcacatgcaggccctgccccctcgc

SEQ ID NO: 143 - DNA, 336 bp, Artificial Sequence
  Q65K CD3z cytoplasmic domain
agagtgaagttcagcaggagcgcagacgcccccgcgtacaagcagggccagaaccagctctataacgagctcaatctaggacgaagagaggagtacgatgttttggacaagagacgtggccgggaccctgagatggggggaaagccgagaaggaagaaccctcaggaaggcctgtacaatgaactgcagaaagataagatggcggaggcctacagtgagattgggatgaaaggcgagcgccggaggggcaaggggcacgatggcctttaccagggtctcagtacagccaccaaggacacctacgacgcccttcacatgcaggccctgccccctcgc

SEQ ID NO: 144 - protein, 5 aa, Artificial Sequence
  linker sequence 1
GGGGS

SEQ ID NO: 145 - protein, 10 aa, Artificial Sequence
  linker sequence 2
GGGGSGGGGS

SEQ ID NO: 146 - protein, 16 aa, Artificial Sequence
  linker sequence 3
GGGSGGGSGGGSGGGS

SEQ ID NO: 147 - protein, 24 aa, Artificial Sequence
  linker sequence 4
GGGGSGGGGSGGGGGGSGSGGGGS

SEQ ID NO: 148 - protein, 34 aa, Artificial Sequence
  linker sequence 5
GGGGSGGGGSGGGGGGSGSGGGGSGGGGSGGGGS

SEQ ID NO: 149 - protein, 15 aa, Artificial Sequence
  Linker sequence 6
GGGGSGGGGSGGGGS

SEQ ID NO: 150 - protein, 20 aa, Artificial Sequence
  Linker sequence 7
GGGGSGGGGSGGGGSGGGGS

SEQ ID NO: 151 - protein, 25 aa, Artificial Sequence
  Linker sequence 8
GGGGSGGGGSGGGGSGGGGSGGGGS

SEQ ID NO: 152 - protein, 420 aa, Artificial Sequence
  BCMA 269A37346 CAR
MALPVTALLLPLALLLHAARPVNRTRRMHQVQLVESGGGLVQPGGSLRLSCEASGFTLDYYAIGWFRQAPGKEREGVICISRSDGSTYYADSVKGRFTISRDNAKKTVYLQMISLKPEDTAAYYCAAGADCSGYLRDYEFRGQGTQVTVSSTSTTTPAPRPPTPAPTIASQPLSLRPEACRPAAGGAVHTRGLDFACDFWVLVVVGGVLACYSLLVTVAFIIFWVRSKRSRLLHSDYMNMTPRRPGPTRKHYQPYAPPRDFAAYRSKRGRKKLLYIFKQPFMRPVQTTQEEDGCSCRFPEEEEGGCELRVKFSRSADAPAYKQGQNQLYNELNLGRREEYDVLDKRRGRDPEMGGKPRRKNPQEGLYNELQKDKMAEAYSEIGMKGERRRGKGHDGLYQGLSTATKDTYDALHMQALPPR

SEQ ID NO: 153 - protein, 426 aa, Artificial Sequence
  BCMA 269A37348 CAR
MALPVTALLLPLALLLHAARPVNRTRRMHQVKLEESGGRLVQPRGSLRLSCAGSGRTFSTYGMAWFRQAPGKEREFVASKASMNYSGRTYYADSVKGRFTIARDNAKNMVFLQMNNLKPEDTAVYYCAAGTGCSTYGCFDAQIIDYWGKGTLVTVSSTSTTTPAPRPPTPAPTIASQPLSLRPEACRPAAGGAVHTRGLDFACDFWVLVVVGGVLACYSLLVTVAFIIFWVRSKRSRLLHSDYMNMTPRRPGPTRKHYQPYAPPRDFAAYRSKRGRKKLLYIFKQPFMRPVQTTQEEDGCSCRFPEEEEGGCELRVKFSRSADAPAYKQGQNQLYNELNLGRREEYDVLDKRRGRDPEMGGKPRRKNPQEGLYNELQKDKMAEAYSEIGMKGERRRGKGHDGLYQGLSTATKDTYDALHMQALPPR

SEQ ID NO: 154 - protein, 416 aa, Artificial Sequence
  BCMA 269A37917 CAR
MALPVTALLLPLALLLHAARPVNRTRRMHEVQLVESGGGLVQAGGSLRLSCAASGRTFTMGWFRQAPGKEREFVAAISLSPTLAYYAESVKGRFTISRDNAKNTVVLQMNSLKPEDTALYYCAADRKSVMSIRPDYWGQGTQVTVSSTSTTTPAPRPPTPAPTIASQPLSLRPEACRPAAGGAVHTRGLDFACDFWVLVVVGGVLACYSLLVTVAFIIFWVRSKRSRLLHSDYMNMTPRRPGPTRKHYQPYAPPRDFAAYRSKRGRKKLLYIFKQPFMRPVQTTQEEDGCSCRFPEEEEGGCELRVKFSRSADAPAYKQGQNQLYNELNLGRREEYDVLDKRRGRDPEMGGKPRRKNPQEGLYNELQKDKMAEAYSEIGMKGERRRGKGHDGLYQGLSTATKDTYDALHMQALPPR

SEQ ID NO: 155 - protein, 418 aa, Artificial Sequence
  BCMA 269A37355 CAR
MALPVTALLLPLALLLHAARPVNRTRRMHAVQLVDSGGGLVQPGGSLRLSCVASGGIFVINAMGWYRQAPGKQRELVASIRGLGRTNYDDSVKGRFTISRDNANNTVYLQMNSLEPEDTAVYYCTVYVTLLGGVNRDYWGQGTQVTVSSTSTTTPAPRPPTPAPTIASQPLSLRPEACRPAAGGAVHTRGLDFACDFWVLVVVGGVLACYSLLVTVAFIIFWVRSKRSRLLHSDYMNMTPRRPGPTRKHYQPYAPPRDFAAYRSKRGRKKLLYIFKQPFMRPVQTTQEEDGCSCRFPEEEEGGCELRVKFSRSADAPAYKQGQNQLYNELNLGRREEYDVLDKRRGRDPEMGGKPRRKNPQEGLYNELQKDKMAEAYSEIGMKGERRRGKGHDGLYQGLSTATKDTYDALHMQALPPR

SEQ ID NO: 156 - protein, 417 aa, Artificial Sequence
  BCMA 269A37915 CAR
MALPVTALLLPLALLLHAARPVNRTRRMHEVQLVESGGGLVQAGGSLRLSCAASGRTFSSIVMGWFRQAPGKEREFVGAIMWNDGITYLQDSVKGRFTIFRDNAKNTVYLQMNSLKLEDTAVYYCAASKGRYSEYEYWGQGTQVTVSSTSTTTPAPRPPTPAPTIASQPLSLRPEACRPAAGGAVHTRGLDFACDFWVLVVVGGVLACYSLLVTVAFIIFWVRSKRSRLLHSDYMNMTPRRPGPTRKHYQPYAPPRDFAAYRSKRGRKKLLYIFKQPFMRPVQTTQEEDGCSCRFPEEEEGGCELRVKFSRSADAPAYKQGQNQLYNELNLGRREEYDVLDKRRGRDPEMGGKPRRKNPQEGLYNELQKDKMAEAYSEIGMKGERRRGKGHDGLYQGLSTATKDTYDALHMQALPPR

SEQ ID NO: 157 - protein, 426 aa, Artificial Sequence
  BCMA 269A37936 CAR
MALPVTALLLPLALLLHAARPVNRTRRMHEVQLVESGGGVVQAGGSLTVSCTASGFTFDRAVIVWFRQAPGKGREGVSFIKPSDGTIYYIDSLKGRFTISSDIAKNTVYLQMKSLESEDSAVYYCAASPEDWYTDWIDWSIYRWQHWGQGTQVTVSSTSTTTPAPRPPTPAPTIASQPLSLRPEACRPAAGGAVHTRGLDFACDFWVLVVVGGVLACYSLLVTVAFIIFWVRSKRSRLLHSDYMNMTPRRPGPTRKHYQPYAPPRDFAAYRSKRGRKKLLYIFKQPFMRPVQTTQEEDGCSCRFPEEEEGGCELRVKFSRSADAPAYKQGQNQLYNELNLGRREEYDVLDKRRGRDPEMGGKPRRKNPQEGLYNELQKDKMAEAYSEIGMKGERRRGKGHDGLYQGLSTATKDTYDALHMQALPPR

SEQ ID NO: 158 - protein, 417 aa, Artificial Sequence
  BCMA 269A37953 CAR
MALPVTALLLPLALLLHAARPVNRTRRMHEVQLVESGGGMVQAGDSLRLSCVQSTYTVNSDVMGWFRQAPGKEREFVGAIMWNDGITYLQDSVKGRFTIFRDNAKNTVYLQMNSLKLEDTAVYYCAASKGRYSEYEYWGQGTQVTVSSTSTTTPAPRPPTPAPTIASQPLSLRPEACRPAAGGAVHTRGLDFACDFWVLVVVGGVLACYSLLVTVAFIIFWVRSKRSRLLHSDYMNMTPRRPGPTRKHYQPYAPPRDFAAYRSKRGRKKLLYIFKQPFMRPVQTTQEEDGCSCRFPEEEEGGCELRVKFSRSADAPAYKQGQNQLYNELNLGRREEYDVLDKRRGRDPEMGGKPRRKNPQEGLYNELQKDKMAEAYSEIGMKGERRRGKGHDGLYQGLSTATKDTYDALHMQALPPR

SEQ ID NO: 159 - protein, 418 aa, Artificial Sequence
  BCMA 269A37965 CAR
MALPVTALLLPLALLLHAARPVNRTRRMHAVQLVESGGGLVQAGDSLRLSCTASGATLTNDHMAWFRQAPGKGREFVAAIDWSGRTTNYADPVEGRFTISRNNAKNTVYLEMNSLKLEDTAVYYCAVLRAWISYDNDYWGQGTQVTVSSTSTTTPAPRPPTPAPTIASQPLSLRPEACRPAAGGAVHTRGLDFACDFWVLVVVGGVLACYSLLVTVAFIIFWVRSKRSRLLHSDYMNMTPRRPGPTRKHYQPYAPPRDFAAYRSKRGRKKLLYIFKQPFMRPVQTTQEEDGCSCRFPEEEEGGCELRVKFSRSADAPAYKQGQNQLYNELNLGRREEYDVLDKRRGRDPEMGGKPRRKNPQEGLYNELQKDKMAEAYSEIGMKGERRRGKGHDGLYQGLSTATKDTYDALHMQALPPR

SEQ ID NO: 160 - protein, 418 aa, Artificial Sequence
  BCMA 269A37972 CAR
MALPVTALLLPLALLLHAARPVNRTRRMHQVQLVESGGGLVQAGGSLRLSCAASGGTLSKNTVAWFRQAPGKERGFVASITWDGRTTYYADSVKGRFTISRDNAKNTVYLQMNSLKPEDTAVYVCADLGKWPAGPADYWGQGTQVTVSSTSTTTPAPRPPTPAPTIASQPLSLRPEACRPAAGGAVHTRGLDFACDFWVLVVVGGVLACYSLLVTVAFIIFWVRSKRSRLLHSDYMNMTPRRPGPTRKHYQPYAPPRDFAAYRSKRGRKKLLYIFKQPFMRPVQTTQEEDGCSCRFPEEEEGGCELRVKFSRSADAPAYKQGQNQLYNELNLGRREEYDVLDKRRGRDPEMGGKPRRKNPQEGLYNELQKDKMAEAYSEIGMKGERRRGKGHDGLYQGLSTATKDTYDALHMQALPPR

SEQ ID NO: 161 - protein, 417 aa, Artificial Sequence
  BCMA 269A37353 CAR
MALPVTALLLPLALLLHAARPVNRTRRMHQVKLEESGGGLVQAGRSLRLSCAASEHTFSSHVMGWFRQAPGKERESVAVIGWRDISTSYADSVKGRFTISRDNAKKTLYLQMNSLKPEDTAVYYCAARRIDAADFDSWGQGTQVTVSSTSTTTPAPRPPTPAPTIASQPLSLRPEACRPAAGGAVHTRGLDFACDFWVLVVVGGVLACYSLLVTVAFIIFWVRSKRSRLLHSDYMNMTPRRPGPTRKHYQPYAPPRDFAAYRSKRGRKKLLYIFKQPFMRPVQTTQEEDGCSCRFPEEEEGGCELRVKFSRSADAPAYKQGQNQLYNELNLGRREEYDVLDKRRGRDPEMGGKPRRKNPQEGLYNELQKDKMAEAYSEIGMKGERRRGKGHDGLYQGLSTATKDTYDALHMQALPPR

SEQ ID NO: 162 - protein, 417 aa, Artificial Sequence
  BCMA 269A37948 CAR
MALPVTALLLPLALLLHAARPVNRTRRMHAVQLVESGGGLVQAGDSLRLTCTASGRAFSTYFMAWFRQAPGKEREFVAGIAWSGGSTAYADSVKGRFTISRDNAKNTVYLQMNSLKSEDTAVYYCASRGIEVEEFGAWGQGTQVTVSSTSTTTPAPRPPTPAPTIASQPLSLRPEACRPAAGGAVHTRGLDFACDFWVLVVVGGVLACYSLLVTVAFIIFWVRSKRSRLLHSDYMNMTPRRPGPTRKHYQPYAPPRDFAAYRSKRGRKKLLYIFKQPFMRPVQTTQEEDGCSCRFPEEEEGGCELRVKFSRSADAPAYKQGQNQLYNELNLGRREEYDVLDKRRGRDPEMGGKPRRKNPQEGLYNELQKDKMAEAYSEIGMKGERRRGKGHDGLYQGLSTATKDTYDALHMQALPPR

SEQ ID NO: 163 - protein, 411 aa, Artificial Sequence
  CD38 38A37333 CAR
MALPVTALLLPLALLLHAARPVNDVQLVESGGGLVQPGGSLRLSCVASGLTFSSYPMMWVRQAPGKGLEWVSRISDSGGYTNYDDSVKGRFTISRDNAKNTLYLQMNSLTPEDTAVYYCRILGLPTTGQGTQVTVSSTRRMHTSTTTPAPRPPTPAPTIASQPLSLRPEACRPAAGGAVHTRGLDFACDFWVLVVVGGVLACYSLLVTVAFIIFWVRSKRSRLLHSDYMNMTPRRPGPTRKHYQPYAPPRDFAAYRSKRGRKKLLYIFKQPFMRPVQTTQEEDGCSCRFPEEEEGGCELRVKFSRSADAPAYKQGQNQLYNELNLGRREEYDVLDKRRGRDPEMGGKPRRKNPQEGLYNELQKDKMAEAYSEIGMKGERRRGKGHDGLYQGLSTATKDTYDALHMQALPPR

SEQ ID NO: 164 - protein, 423 aa, Artificial Sequence
  CD38 38A37336 CAR
MALPVTALLLPLALLLHAARPVNEVQLVESGGGLVQPGGSLRLSCAASGFTFSSNWMYWVRQAPGKGLEWVATISTDGRGTYYKDSVKGRFTVSRDNAMSTLLLQMNNLKSEDTAVYYCAKEPRVLMAYLRNLGDFGSWGQGTQVTVSSTRRMHTSTTTPAPRPPTPAPTIASQPLSLRPEACRPAAGGAVHTRGLDFACDFWVLVVVGGVLACYSLLVTVAFIIFWVRSKRSRLLHSDYMNMTPRRPGPTRKHYQPYAPPRDFAAYRSKRGRKKLLYIFKQPFMRPVQTTQEEDGCSCRFPEEEEGGCELRVKFSRSADAPAYKQGQNQLYNELNLGRREEYDVLDKRRGRDPEMGGKPRRKNPQEGLYNELQKDKMAEAYSEIGMKGERRRGKGHDGLYQGLSTATKDTYDALHMQALPPR

SEQ ID NO: 165 - protein, 412 aa, Artificial Sequence
  CD38 38A37699 CAR
MALPVTALLLPLALLLHAARPVNQVQLVESGGGLVQAGGSLRLSCAASGRIFSINAMGWYRQAPGKQRELVAAISTAGSTNYGDSVKGRFTISRDNAKNTVYLQMNSLKPEDTAVYYCNLNFPPYVYWGQGTQVTVSSTRRMHTSTTTPAPRPPTPAPTIASQPLSLRPEACRPAAGGAVHTRGLDFACDFWVLVVVGGVLACYSLLVTVAFIIFWVRSKRSRLLHSDYMNMTPRRPGPTRKHYQPYAPPRDFAAYRSKRGRKKLLYIFKQPFMRPVQTTQEEDGCSCRFPEEEEGGCELRVKFSRSADAPAYKQGQNQLYNELNLGRREEYDVLDKRRGRDPEMGGKPRRKNPQEGLYNELQKDKMAEAYSEIGMKGERRRGKGHDGLYQGLSTATKDTYDALHMQALPPR

SEQ ID NO: 166 - protein, 416 aa, Artificial Sequence
  CD38 38A37331 CAR
MALPVTALLLPLALLLHAARPVNQVKLEESGGGLVQPGESLRLSCSASGSIFKVFRVFAMSWYRQGPGKQRELVASISSGETTTYADSVKGRFTISRDNAKNTAYLQMDSLKPEDTAVYYCNADHTFTGDFWGQGTQVTVSSTRRMHTSTTTPAPRPPTPAPTIASQPLSLRPEACRPAAGGAVHTRGLDFACDFWVLVVVGGVLACYSLLVTVAFIIFWVRSKRSRLLHSDYMNMTPRRPGPTRKHYQPYAPPRDFAAYRSKRGRKKLLYIFKQPFMRPVQTTQEEDGCSCRFPEEEEGGCELRVKFSRSADAPAYKQGQNQLYNELNLGRREEYDVLDKRRGRDPEMGGKPRRKNPQEGLYNELQKDKMAEAYSEIGMKGERRRGKGHDGLYQGLSTATKDTYDALHMQALPPR

SEQ ID NO: 167 - protein, 413 aa, Artificial Sequence
  CD38 38A37717 CAR
MALPVTALLLPLALLLHAARPVNEVQLVESGGGLVQAGGSLRLSCIATGKVFSIYDMGWYRQAPGKQRELVAEITSSGTTHYDDFVSGRFTISRDNAKNTVYLQMNTLKAEDTAVYYCRANHVFGGSYWGQGTQVTVSSTRRMHTSTTTPAPRPPTPAPTIASQPLSLRPEACRPAAGGAVHTRGLDFACDFWVLVVVGGVLACYSLLVTVAFIIFWVRSKRSRLLHSDYMNMTPRRPGPTRKHYQPYAPPRDFAAYRSKRGRKKLLYIFKQPFMRPVQTTQEEDGCSCRFPEEEEGGCELRVKFSRSADAPAYKQGQNQLYNELNLGRREEYDVLDKRRGRDPEMGGKPRRKNPQEGLYNELQKDKMAEAYSEIGMKGERRRGKGHDGLYQGLSTATKDTYDALHMQALPPR

SEQ ID NO: 168 - protein, 412 aa, Artificial Sequence
  CD38 38A37719 CAR
MALPVTALLLPLALLLHAARPVNQVKLEESGGGSVQTGGSLRLSCAASASIFTRLPMGWYRQAPGKQRELVVGIVPSGRINYADSVKGRFTISRDNAKNTVYLQMNSLRPEDTAVYYCRADTFPLPTWGQGTQVTVSSTRRMHTSTTTPAPRPPTPAPTIASQPLSLRPEACRPAAGGAVHTRGLDFACDFWVLVVVGGVLACYSLLVTVAFIIFWVRSKRSRLLHSDYMNMTPRRPGPTRKHYQPYAPPRDFAAYRSKRGRKKLLYIFKQPFMRPVQTTQEEDGCSCRFPEEEEGGCELRVKFSRSADAPAYKQGQNQLYNELNLGRREEYDVLDKRRGRDPEMGGKPRRKNPQEGLYNELQKDKMAEAYSEIGMKGERRRGKGHDGLYQGLSTATKDTYDALHMQALPPR

SEQ ID NO: 169 - protein, 423 aa, Artificial Sequence
  CD38 38A37330 CAR
MALPVTALLLPLALLLHAARPVNQVQLVESGGGLVQAGDSLRLSCAASGRAYATMAWFRQAPGKEREFVAHLRVSGDTTYYTDSVKGRFTISRDNAKNTAYLQMNMLKPEDTAVYYCAAGPYGILAAARVSNPGNYDYWGQGTQVTVSSTRRMHTSTTTPAPRPPTPAPTIASQPLSLRPEACRPAAGGAVHTRGLDFACDFWVLVVVGGVLACYSLLVTVAFIIFWVRSKRSRLLHSDYMNMTPRRPGPTRKHYQPYAPPRDFAAYRSKRGRKKLLYIFKQPFMRPVQTTQEEDGCSCRFPEEEEGGCELRVKFSRSADAPAYKQGQNQLYNELNLGRREEYDVLDKRRGRDPEMGGKPRRKNPQEGLYNELQKDKMAEAYSEIGMKGERRRGKGHDGLYQGLSTATKDTYDALHMQALPPR

SEQ ID NO: 170 - protein, 420 aa, Artificial Sequence
  CD38 38A37334 CAR
MALPVTALLLPLALLLHAARPVNEVQLVESGGGLVQAGGSLRLSCAASGLTFSSYIMGWFRQAPGEERELVAEISSGGMTSYADSVKGRFTISRDNAKKTGYLQMNSLKPEDTAVYYCAAPERGSIWYSRYEYKYWGQGTQVTVSSTRRMHTSTTTPAPRPPTPAPTIASQPLSLRPEACRPAAGGAVHTRGLDFACDFWVLVVVGGVLACYSLLVTVAFIIFWVRSKRSRLLHSDYMNMTPRRPGPTRKHYQPYAPPRDFAAYRSKRGRKKLLYIFKQPFMRPVQTTQEEDGCSCRFPEEEEGGCELRVKFSRSADAPAYKQGQNQLYNELNLGRREEYDVLDKRRGRDPEMGGKPRRKNPQEGLYNELQKDKMAEAYSEIGMKGERRRGKGHDGLYQGLSTATKDTYDALHMQALPPR

SEQ ID NO: 171 - protein, 417 aa, Artificial Sequence
  CD38 38A37730 CAR
MALPVTALLLPLALLLHAARPVNAVQLVDSGGGLAQTGGSLRLSCAASQGIFTINAMGWYRQVPGKQRELVAEVSSGGRTDYADSVKGRFTISRDNAKNTVYLQMNSLKPEDTGVYYCRVSGWHVFVGDRIVWGQGTLVTVSSTRRMHTSTTTPAPRPPTPAPTIASQPLSLRPEACRPAAGGAVHTRGLDFACDFWVLVVVGGVLACYSLLVTVAFIIFWVRSKRSRLLHSDYMNMTPRRPGPTRKHYQPYAPPRDFAAYRSKRGRKKLLYIFKQPFMRPVQTTQEEDGCSCRFPEEEEGGCELRVKFSRSADAPAYKQGQNQLYNELNLGRREEYDVLDKRRGRDPEMGGKPRRKNPQEGLYNELQKDKMAEAYSEIGMKGERRRGKGHDGLYQGLSTATKDTYDALHMQALPPR

SEQ ID NO: 172 - protein, 420 aa, Artificial Sequence
  CD38 38A37340 CAR
MALPVTALLLPLALLLHAARPVNDVQLVESGGGLVQAGDSLRLSCAASGRTFSSYAMAWFRQAPGKEREIVSSISTSGGITDYADSVKGRFTISKDSAKMNTVYLQMNSLEPEDTAVYYCAARTWYLRTSLQYDYWGQGTQVTVSSTRRMHTSTTTPAPRPPTPAPTIASQPLSLRPEACRPAAGGAVHTRGLDFACDFWVLVVVGGVLACYSLLVTVAFIIFWVRSKRSRLLHSDYMNMTPRRPGPTRKHYQPYAPPRDFAAYRSKRGRKKLLYIFKQPFMRPVQTTQEEDGCSCRFPEEEEGGCELRVKFSRSADAPAYKQGQNQLYNELNLGRREEYDVLDKRRGRDPEMGGKPRRKNPQEGLYNELQKDKMAEAYSEIGMKGERRRGKGHDGLYQGLSTATKDTYDALHMQALPPR

SEQ ID NO: 173 - protein, 418 aa, Artificial Sequence
  CD38 38A37731 CAR
MALPVTALLLPLALLLHAARPVNQVKLEESGGGLVQAGGSLRLSCVASGTIVSISTMGWYRQAPGKQRELVATITRRGRTNYTDSVKGRFTISRDNAKNTVYLQMNSLKPEDTAVYYCNAEVQLDIWASAYDYWGQGTQVTVASTRRMHTSTTTPAPRPPTPAPTIASQPLSLRPEACRPAAGGAVHTRGLDFACDFWVLVVVGGVLACYSLLVTVAFIIFWVRSKRSRLLHSDYMNMTPRRPGPTRKHYQPYAPPRDFAAYRSKRGRKKLLYIFKQPFMRPVQTTQEEDGCSCRFPEEEEGGCELRVKFSRSADAPAYKQGQNQLYNELNLGRREEYDVLDKRRGRDPEMGGKPRRKNPQEGLYNELQKDKMAEAYSEIGMKGERRRGKGHDGLYQGLSTATKDTYDALHMQALPPR

SEQ ID NO: 174 - protein, 412 aa, Artificial Sequence
  CD38 38A37326 CAR
MALPVTALLLPLALLLHAARPVNEVQLVESGGGLVQAGGSLRLSCAASGRTYAMGWYRQAPGKQRDLVATISGAGNTKYADSVKGRFTISRDNAKNTMYLQMNSLKPEDTAVYYCAAGKWFPAANEYWGQGTQVTVSSTRRMHTSTTTPAPRPPTPAPTIASQPLSLRPEACRPAAGGAVHTRGLDFACDFWVLVVVGGVLACYSLLVTVAFIIFWVRSKRSRLLHSDYMNMTPRRPGPTRKHYQPYAPPRDFAAYRSKRGRKKLLYIFKQPFMRPVQTTQEEDGCSCRFPEEEEGGCELRVKFSRSADAPAYKQGQNQLYNELNLGRREEYDVLDKRRGRDPEMGGKPRRKNPQEGLYNELQKDKMAEAYSEIGMKGERRRGKGHDGLYQGLSTATKDTYDALHMQALPPR

SEQ ID NO: 175 - DNA, 1263 bp, Artificial Sequence
  BCMA 269A37346 CAR
atggccttaccagtgaccgccttgctcctgccgctggccttgctgctccacgccgccaggccggttaaccgcacgcgtcgcatgcatcaggtgcagctggtggagtctgggggaggcttggtgcagcctgggggttctctgaggctctcctgtgaagcctctggattcactttggattattatgccataggctggttccgccaggccccagggaaggagcgcgagggggtcatatgtattagtagaagtgatggtagcacatactatgcagactccgtgaagggccgattcaccatctccagagacaacgccaagaaaacggtgtatctgcaaatgatcagcctgaaacctgaggacacggccgcttattactgtgcagcaggggccgattgttcggggtacctacgagattatgagttccgggggcaggggacccaggtcaccgtctcctcaactagtaccacgacgccagcgccgcgaccaccaacaccggcgcccaccatcgcgtcgcagcccctgtccctgcgcccagaggcgtgccggccagcggcggggggcgcagtgcacacgagggggctggacttcgcctgtgatttttgggtgctggtggtggttggtggagtcctggcttgctatagcttgctagtaacagtggcctttattattttctgggtgaggagtaagaggagcaggctcctgcacagtgactacatgaacatgactccccgccgccccgggcccacccgcaagcattaccagccctatgccccaccacgcgacttcgcagcctatcgctccaaacggggcagaaagaaactcctgtatatattcaaacaaccatttatgagaccagtacaaactactcaagaggaagatggctgtagctgccgatttccagaagaagaagaaggaggatgtgaactgagagtgaagttcagcaggagcgcagacgcccccgcgtacaagcagggccagaaccagctctataacgagctcaatctaggacgaagagaggagtacgatgttttggacaagagacgtggccgggaccctgagatggggggaaagccgagaaggaagaaccctcaggaaggcctgtacaatgaactgcagaaagataagatggcggaggcctacagtgagattgggatgaaaggcgagcgccggaggggcaaggggcacgatggcctttaccagggtctcagtacagccaccaaggacacctacgacgcccttcacatgcaggccctgccccctcgctga

SEQ ID NO: 176 - DNA, 1281 bp, Artificial Sequence
  BCMA 269A37348 CAR
atggccttaccagtgaccgccttgctcctgccgctggccttgctgctccacgccgccaggccggttaaccgcacgcgtcgcatgcatcaggtaaagctggaggagtctgggggacgattggtgcagccaaggggctctctgagactctcctgtgcaggctctggacgcactttcagtacctatggtatggcctggttccgccaggctccagggaaggagcgtgagttcgtagcgtctaaagcatcgatgaattacagcggtagaacatactatgcagactccgtgaagggccgattcaccatcgccagagacaacgccaagaacatggtgtttctgcaaatgaacaacctgaagcctgaggacacggccgtttattactgtgcagcgggcactggatgctcaacatatgggtgttttgacgcccagataatagactactggggcaaagggaccctggtcaccgtctcctcaactagtaccacgacgccagcgccgcgaccaccaacaccggcgcccaccatcgcgtcgcagcccctgtccctgcgcccagaggcgtgccggccagcggcggggggcgcagtgcacacgagggggctggacttcgcctgtgatttttgggtgctggtggtggttggtggagtcctggcttgctatagcttgctagtaacagtggcctttattattttctgggtgaggagtaagaggagcaggctcctgcacagtgactacatgaacatgactccccgccgccccgggcccacccgcaagcattaccagccctatgccccaccacgcgacttcgcagcctatcgctccaaacggggcagaaagaaactcctgtatatattcaaacaaccatttatgagaccagtacaaactactcaagaggaagatggctgtagctgccgatttccagaagaagaagaaggaggatgtgaactgagagtgaagttcagcaggagcgcagacgcccccgcgtacaagcagggccagaaccagctctataacgagctcaatctaggacgaagagaggagtacgatgttttggacaagagacgtggccgggaccctgagatggggggaaagccgagaaggaagaaccctcaggaaggcctgtacaatgaactgcagaaagataagatggcggaggcctacagtgagattgggatgaaaggcgagcgccggaggggcaaggggcacgatggcctttaccagggtctcagtacagccaccaaggacacctacgacgcccttcacatgcaggccctgccccctcgctga

SEQ ID NO: 177 - DNA, 1251 bp, Artificial Sequence
  BCMA 269A37917 CAR
atggccttaccagtgaccgccttgctcctgccgctggccttgctgctccacgccgccaggccggttaaccgcacgcgtcgcatgcatgaggtgcagctggtggagtctgggggaggcttggtgcaggctggggggtctctgagactctcctgtgcagcctctggacgcaccttcaccatggggtggttccgtcaggctccagggaaggagcgtgagtttgtagcagctattagtttgagtcctactttagcatattatgcagagtccgtgaagggccgattcaccatcagccgagacaacgccaagaacacggtggttttgcaaatgaacagcctgaaacctgaggacacggccctttattactgtgcagcagaccggaaatcagtaatgtctattcggcccgactactggggccaggggacccaggtcaccgtctcctcaactagtaccacgacgccagcgccgcgaccaccaacaccggcgcccaccatcgcgtcgcagcccctgtccctgcgcccagaggcgtgccggccagcggcggggggcgcagtgcacacgagggggctggacttcgcctgtgatttttgggtgctggtggtggttggtggagtcctggcttgctatagcttgctagtaacagtggcctttattattttctgggtgaggagtaagaggagcaggctcctgcacagtgactacatgaacatgactccccgccgccccgggcccacccgcaagcattaccagccctatgccccaccacgcgacttcgcagcctatcgctccaaacggggcagaaagaaactcctgtatatattcaaacaaccatttatgagaccagtacaaactactcaagaggaagatggctgtagctgccgatttccagaagaagaagaaggaggatgtgaactgagagtgaagttcagcaggagcgcagacgcccccgcgtacaagcagggccagaaccagctctataacgagctcaatctaggacgaagagaggagtacgatgttttggacaagagacgtggccgggaccctgagatggggggaaagccgagaaggaagaaccctcaggaaggcctgtacaatgaactgcagaaagataagatggcggaggcctacagtgagattgggatgaaaggcgagcgccggaggggcaaggggcacgatggcctttaccagggtctcagtacagccaccaaggacacctacgacgcccttcacatgcaggccctgccccctcgctga

SEQ ID NO: 178 - DNA, 1257 bp, Artificial Sequence
  BCMA 269A37355 CAR
atggccttaccagtgaccgccttgctcctgccgctggccttgctgctccacgccgccaggccggttaaccgcacgcgtcgcatgcatgccgtgcagctggtggattctgggggaggcttggtgcagcctggggggtctctgagactctcctgtgtagcctctggaggtatcttcgtcatcaatgccatgggctggtaccgccaggctccaggaaagcagcgcgagttggtcgcatctattcgtggactaggcagaacaaactatgacgactccgtgaagggccgattcaccatctccagagacaacgccaacaacacggtgtatctgcagatgaacagcctggaacctgaggacacggccgtctactactgtacagtctacgttacactacttggtggggttaatagggactactggggccaggggacccaggtcaccgtctcctcaactagtaccacgacgccagcgccgcgaccaccaacaccggcgcccaccatcgcgtcgcagcccctgtccctgcgcccagaggcgtgccggccagcggcggggggcgcagtgcacacgagggggctggacttcgcctgtgatttttgggtgctggtggtggttggtggagtcctggcttgctatagcttgctagtaacagtggcctttattattttctgggtgaggagtaagaggagcaggctcctgcacagtgactacatgaacatgactccccgccgccccgggcccacccgcaagcattaccagccctatgccccaccacgcgacttcgcagcctatcgctccaaacggggcagaaagaaactcctgtatatattcaaacaaccatttatgagaccagtacaaactactcaagaggaagatggctgtagctgccgatttccagaagaagaagaaggaggatgtgaactgagagtgaagttcagcaggagcgcagacgcccccgcgtacaagcagggccagaaccagctctataacgagctcaatctaggacgaagagaggagtacgatgttttggacaagagacgtggccgggaccctgagatggggggaaagccgagaaggaagaaccctcaggaaggcctgtacaatgaactgcagaaagataagatggcggaggcctacagtgagattgggatgaaaggcgagcgccggaggggcaaggggcacgatggcctttaccagggtctcagtacagccaccaaggacacctacgacgcccttcacatgcaggccctgccccctcgctga

SEQ ID NO: 179 - DNA, 1254 bp, Artificial Sequence
  BCMA 269A37915 CAR
atggccttaccagtgaccgccttgctcctgccgctggccttgctgctccacgccgccaggccggttaaccgcacgcgtcgcatgcatgaggtgcagctggtggagtctgggggaggattggtgcaggctgggggctctctgagactctcctgtgcagcctctggacggaccttcagtagcattgtcatgggctggttccgccaggctccagggaaggagcgtgagtttgtaggagcgattatgtggaatgatggtattacatacttgcaagactccgtgaagggccgatttaccatcttcagagacaatgccaagaacacggtgtatctgcaaatgaacagcctgaaacttgaggatacggccgtttattactgtgcagcatccaagggtagatactcggaatatgagtactggggccaggggacccaggtcaccgtctcctcaactagtaccacgacgccagcgccgcgaccaccaacaccggcgcccaccatcgcgtcgcagcccctgtccctgcgcccagaggcgtgccggccagcggcggggggcgcagtgcacacgagggggctggacttcgcctgtgatttttgggtgctggtggtggttggtggagtcctggcttgctatagcttgctagtaacagtggcctttattattttctgggtgaggagtaagaggagcaggctcctgcacagtgactacatgaacatgactccccgccgccccgggcccacccgcaagcattaccagccctatgccccaccacgcgacttcgcagcctatcgctccaaacggggcagaaagaaactcctgtatatattcaaacaaccatttatgagaccagtacaaactactcaagaggaagatggctgtagctgccgatttccagaagaagaagaaggaggatgtgaactgagagtgaagttcagcaggagcgcagacgcccccgcgtacaagcagggccagaaccagctctataacgagctcaatctaggacgaagagaggagtacgatgttttggacaagagacgtggccgggaccctgagatggggggaaagccgagaaggaagaaccctcaggaaggcctgtacaatgaactgcagaaagataagatggcggaggcctacagtgagattgggatgaaaggcgagcgccggaggggcaaggggcacgatggcctttaccagggtctcagtacagccaccaaggacacctacgacgcccttcacatgcaggccctgccccctcgctga

SEQ ID NO: 180 - DNA, 1281 bp, Artificial Sequence
  BCMA 269A37936 CAR
atggccttaccagtgaccgccttgctcctgccgctggccttgctgctccacgccgccaggccggttaaccgcacgcgtcgcatgcatgaggtgcagctggtggagtctgggggaggcgtggtgcaggctggggggtctctgacagtctcctgtacagcctctggattcactttcgaccgtgctgtcatagtctggttccgccaggcccccgggaagggccgtgagggggtctcatttattaaacctagtgatggcaccatatactacattgactccctgaagggccgattcacgatctccagtgacatcgccaagaatacggtatatctgcaaatgaaaagtctggaatcggaggactcggccgtttattactgtgcggcctcgcctgaggactggtacacggattggatcgactggagtatatatcggtggcagcactggggccaggggacccaggtcactgtctcctcaactagtaccacgacgccagcgccgcgaccaccaacaccggcgcccaccatcgcgtcgcagcccctgtccctgcgcccagaggcgtgccggccagcggcggggggcgcagtgcacacgagggggctggacttcgcctgtgatttttgggtgctggtggtggttggtggagtcctggcttgctatagcttgctagtaacagtggcctttattattttctgggtgaggagtaagaggagcaggctcctgcacagtgactacatgaacatgactccccgccgccccgggcccacccgcaagcattaccagccctatgccccaccacgcgacttcgcagcctatcgctccaaacggggcagaaagaaactcctgtatatattcaaacaaccatttatgagaccagtacaaactactcaagaggaagatggctgtagctgccgatttccagaagaagaagaaggaggatgtgaactgagagtgaagttcagcaggagcgcagacgcccccgcgtacaagcagggccagaaccagctctataacgagctcaatctaggacgaagagaggagtacgatgttttggacaagagacgtggccgggaccctgagatggggggaaagccgagaaggaagaaccctcaggaaggcctgtacaatgaactgcagaaagataagatggcggaggcctacagtgagattgggatgaaaggcgagcgccggaggggcaaggggcacgatggcctttaccagggtctcagtacagccaccaaggacacctacgacgcccttcacatgcaggccctgccccctcgctga

SEQ ID NO: 181 - DNA, 1254 bp, Artificial Sequence
  BCMA 269A37953 CAR
atggccttaccagtgaccgccttgctcctgccgctggccttgctgctccacgccgccaggccggttaaccgcacgcgtcgcatgcatgaggtgcagctggtggagtctgggggaggaatggtgcaggctggggactctctgagactatcctgtgtgcagtctacttacaccgtcaatagcgatgtcatgggctggttccgccaggctccagggaaggagcgtgagtttgtaggagcgattatgtggaatgatggtattacatacttgcaagactccgtgaagggccgatttaccatcttcagagacaacgccaagaacacggtgtatctgcaaatgaacagcctgaaacttgaggatacggccgtttattactgtgcagcatccaagggtagatactcggaatatgagtactggggccaggggacccaggtcaccgtctcctcaactagtaccacgacgccagcgccgcgaccaccaacaccggcgcccaccatcgcgtcgcagcccctgtccctgcgcccagaggcgtgccggccagcggcggggggcgcagtgcacacgagggggctggacttcgcctgtgatttttgggtgctggtggtggttggtggagtcctggcttgctatagcttgctagtaacagtggcctttattattttctgggtgaggagtaagaggagcaggctcctgcacagtgactacatgaacatgactccccgccgccccgggcccacccgcaagcattaccagccctatgccccaccacgcgacttcgcagcctatcgctccaaacggggcagaaagaaactcctgtatatattcaaacaaccatttatgagaccagtacaaactactcaagaggaagatggctgtagctgccgatttccagaagaagaagaaggaggatgtgaactgagagtgaagttcagcaggagcgcagacgcccccgcgtacaagcagggccagaaccagctctataacgagctcaatctaggacgaagagaggagtacgatgttttggacaagagacgtggccgggaccctgagatggggggaaagccgagaaggaagaaccctcaggaaggcctgtacaatgaactgcagaaagataagatggcggaggcctacagtgagattgggatgaaaggcgagcgccggaggggcaaggggcacgatggcctttaccagggtctcagtacagccaccaaggacacctacgacgcccttcacatgcaggccctgccccctcgctga

SEQ ID NO: 182 - DNA, 1257 bp, Artificial Sequence
  BCMA 269A37965 CAR
atggccttaccagtgaccgccttgctcctgccgctggccttgctgctccacgccgccaggccggttaaccgcacgcgtcgcatgcatgcggtgcagctggtggagtctgggggaggattggtgcaggctggggactctctgagactctcctgtacagcctctggtgcaaccttgactaacgatcacatggcatggttccgccaggctccagggaaggggcgtgaatttgtagcagctattgactggagtggtcgtaccacaaattacgcagaccccgtagagggccgattcaccatctccagaaacaacgccaagaacacggtgtatctggaaatgaacagcctgaaacttgaggacacggccgtttattactgtgcggtcctccgcgcttggatctcatatgacaatgactactggggccaggggacccaggtcaccgtctcctcaactagtaccacgacgccagcgccgcgaccaccaacaccggcgcccaccatcgcgtcgcagcccctgtccctgcgcccagaggcgtgccggccagcggcggggggcgcagtgcacacgagggggctggacttcgcctgtgatttttgggtgctggtggtggttggtggagtcctggcttgctatagcttgctagtaacagtggcctttattattttctgggtgaggagtaagaggagcaggctcctgcacagtgactacatgaacatgactccccgccgccccgggcccacccgcaagcattaccagccctatgccccaccacgcgacttcgcagcctatcgctccaaacggggcagaaagaaactcctgtatatattcaaacaaccatttatgagaccagtacaaactactcaagaggaagatggctgtagctgccgatttccagaagaagaagaaggaggatgtgaactgagagtgaagttcagcaggagcgcagacgcccccgcgtacaagcagggccagaaccagctctataacgagctcaatctaggacgaagagaggagtacgatgttttggacaagagacgtggccgggaccctgagatggggggaaagccgagaaggaagaaccctcaggaaggcctgtacaatgaactgcagaaagataagatggcggaggcctacagtgagattgggatgaaaggcgagcgccggaggggcaaggggcacgatggcctttaccagggtctcagtacagccaccaaggacacctacgacgcccttcacatgcaggccctgccccctcgctga

SEQ ID NO: 183 - DNA, 1257 bp, Artificial Sequence
  BCMA 269A37972 CAR
atggccttaccagtgaccgccttgctcctgccgctggccttgctgctccacgccgccaggccggttaaccgcacgcgtcgcatgcatcaggtgcagctggtggagtctgggggaggattggtgcaggctgggggctctctgagactctcctgtgcagcctctggaggcaccttaagtaaaaataccgtggcttggttccgccaggctccagggaaggagcgtgggtttgtagcgtctattacctgggatggtcgtacgacatactatgcagactccgtgaagggccgattcaccatctccagagacaacgccaagaacacagtgtatctgcaaatgaacagcctgaaacctgaggatacggccgtttatgtctgtgcagacttagggaaatggcctgcgggcccggcggactactggggccaggggacccaggtcaccgtctcctcaactagtaccacgacgccagcgccgcgaccaccaacaccggcgcccaccatcgcgtcgcagcccctgtccctgcgcccagaggcgtgccggccagcggcggggggcgcagtgcacacgagggggctggacttcgcctgtgatttttgggtgctggtggtggttggtggagtcctggcttgctatagcttgctagtaacagtggcctttattattttctgggtgaggagtaagaggagcaggctcctgcacagtgactacatgaacatgactccccgccgccccgggcccacccgcaagcattaccagccctatgccccaccacgcgacttcgcagcctatcgctccaaacggggcagaaagaaactcctgtatatattcaaacaaccatttatgagaccagtacaaactactcaagaggaagatggctgtagctgccgatttccagaagaagaagaaggaggatgtgaactgagagtgaagttcagcaggagcgcagacgcccccgcgtacaagcagggccagaaccagctctataacgagctcaatctaggacgaagagaggagtacgatgttttggacaagagacgtggccgggaccctgagatggggggaaagccgagaaggaagaaccctcaggaaggcctgtacaatgaactgcagaaagataagatggcggaggcctacagtgagattgggatgaaaggcgagcgccggaggggcaaggggcacgatggcctttaccagggtctcagtacagccaccaaggacacctacgacgcccttcacatgcaggccctgccccctcgctga

SEQ ID NO: 184 - DNA, 1254 bp, Artificial Sequence
  BCMA 269A37353 CAR
atggccttaccagtgaccgccttgctcctgccgctggccttgctgctccacgccgccaggccggttaaccgcacgcgtcgcatgcatcaggtaaagctggaggagtctgggggaggcttggtgcaggctgggcggtctctgagactctcctgtgcagcctctgaacacaccttcagtagccatgtcatgggctggttccgccaggctccagggaaggagcgtgagtctgttgcagttattggctggagagatattagcacaagctatgcagactccgtgaagggccgattcaccatctccagagacaacgccaagaagacgctgtatctgcaaatgaatagcctgaaacctgaggacacggccgtttactactgtgcagcacgtcggatcgacgcagctgactttgattcctgggggcaggggacccaggtcaccgtctcctcgactagtaccacgacgccagcgccgcgaccaccaacaccggcgcccaccatcgcgtcgcagcccctgtccctgcgcccagaggcgtgccggccagcggcggggggcgcagtgcacacgagggggctggacttcgcctgtgatttttgggtgctggtggtggttggtggagtcctggcttgctatagcttgctagtaacagtggcctttattattttctgggtgaggagtaagaggagcaggctcctgcacagtgactacatgaacatgactccccgccgccccgggcccacccgcaagcattaccagccctatgccccaccacgcgacttcgcagcctatcgctccaaacggggcagaaagaaactcctgtatatattcaaacaaccatttatgagaccagtacaaactactcaagaggaagatggctgtagctgccgatttccagaagaagaagaaggaggatgtgaactgagagtgaagttcagcaggagcgcagacgcccccgcgtacaagcagggccagaaccagctctataacgagctcaatctaggacgaagagaggagtacgatgttttggacaagagacgtggccgggaccctgagatggggggaaagccgagaaggaagaaccctcaggaaggcctgtacaatgaactgcagaaagataagatggcggaggcctacagtgagattgggatgaaaggcgagcgccggaggggcaaggggcacgatggcctttaccagggtctcagtacagccaccaaggacacctacgacgcccttcacatgcaggccctgccccctcgctga

SEQ ID NO: 185 - DNA, 1254 bp, Artificial Sequence
  BCMA 269A37948 CAR
atggccttaccagtgaccgccttgctcctgccgctggccttgctgctccacgccgccaggccggttaaccgcacgcgtcgcatgcatgcggtgcagctggtggagtctgggggaggattggtgcaggctggggactctctgagactcacctgtacagcctctggacgcgccttcagtacctatttcatggcctggttccgccaggctccagggaaggagcgtgagtttgtagcaggaattgcatggagtggtggtagcacggcgtatgcagactccgtgaagggccgattcaccatctccagagacaacgccaagaacacggtgtatctgcaaatgaacagcctgaaatctgaggacacggccgtttattactgtgccagcagggggattgaggtcgaagagtttggtgcctggggccaggggacccaggtcaccgtctcgtcgactagtaccacgacgccagcgccgcgaccaccaacaccggcgcccaccatcgcgtcgcagcccctgtccctgcgcccagaggcgtgccggccagcggcggggggcgcagtgcacacgagggggctggacttcgcctgtgatttttgggtgctggtggtggttggtggagtcctggcttgctatagcttgctagtaacagtggcctttattattttctgggtgaggagtaagaggagcaggctcctgcacagtgactacatgaacatgactccccgccgccccgggcccacccgcaagcattaccagccctatgccccaccacgcgacttcgcagcctatcgctccaaacggggcagaaagaaactcctgtatatattcaaacaaccatttatgagaccagtacaaactactcaagaggaagatggctgtagctgccgatttccagaagaagaagaaggaggatgtgaactgagagtgaagttcagcaggagcgcagacgcccccgcgtacaagcagggccagaaccagctctataacgagctcaatctaggacgaagagaggagtacgatgttttggacaagagacgtggccgggaccctgagatggggggaaagccgagaaggaagaaccctcaggaaggcctgtacaatgaactgcagaaagataagatggcggaggcctacagtgagattgggatgaaaggcgagcgccggaggggcaaggggcacgatggcctttaccagggtctcagtacagccaccaaggacacctacgacgcccttcacatgcaggccctgccccctcgctga

SEQ ID NO: 186 - DNA, 1236 bp, Artificial Sequence
  CD38 38A37333 CAR
atggccttaccagtgaccgccttgctcctgccgctggccttgctgctccacgccgccaggccggttaacgatgtgcagctggtggagtctgggggaggcttggtgcagcctggggggtctctgagactctcctgtgtagcctctggattgaccttcagtagctaccccatgatgtgggtccgccaggctccaggaaaggggctcgagtgggtctcacgtattagcgatagtggtggttacacaaactatgacgactccgtgaagggccgattcaccatctccagagacaacgccaagaacacgctgtatctgcaaatgaacagcctgacacctgaggacacggccgtgtattactgtagaatcctggggttgcccaccacgggccaggggacccaggtcaccgtctcctcaacgcgtcgcatgcatactagtaccacgacgccagcgccgcgaccaccaacaccggcgcccaccatcgcgtcgcagcccctgtccctgcgcccagaggcgtgccggccagcggcggggggcgcagtgcacacgagggggctggacttcgcctgtgatttttgggtgctggtggtggttggtggagtcctggcttgctatagcttgctagtaacagtggcctttattattttctgggtgaggagtaagaggagcaggctcctgcacagtgactacatgaacatgactccccgccgccccgggcccacccgcaagcattaccagccctatgccccaccacgcgacttcgcagcctatcgctccaaacggggcagaaagaaactcctgtatatattcaaacaaccatttatgagaccagtacaaactactcaagaggaagatggctgtagctgccgatttccagaagaagaagaaggaggatgtgaactgagagtgaagttcagcaggagcgcagacgcccccgcgtacaagcagggccagaaccagctctataacgagctcaatctaggacgaagagaggagtacgatgttttggacaagagacgtggccgggaccctgagatggggggaaagccgagaaggaagaaccctcaggaaggcctgtacaatgaactgcagaaagataagatggcggaggcctacagtgagattgggatgaaaggcgagcgccggaggggcaaggggcacgatggcctttaccagggtctcagtacagccaccaaggacacctacgacgcccttcacatgcaggccctgccccctcgctga

SEQ ID NO: 187 - DNA, 1272 bp, Artificial Sequence
  CD38 38A37336 CAR
atggccttaccagtgaccgccttgctcctgccgctggccttgctgctccacgccgccaggccggttaacgaggtgcagctggtggagtctgggggaggcctggtgcagcctggggggtctctgagactctcctgtgcagcctctggattcaccttcagtagcaactggatgtattgggtccgtcaggctccagggaaggggctcgagtgggtcgcaactattagtactgatggtcgtggaacatactataaagactctgtgaagggccgattcaccgtctccagagacaacgccatgagtacgctgcttctgcaaatgaacaatctgaaatctgaagatacggccgtgtattattgtgcaaaagagccgagggtgttgatggcttacctgcggaacctgggtgactttggttcctggggccaggggacccaggtcaccgtctcctcgacgcgtcgcatgcatactagtaccacgacgccagcgccgcgaccaccaacaccggcgcccaccatcgcgtcgcagcccctgtccctgcgcccagaggcgtgccggccagcggcggggggcgcagtgcacacgagggggctggacttcgcctgtgatttttgggtgctggtggtggttggtggagtcctggcttgctatagcttgctagtaacagtggcctttattattttctgggtgaggagtaagaggagcaggctcctgcacagtgactacatgaacatgactccccgccgccccgggcccacccgcaagcattaccagccctatgccccaccacgcgacttcgcagcctatcgctccaaacggggcagaaagaaactcctgtatatattcaaacaaccatttatgagaccagtacaaactactcaagaggaagatggctgtagctgccgatttccagaagaagaagaaggaggatgtgaactgagagtgaagttcagcaggagcgcagacgcccccgcgtacaagcagggccagaaccagctctataacgagctcaatctaggacgaagagaggagtacgatgttttggacaagagacgtggccgggaccctgagatggggggaaagccgagaaggaagaaccctcaggaaggcctgtacaatgaactgcagaaagataagatggcggaggcctacagtgagattgggatgaaaggcgagcgccggaggggcaaggggcacgatggcctttaccagggtctcagtacagccaccaaggacacctacgacgcccttcacatgcaggccctgccccctcgctga

SEQ ID NO: 188 - DNA, 1239 bp, Artificial Sequence
  CD38 38A37669 CAR
atggccttaccagtgaccgccttgctcctgccgctggccttgctgctccacgccgccaggccggttaaccaggtgcagctggtggagtctgggggaggcttggtgcaggctggggggtctctgagactctcctgtgcagcctctggaaggatcttcagtatcaatgccatgggctggtaccgccaggctccagggaagcagcgcgagttggtcgccgctattagtacggctggtagcacaaactatggagactccgtgaagggccgattcaccatctccagagacaacgccaagaacacggtgtatctgcaaatgaacagcctgaaacctgaggacacagctgtttattactgtaatttaaattttcccccgtatgtgtactggggccaggggacccaggtcaccgtctcctcaacgcgtcgcatgcatactagtaccacgacgccagcgccgcgaccaccaacaccggcgcccaccatcgcgtcgcagcccctgtccctgcgcccagaggcgtgccggccagcggcggggggcgcagtgcacacgagggggctggacttcgcctgtgatttttgggtgctggtggtggttggtggagtcctggcttgctatagcttgctagtaacagtggcctttattattttctgggtgaggagtaagaggagcaggctcctgcacagtgactacatgaacatgactccccgccgccccgggcccacccgcaagcattaccagccctatgccccaccacgcgacttcgcagcctatcgctccaaacggggcagaaagaaactcctgtatatattcaaacaaccatttatgagaccagtacaaactactcaagaggaagatggctgtagctgccgatttccagaagaagaagaaggaggatgtgaactgagagtgaagttcagcaggagcgcagacgcccccgcgtacaagcagggccagaaccagctctataacgagctcaatctaggacgaagagaggagtacgatgttttggacaagagacgtggccgggaccctgagatggggggaaagccgagaaggaagaaccctcaggaaggcctgtacaatgaactgcagaaagataagatggcggaggcctacagtgagattgggatgaaaggcgagcgccggaggggcaaggggcacgatggcctttaccagggtctcagtacagccaccaaggacacctacgacgcccttcacatgcaggccctgccccctcgctga

SEQ ID NO: 189 - DNA, 1251 bp, Artificial Sequence
  CD38 38A37331 CAR
atggccttaccagtgaccgccttgctcctgccgctggccttgctgctccacgccgccaggccggttaaccaggtaaagctggaggagtctgggggaggtctggtgcagcctggggagtctctgagactctcctgttcagcctctggaagcatcttcaaagttttcagagtctttgccatgagctggtaccgccagggtcccgggaaacagcgcgagttggtcgcatccattagtagtggcgagaccacaacctatgcagactccgtgaagggccgattcaccatctccagagacaacgccaagaatacggcgtatctgcaaatggacagcctgaaacctgaggacacggccgtctattactgtaatgcggatcacacctttacaggagacttctggggccaggggacccaggtcaccgtctcctcaacgcgtcgcatgcatactagtaccacgacgccagcgccgcgaccaccaacaccggcgcccaccatcgcgtcgcagcccctgtccctgcgcccagaggcgtgccggccagcggcggggggcgcagtgcacacgagggggctggacttcgcctgtgatttttgggtgctggtggtggttggtggagtcctggcttgctatagcttgctagtaacagtggcctttattattttctgggtgaggagtaagaggagcaggctcctgcacagtgactacatgaacatgactccccgccgccccgggcccacccgcaagcattaccagccctatgccccaccacgcgacttcgcagcctatcgctccaaacggggcagaaagaaactcctgtatatattcaaacaaccatttatgagaccagtacaaactactcaagaggaagatggctgtagctgccgatttccagaagaagaagaaggaggatgtgaactgagagtgaagttcagcaggagcgcagacgcccccgcgtacaagcagggccagaaccagctctataacgagctcaatctaggacgaagagaggagtacgatgttttggacaagagacgtggccgggaccctgagatggggggaaagccgagaaggaagaaccctcaggaaggcctgtacaatgaactgcagaaagataagatggcggaggcctacagtgagattgggatgaaaggcgagcgccggaggggcaaggggcacgatggcctttaccagggtctcagtacagccaccaaggacacctacgacgcccttcacatgcaggccctgccccctcgctga

SEQ ID NO: 190 - DNA, 1242 bp, Artificial Sequence
  CD38 38A37717 CAR
atggccttaccagtgaccgccttgctcctgccgctggccttgctgctccacgccgccaggccggttaacgaggtgcagctggtggaaagcggggggggactggtgcaggcaggcgggtcactgagactgtcatgtatcgcaactgggaaggtgtttagcatctacgacatgggctggtataggcaggcaccaggaaagcagagggagctggtggccgagatcaccagctccggcaccacacactacgacgatttcgtgtctggccggtttaccatcagcagagacaacgccaagaatacagtgtatctgcagatgaacaccctgaaggccgaggatacagccgtgtactattgccgggctaatcacgtcttcggcggctcctactgggggcagggaactcaggtcactgtgtcatccacgcgtcgcatgcatactagtaccacgacgccagcgccgcgaccaccaacaccggcgcccaccatcgcgtcgcagcccctgtccctgcgcccagaggcgtgccggccagcggcggggggcgcagtgcacacgagggggctggacttcgcctgtgatttttgggtgctggtggtggttggtggagtcctggcttgctatagcttgctagtaacagtggcctttattattttctgggtgaggagtaagaggagcaggctcctgcacagtgactacatgaacatgactccccgccgccccgggcccacccgcaagcattaccagccctatgccccaccacgcgacttcgcagcctatcgctccaaacggggcagaaagaaactcctgtatatattcaaacaaccatttatgagaccagtacaaactactcaagaggaagatggctgtagctgccgatttccagaagaagaagaaggaggatgtgaactgagagtgaagttcagcaggagcgcagacgcccccgcgtacaagcagggccagaaccagctctataacgagctcaatctaggacgaagagaggagtacgatgttttggacaagagacgtggccgggaccctgagatggggggaaagccgagaaggaagaaccctcaggaaggcctgtacaatgaactgcagaaagataagatggcggaggcctacagtgagattgggatgaaaggcgagcgccggaggggcaaggggcacgatggcctttaccagggtctcagtacagccaccaaggacacctacgacgcccttcacatgcaggccctgccccctcgctga

SEQ ID NO: 191 - DNA, 1239 bp, Artificial Sequence
  CD38 38A37719 CAR
atggccttaccagtgaccgccttgctcctgccgctggccttgctgctccacgccgccaggccggttaaccaggtaaagctggaggagtctgggggaggctcggtgcagactggggggtctctgagactctcctgtgcagcctctgcaagcatcttcactaggctgcccatgggctggtaccgccaggctccagggaagcagcgcgagttggtcgtaggcattgttcctagtggtaggataaactatgcagactccgtgaagggccgattcaccatctccagagacaacgccaagaacacggtgtatctgcaaatgaacagcctgcgccctgaggacacagccgtctattactgccgcgccgataccttccccttgcccacctggggccaggggacccaggtcaccgtctcctcaacgcgtcgcatgcatactagtaccacgacgccagcgccgcgaccaccaacaccggcgcccaccatcgcgtcgcagcccctgtccctgcgcccagaggcgtgccggccagcggcggggggcgcagtgcacacgagggggctggacttcgcctgtgatttttgggtgctggtggtggttggtggagtcctggcttgctatagcttgctagtaacagtggcctttattattttctgggtgaggagtaagaggagcaggctcctgcacagtgactacatgaacatgactccccgccgccccgggcccacccgcaagcattaccagccctatgccccaccacgcgacttcgcagcctatcgctccaaacggggcagaaagaaactcctgtatatattcaaacaaccatttatgagaccagtacaaactactcaagaggaagatggctgtagctgccgatttccagaagaagaagaaggaggatgtgaactgagagtgaagttcagcaggagcgcagacgcccccgcgtacaagcagggccagaaccagctctataacgagctcaatctaggacgaagagaggagtacgatgttttggacaagagacgtggccgggaccctgagatggggggaaagccgagaaggaagaaccctcaggaaggcctgtacaatgaactgcagaaagataagatggcggaggcctacagtgagattgggatgaaaggcgagcgccggaggggcaaggggcacgatggcctttaccagggtctcagtacagccaccaaggacacctacgacgcccttcacatgcaggccctgccccctcgctga

SEQ ID NO: 192 - DNA, 1272 bp, Artificial Sequence
  CD38 38A37330 CAR
atggccttaccagtgaccgccttgctcctgccgctggccttgctgctccacgccgccaggccggttaaccaggtgcagctggtggagtctgggggaggattggtgcaggctggggactctctgagactctcctgtgcagcctctggacgcgcctacgctacgatggcctggttccgccaggctccagggaaggagcgtgagtttgtagcacatctgcgcgtgagtggtgataccacttactatacagactccgtgaagggccgattcaccatctccagagacaacgccaagaacacggcgtatctgcaaatgaacatgttgaaacctgaggacacggccgtttattactgtgcagcgggaccgtatggcattcttgccgctgccagggtcagtaatccaggaaattatgattattggggccaggggacccaggtcaccgtctcctcaacgcgtcgcatgcatactagtaccacgacgccagcgccgcgaccaccaacaccggcgcccaccatcgcgtcgcagcccctgtccctgcgcccagaggcgtgccggccagcggcggggggcgcagtgcacacgagggggctggacttcgcctgtgatttttgggtgctggtggtggttggtggagtcctggcttgctatagcttgctagtaacagtggcctttattattttctgggtgaggagtaagaggagcaggctcctgcacagtgactacatgaacatgactccccgccgccccgggcccacccgcaagcattaccagccctatgccccaccacgcgacttcgcagcctatcgctccaaacggggcagaaagaaactcctgtatatattcaaacaaccatttatgagaccagtacaaactactcaagaggaagatggctgtagctgccgatttccagaagaagaagaaggaggatgtgaactgagagtgaagttcagcaggagcgcagacgcccccgcgtacaagcagggccagaaccagctctataacgagctcaatctaggacgaagagaggagtacgatgttttggacaagagacgtggccgggaccctgagatggggggaaagccgagaaggaagaaccctcaggaaggcctgtacaatgaactgcagaaagataagatggcggaggcctacagtgagattgggatgaaaggcgagcgccggaggggcaaggggcacgatggcctttaccagggtctcagtacagccaccaaggacacctacgacgcccttcacatgcaggccctgccccctcgctga

SEQ ID NO: 193 - DNA, 1263 bp, Artificial Sequence
  CD38 38A37334 CAR
atggccttaccagtgaccgccttgctcctgccgctggccttgctgctccacgccgccaggccggttaacgaggtgcagctggtggagtctgggggaggattggtgcaggctgggggctctctgagactctcctgtgcagcctctggactcaccttcagtagttatattatgggctggttccgccaggctccaggcgaggagcgcgagttggtcgcggaaattagtagcggtggtatgacatcgtatgcagactccgtgaagggccgattcaccatctccagagacaacgccaagaagacggggtatctgcaaatgaacagcctgaaacctgaggacacggccgtttactattgtgcagcccctgagaggggtagtatctggtacagccgctacgaatataagtactggggccaggggacccaggtcaccgtctcctcaacgcgtcgcatgcatactagtaccacgacgccagcgccgcgaccaccaacaccggcgcccaccatcgcgtcgcagcccctgtccctgcgcccagaggcgtgccggccagcggcggggggcgcagtgcacacgagggggctggacttcgcctgtgatttttgggtgctggtggtggttggtggagtcctggcttgctatagcttgctagtaacagtggcctttattattttctgggtgaggagtaagaggagcaggctcctgcacagtgactacatgaacatgactccccgccgccccgggcccacccgcaagcattaccagccctatgccccaccacgcgacttcgcagcctatcgctccaaacggggcagaaagaaactcctgtatatattcaaacaaccatttatgagaccagtacaaactactcaagaggaagatggctgtagctgccgatttccagaagaagaagaaggaggatgtgaactgagagtgaagttcagcaggagcgcagacgcccccgcgtacaagcagggccagaaccagctctataacgagctcaatctaggacgaagagaggagtacgatgttttggacaagagacgtggccgggaccctgagatggggggaaagccgagaaggaagaaccctcaggaaggcctgtacaatgaactgcagaaagataagatggcggaggcctacagtgagattgggatgaaaggcgagcgccggaggggcaaggggcacgatggcctttaccagggtctcagtacagccaccaaggacacctacgacgcccttcacatgcaggccctgccccctcgctga

SEQ ID NO: 194 - DNA, 1254 bp, Artificial Sequence
  CD38 38A37730 CAR
atggccttaccagtgaccgccttgctcctgccgctggccttgctgctccacgccgccaggccggttaacgccgtgcagctggtggattctgggggaggcttggcgcagactggggggtctctgagactctcctgtgcagcctctcaagggatcttcactatcaatgccatgggctggtaccgccaggttccagggaagcagcgggagttggtcgcagaagttagtagtggtggccgcacagactatgcagactccgtgaagggccgattcaccatctccagagacaacgccaagaacacggtgtacctgcaaatgaacagcctgaaacctgaggacacaggcgtctattattgtcgagtttctggatggcatgtgtttgtcggtgaccgcatagtttggggccagggcaccctggtcactgtctcctcaacgcgtcgcatgcatactagtaccacgacgccagcgccgcgaccaccaacaccggcgcccaccatcgcgtcgcagcccctgtccctgcgcccagaggcgtgccggccagcggcggggggcgcagtgcacacgagggggctggacttcgcctgtgatttttgggtgctggtggtggttggtggagtcctggcttgctatagcttgctagtaacagtggcctttattattttctgggtgaggagtaagaggagcaggctcctgcacagtgactacatgaacatgactccccgccgccccgggcccacccgcaagcattaccagccctatgccccaccacgcgacttcgcagcctatcgctccaaacggggcagaaagaaactcctgtatatattcaaacaaccatttatgagaccagtacaaactactcaagaggaagatggctgtagctgccgatttccagaagaagaagaaggaggatgtgaactgagagtgaagttcagcaggagcgcagacgcccccgcgtacaagcagggccagaaccagctctataacgagctcaatctaggacgaagagaggagtacgatgttttggacaagagacgtggccgggaccctgagatggggggaaagccgagaaggaagaaccctcaggaaggcctgtacaatgaactgcagaaagataagatggcggaggcctacagtgagattgggatgaaaggcgagcgccggaggggcaaggggcacgatggcctttaccagggtctcagtacagccaccaaggacacctacgacgcccttcacatgcaggccctgccccctcgctga

SEQ ID NO: 195 - DNA, 1263 bp, Artificial Sequence
  CD38 38A37340 CAR
atggccttaccagtgaccgccttgctcctgccgctggccttgctgctccacgccgccaggccggttaacgatgtgcagctggtggagtctgggggaggattggtgcaggctggggactctctgagactctcctgtgcagcctctggacgcaccttcagtagctatgccatggcctggttccgccaggctccagggaaggagcgtgagattgtttcgtctatcagtaccagtggtggtatcacagactatgcagactccgtgaagggccgattcaccatctccaaagacagcgcgaagatgaacacggtgtatctgcaaatgaatagcctagaacctgaggacacggccgtttactactgtgcggcccgtacatggtaccttcgtacttctctccaatatgactattggggccaggggacccaggtcaccgtctcctcaacgcgtcgcatgcatactagtaccacgacgccagcgccgcgaccaccaacaccggcgcccaccatcgcgtcgcagcccctgtccctgcgcccagaggcgtgccggccagcggcggggggcgcagtgcacacgagggggctggacttcgcctgtgatttttgggtgctggtggtggttggtggagtcctggcttgctatagcttgctagtaacagtggcctttattattttctgggtgaggagtaagaggagcaggctcctgcacagtgactacatgaacatgactccccgccgccccgggcccacccgcaagcattaccagccctatgccccaccacgcgacttcgcagcctatcgctccaaacggggcagaaagaaactcctgtatatattcaaacaaccatttatgagaccagtacaaactactcaagaggaagatggctgtagctgccgatttccagaagaagaagaaggaggatgtgaactgagagtgaagttcagcaggagcgcagacgcccccgcgtacaagcagggccagaaccagctctataacgagctcaatctaggacgaagagaggagtacgatgttttggacaagagacgtggccgggaccctgagatggggggaaagccgagaaggaagaaccctcaggaaggcctgtacaatgaactgcagaaagataagatggcggaggcctacagtgagattgggatgaaaggcgagcgccggaggggcaaggggcacgatggcctttaccagggtctcagtacagccaccaaggacacctacgacgcccttcacatgcaggccctgccccctcgctga

SEQ ID NO: 196 - DNA, 1257 bp, Artificial Sequence
  CD38 38A37731 CAR
atggccttaccagtgaccgccttgctcctgccgctggccttgctgctccacgccgccaggccggttaaccaggtaaagctggaggagtctgggggaggcttggtgcaggctggggggtctctgagactctcctgtgtagcctctggaaccatcgtcagtatcagtaccatgggctggtaccgccaggctccagggaagcagcgcgagttggtcgcgactataaccaggcgtggacgcacgaactatacagactccgtgaagggccgattcaccatctccagagacaacgccaaaaacacggtgtatctgcaaatgaacagcctgaaacctgaggacacagccgtctattactgtaatgcagaggtgcaactggatatatgggcatctgcgtatgactactggggccaggggacccaggtcaccgtcgcctcaacgcgtcgcatgcatactagtaccacgacgccagcgccgcgaccaccaacaccggcgcccaccatcgcgtcgcagcccctgtccctgcgcccagaggcgtgccggccagcggcggggggcgcagtgcacacgagggggctggacttcgcctgtgatttttgggtgctggtggtggttggtggagtcctggcttgctatagcttgctagtaacagtggcctttattattttctgggtgaggagtaagaggagcaggctcctgcacagtgactacatgaacatgactccccgccgccccgggcccacccgcaagcattaccagccctatgccccaccacgcgacttcgcagcctatcgctccaaacggggcagaaagaaactcctgtatatattcaaacaaccatttatgagaccagtacaaactactcaagaggaagatggctgtagctgccgatttccagaagaagaagaaggaggatgtgaactgagagtgaagttcagcaggagcgcagacgcccccgcgtacaagcagggccagaaccagctctataacgagctcaatctaggacgaagagaggagtacgatgttttggacaagagacgtggccgggaccctgagatggggggaaagccgagaaggaagaaccctcaggaaggcctgtacaatgaactgcagaaagataagatggcggaggcctacagtgagattgggatgaaaggcgagcgccggaggggcaaggggcacgatggcctttaccagggtctcagtacagccaccaaggacacctacgacgcccttcacatgcaggccctgccccctcgctga

SEQ ID NO: 197 - DNA, 1239 bp, Artificial Sequence
  CD38 38A37326 CAR
atggccttaccagtgaccgccttgctcctgccgctggccttgctgctccacgccgccaggccggttaacgaggtgcagctggtggagtctgggggaggattggtgcaggctgggggctctctgagactctcctgtgcagcctctggacgcacctatgccatgggctggtatcgccaggctccagggaagcagcgcgacttggtcgcaactattagtggtgcgggtaacacaaagtatgcagactccgtgaagggccgattcaccatctccagagacaacgccaagaacacaatgtatctgcaaatgaacagcctgaaacctgaggacacggccgtttattactgtgccgcgggtaaatggttccctgctgcgaatgagtactggggccaggggacccaggtcaccgtctcctcaacgcgtcgcatgcatactagtaccacgacgccagcgccgcgaccaccaacaccggcgcccaccatcgcgtcgcagcccctgtccctgcgcccagaggcgtgccggccagcggcggggggcgcagtgcacacgagggggctggacttcgcctgtgatttttgggtgctggtggtggttggtggagtcctggcttgctatagcttgctagtaacagtggcctttattattttctgggtgaggagtaagaggagcaggctcctgcacagtgactacatgaacatgactccccgccgccccgggcccacccgcaagcattaccagccctatgccccaccacgcgacttcgcagcctatcgctccaaacggggcagaaagaaactcctgtatatattcaaacaaccatttatgagaccagtacaaactactcaagaggaagatggctgtagctgccgatttccagaagaagaagaaggaggatgtgaactgagagtgaagttcagcaggagcgcagacgcccccgcgtacaagcagggccagaaccagctctataacgagctcaatctaggacgaagagaggagtacgatgttttggacaagagacgtggccgggaccctgagatggggggaaagccgagaaggaagaaccctcaggaaggcctgtacaatgaactgcagaaagataagatggcggaggcctacagtgagattgggatgaaaggcgagcgccggaggggcaaggggcacgatggcctttaccagggtctcagtacagccaccaaggacacctacgacgcccttcacatgcaggccctgccccctcgctga

SEQ ID NO: 198 - protein, 495 aa, Artificial Sequence
  BCMAx2 269A37946 GSI5014 CAR
MALPVTALLLPLALLLHAARPQVQLVESGGGLVQPGGSLRLSCEASGFTLDYYAIGWFRQAPGKEREGVICISRSDGSTYYADSVKGRFTISRDNAKKTVYLQMISLKPEDTAAYYCAAGADCSGYLRDYEFRGQGTQVTVSSGGGGSQVQLVESGGGLVQPGGSLRLSCEASGFTLDYYAIGWFRQAPGKEREGVICISRSDGSTYYADSVKGRFTISRDNAKKTVYLQMISLKPEDTAAYYCAAGADCSGYLRDYEFRGQGTQVTVSSTSTTTPAPRPPTPAPTIASQPLSLRPEACRPAAGGAVHTRGLDFACDIYIWAPLAGTCGVLLLSLVITLYCKRGRKKLLYIFKQPFMRPVQTTQEEDGCSCRFPEEEEGGCELRVKFSRSADAPAYQQGQNQLYNELNLGRREEYDVLDKRRGRDPEMGGKPRRKNPQEGLYNELQKDKMAEAYSEIGMKGERRRGKGHDGLYQGLSTATKDTYDALHMQALPPR

SEQ ID NO: 199 - protein, 622 aa, Artificial Sequence
  BCMAx3 269A37946 GSI5015 CAR
MALPVTALLLPLALLLHAARPQVQLVESGGGLVQPGGSLRLSCEASGFTLDYYAIGWFRQAPGKEREGVICISRSDGSTYYADSVKGRFTISRDNAKKTVYLQMISLKPEDTAAYYCAAGADCSGYLRDYEFRGQGTQVTVSSGGGGSQVQLVESGGGLVQPGGSLRLSCEASGFTLDYYAIGWFRQAPGKEREGVICISRSDGSTYYADSVKGRFTISRDNAKKTVYLQMISLKPEDTAAYYCAAGADCSGYLRDYEFRGQGTQVTVSSGGGGSQVQLVESGGGLVQPGGSLRLSCEASGFTLDYYAIGWFRQAPGKEREGVICISRSDGSTYYADSVKGRFTISRDNAKKTVYLQMISLKPEDTAAYYCAAGADCSGYLRDYEFRGQGTQVTVSSTSTTTPAPRPPTPAPTIASQPLSLRPEACRPAAGGAVHTRGLDFACDIYIWAPLAGTCGVLLLSLVITLYCKRGRKKLLYIFKQPFMRPVQTTQEEDGCSCRFPEEEEGGCELRVKFSRSADAPAYQQGQNQLYNELNLGRREEYDVLDKRRGRDPEMGGKPRRKNPQEGLYNELQKDKMAEAYSEIGMKGERRRGKGHDGLYQGLSTATKDTYDALHMQALPPR

SEQ ID NO: 200 - protein, 483 aa, Artificial Sequence
  CD38x2 38A37717 GSI5016 CAR
MALPVTALLLPLALLLHAARPEVQLVESGGGLVQAGGSLRLSCIATGKVFSIYDMGWYRQAPGKQRELVAEITSSGTTHYDDFVSGRFTISRDNAKNTVYLQMNTLKAEDTAVYYCRANHVFGGSYWGQGTQVTVSSGGGGSEVQLVESGGGLVQAGGSLRLSCIATGKVFSIYDMGWYRQAPGKQRELVAEITSSGTTHYDDFVSGRFTISRDNAKNTVYLQMNTLKAEDTAVYYCRANHVFGGSYWGQGTQVTVSSTSTTTPAPRPPTPAPTIASQPLSLRPEACRPAAGGAVHTRGLDFACDIYIWAPLAGTCGVLLLSLVITLYCKRGRKKLLYIFKQPFMRPVQTTQEEDGCSCRFPEEEEGGCELRVKFSRSADAPAYQQGQNQLYNELNLGRREEYDVLDKRRGRDPEMGGKPRRKNPQEGLYNELQKDKMAEAYSEIGMKGERRRGKGHDGLYQGLSTATKDTYDALHMQALPPR

SEQ ID NO: 201 - protein, 604 aa, Artificial Sequence
  CD38x3 38A37717 GSI5017 CAR
MALPVTALLLPLALLLHAARPEVQLVESGGGLVQAGGSLRLSCIATGKVFSIYDMGWYRQAPGKQRELVAEITSSGTTHYDDFVSGRFTISRDNAKNTVYLQMNTLKAEDTAVYYCRANHVFGGSYWGQGTQVTVSSGGGGSEVQLVESGGGLVQAGGSLRLSCIATGKVFSIYDMGWYRQAPGKQRELVAEITSSGTTHYDDFVSGRFTISRDNAKNTVYLQMNTLKAEDTAVYYCRANHVFGGSYWGQGTQVTVSSGGGGSEVQLVESGGGLVQAGGSLRLSCIATGKVFSIYDMGWYRQAPGKQRELVAEITSSGTTHYDDFVSGRFTISRDNAKNTVYLQMNTLKAEDTAVYYCRANHVFGGSYWGQGTQVTVSSTSTTTPAPRPPTPAPTIASQPLSLRPEACRPAAGGAVHTRGLDFACDIYIWAPLAGTCGVLLLSLVITLYCKRGRKKLLYIFKQPFMRPVQTTQEEDGCSCRFPEEEEGGCELRVKFSRSADAPAYQQGQNQLYNELNLGRREEYDVLDKRRGRDPEMGGKPRRKNPQEGLYNELQKDKMAEAYSEIGMKGERRRGKGHDGLYQGLSTATKDTYDALHMQALPPR

SEQ ID NO: 202 - DNA, 1488 bp, Artificial Sequence
  BCMAx2 269A37946 GSI5014 CAR
atggctctgcccgtcactgctctgctgctgcccctggctctgctgctgcacgctgctcgccctcaggtccagctggtggaaagcggaggaggcctggtgcagccaggaggcagcctgaggctgtcctgcgaggcctctggcttcaccctggactactatgccatcggctggtttaggcaggcacctggaaaggagagggagggagtgatctgtatctctcgcagcgacggcagcacatactatgccgattccgtgaagggccggttcaccatcagcagagacaacgccaagaagacagtgtacctgcagatgatctccctgaagcctgaggataccgcagcatactattgcgcagcaggagcagactgtagcggatacctgagggattatgagtttaggggacagggaacccaggtgacagtgagctccggaggaggaggctcccaggtgcagctggtggagtctggaggcggcctggtgcagcctggaggcagcctgagactgagctgtgaagcttccggatttaccctggactactatgcaatcggatggtttaggcaggcaccaggaaaggagagagaaggcgtgatctgtatctccagatctgacggctctacatactatgccgatagtgtcaaaggacggttcaccatctctagagataatgccaagaagacagtctatctgcagatgattagcctgaagcccgaggacacagccgcctattactgcgcagcaggagcagattgtagtgggtatctgagggactatgagtttcgggggcaggggacacaggtgacagtgagttctactagtaccacgacgccagcgccgcgaccaccaacaccggcgcccaccatcgcgtcgcagcccctgtccctgcgcccagaggcgtgccggccagcggcggggggcgcagtgcacacgagggggctggacttcgcctgtgatatctacatctgggcgcccttggccgggacttgtggggtccttctcctgtcactggttatcaccctttactgcaaacggggcagaaagaaactcctgtatatattcaaacaaccatttatgagaccagtacaaactactcaagaggaagatggctgtagctgccgatttccagaagaagaagaaggaggatgtgaactgagagtgaagttcagcaggagcgcagacgcccccgcgtaccagcagggccagaaccagctctataacgagctcaatctaggacgaagagaggagtacgatgttttggacaagagacgtggccgggaccctgagatggggggaaagccgagaaggaagaaccctcaggaaggcctgtacaatgaactgcagaaagataagatggcggaggcctacagtgagattgggatgaaaggcgagcgccggaggggcaaggggcacgatggcctttaccagggtctcagtacagccaccaaggacacctacgacgcccttcacatgcaggccctgccccctcgctaa

SEQ ID NO: 203 - DNA, 1869 bp, Artificial Sequence
  BCMAx3 269A37946 GSI5015 CAR
atggctctgcccgtcactgctctgctgctgcctctggccctgctgctgcacgccgcacgccctcaggtccagctggtcgagtcaggaggaggcctggtgcagccaggaggctccctgcggctgtcttgcgaggccagcggcttcaccctggactactatgccatcggctggtttaggcaggcacctggaaaggagagggagggagtgatctgtatctccagatctgacggctccacatactatgccgattctgtgaagggccggttcaccatctctagagacaacgccaagaagacagtgtacctgcagatgatcagcctgaagcccgaggataccgcagcatactattgcgcagcaggagcagactgttccggatacctgagggattatgagtttaggggacagggaacccaggtgacagtgagctccggaggaggaggctcccaggtgcagctggtggagtctggaggcggcctggtgcagcctggaggctccctgaggctgtcttgcgaggcaagcggcttcaccctggattactatgcaatcggatggtttaggcaggcaccaggaaaggagagagaaggcgtgatctgtatcagccgctccgacggcagtacctactatgccgattccgtcaaaggccggttcaccatctccagagacaatgccaagaagacagtctatctgcagatgatctctctgaagcctgaggatacagccgcctattactgtgccgcaggagcagactgtagtggctatctgagagattatgagtttcgcggccagggcacccaggtgacagtgtctagcggaggaggaggcagccaggtccagctggtggaatccggcggaggcctggtgcagcccggcggctccctgagactgtcctgtgaagcctccggatttactctggattattacgctattggatggttcagacaggcccctggcaaagaaagagaaggggtgatctgtatctctcggagcgacggctctacatactatgccgatagcgtcaagggaagatttaccatctccagagataatgccaagaagacagtgtatctgcagatgatttccctgaagcccgaggacactgccgcctattactgtgcagcaggagcagattgtagcgggtatctgcgggattatgaatttagaggacagggcactcaggtgacagtctcaagcactagtaccacgacgccagcgccgcgaccaccaacaccggcgcccaccatcgcgtcgcagcccctgtccctgcgcccagaggcgtgccggccagcggcggggggcgcagtgcacacgagggggctggacttcgcctgtgatatctacatctgggcgcccttggccgggacttgtggggtccttctcctgtcactggttatcaccctttactgcaaacggggcagaaagaaactcctgtatatattcaaacaaccatttatgagaccagtacaaactactcaagaggaagatggctgtagctgccgatttccagaagaagaagaaggaggatgtgaactgagagtgaagttcagcaggagcgcagacgcccccgcgtaccagcagggccagaaccagctctataacgagctcaatctaggacgaagagaggagtacgatgttttggacaagagacgtggccgggaccctgagatggggggaaagccgagaaggaagaaccctcaggaaggcctgtacaatgaactgcagaaagataagatggcggaggcctacagtgagattgggatgaaaggcgagcgccggaggggcaaggggcacgatggcctttaccagggtctcagtacagccaccaaggacacctacgacgcccttcacatgcaggccctgccccctcgctaa

SEQ ID NO: 204 - DNA, 1452 bp, Artificial Sequence
  CD38x2 38A37717 GSI5016 CAR
atggccctgcctgtcaccgctctgctgctgcctctggccctgctgctgcacgctgctagacccgaagtccagctggtcgaaagtgggggaggcctggtgcaggcaggaggcagcctgaggctgtcctgcatcgccaccggcaaggtgttcagcatctacgacatgggatggtataggcaggcaccaggaaagcagagagagctggtggccgagatcacaagctccggcaccacacactacgacgatttcgtgtccggccggtttaccatctctagagacaacgccaagaatacagtgtatctgcagatgaacaccctgaaggccgaggatacagccgtgtactattgccgggccaatcacgtgttcggaggatcctactggggacagggaacccaggtgacagtgtctagcggaggaggaggatctgaggtgcagctggtggagagcggaggcggcctggtgcaggccggaggctctctgagactgagctgtattgctaccggcaaggtgttttctatctacgatatgggctggtataggcaggcacctggaaagcagagggagctggtggctgaaatcacctcctctggaactacccattacgacgatttcgtgagcggcaggtttaccatctcccgcgataatgctaaaaacaccgtctacctgcagatgaatactctgaaagctgaagacacagccgtgtactattgtcgggctaaccatgtcttcgggggctcctattgggggcagggaactcaggtcaccgtgtcatcaactagtaccacgacgccagcgccgcgaccaccaacaccggcgcccaccatcgcgtcgcagcccctgtccctgcgcccagaggcgtgccggccagcggcggggggcgcagtgcacacgagggggctggacttcgcctgtgatatctacatctgggcgcccttggccgggacttgtggggtccttctcctgtcactggttatcaccctttactgcaaacggggcagaaagaaactcctgtatatattcaaacaaccatttatgagaccagtacaaactactcaagaggaagatggctgtagctgccgatttccagaagaagaagaaggaggatgtgaactgagagtgaagttcagcaggagcgcagacgcccccgcgtaccagcagggccagaaccagctctataacgagctcaatctaggacgaagagaggagtacgatgttttggacaagagacgtggccgggaccctgagatggggggaaagccgagaaggaagaaccctcaggaaggcctgtacaatgaactgcagaaagataagatggcggaggcctacagtgagattgggatgaaaggcgagcgccggaggggcaaggggcacgatggcctttaccagggtctcagtacagccaccaaggacacctacgacgcccttcacatgcaggccctgccccctcgctaa

SEQ ID NO: 205 - DNA, 1815 bp, Artificial Sequence
  CD38x3 38A37717 GSI5017 CAR
atggctctgcctgtcaccgcactgctgctgcccctggccctgctgctgcacgccgcaagacctgaagtccagctggtcgaatccggaggaggcctggtgcaggcaggaggctccctgcggctgtcttgcatcgccaccggcaaggtgttcagcatctacgacatgggctggtataggcaggcaccaggaaagcagagggagctggtggccgagatcacaagctccggcaccacacactacgacgatttcgtgtccggccggtttaccatctctagagacaacgccaagaatacagtgtatctgcagatgaacaccctgaaggccgaggatacagccgtgtactattgccgggccaatcacgtgttcggaggatcttactggggacagggaacccaggtgacagtgtctagcggaggaggaggatccgaggtgcagctggtggagtctggaggcggcctggtgcaggccggaggcagcctgagactgtcctgtattgctaccggcaaggtgttttccatctacgatatgggctggtatcggcaggcccctggcaagcagagagagctggtggctgaaatcacatcctctggaactacccattacgacgatttcgtgagcggcaggtttaccatctcccgcgataatgctaaaaacaccgtctacctgcagatgaatactctgaaagctgaagacaccgctgtgtactattgcagagctaaccatgtgttcggaggaagctattggggccagggcactcaggtgacagtgagctccggcggcggcggcagtgaagtgcagctggtggagtccggagggggcctggtgcaggccggcggctctctgcgcctgagctgtattgcaactggaaaagtgttttccatttatgatatgggatggtacagacaggcccctgggaaacagagagagctggtggcagaaatcacctctagtggaactacccactatgatgatttcgtgtctggccggtttaccatcagcagggataatgctaaaaacactgtctacctgcagatgaacactctgaaagctgaagataccgccgtgtactattgtagggctaaccatgtctttggggggtcatactgggggcaggggactcaggtcaccgtctcatccactagtaccacgacgccagcgccgcgaccaccaacaccggcgcccaccatcgcgtcgcagcccctgtccctgcgcccagaggcgtgccggccagcggcggggggcgcagtgcacacgagggggctggacttcgcctgtgatatctacatctgggcgcccttggccgggacttgtggggtccttctcctgtcactggttatcaccctttactgcaaacggggcagaaagaaactcctgtatatattcaaacaaccatttatgagaccagtacaaactactcaagaggaagatggctgtagctgccgatttccagaagaagaagaaggaggatgtgaactgagagtgaagttcagcaggagcgcagacgcccccgcgtaccagcagggccagaaccagctctataacgagctcaatctaggacgaagagaggagtacgatgttttggacaagagacgtggccgggaccctgagatggggggaaagccgagaaggaagaaccctcaggaaggcctgtacaatgaactgcagaaagataagatggcggaggcctacagtgagattgggatgaaaggcgagcgccggaggggcaaggggcacgatggcctttaccagggtctcagtacagccaccaaggacacctacgacgcccttcacatgcaggccctgccccctcgctaa

SEQ ID NO: 206 - protein, 502 aa, Artificial Sequence
  CD19XCD20 single-domain antibody-based bispecific CAR
MALPVTALLLPLALLLHAARPQVKLEESGGELVQPGGPLRLSCAASGNIFSINRMGWYRQAPGKQRAFVASITVRGITNYADSVKGRFTISVDKSKNTIYLQMNALKPEDTAVYYCNAVSSNRDPDYWGQGTQVTVSSGGGSGGGSGGGSGGGSPVQLVESGGGLVQAGDSLRLSCAASGRTFGIGTMGWFRQPPGKEREFVAAIRWSTGGTRYADSVKGRFTISRDNAKLTVDLQMDSLKPEDTAVYYCAADRLSLDLSGRYHYNPAVYDYWGQGTQVTVSSIEVMYPPPYLDNEKSNGTIIHVKGKHLCPSPLFPGPSKPFWVLVVVGGVLACYSLLVTVAFIIFWVRSKRSRLLHSDYMNMTPRRPGPTRKHYQPYAPPRDFAAYRSRVKFSRSADAPAYQQGQNQLYNELNLGRREEYDVLDKRRGRDPEMGGKPRRKNPQEGLYNELQKDKMAEAYSEIGMKGERRRGKGHDGLYQGLSTATKDTYDALHMQALPPR

SEQ ID NO: 207 - protein, 489 aa, Artificial Sequence
  CD38xBCMA 38A37717 269A37346 GSI5001 CAR
MALPVTALLLPLALLLHAARPEVQLVESGGGLVQAGGSLRLSCIATGKVFSIYDMGWYRQAPGKQRELVAEITSSGTTHYDDFVSGRFTISRDNAKNTVYLQMNTLKAEDTAVYYCRANHVFGGSYWGQGTQVTVSSGGGGSQVQLVESGGGLVQPGGSLRLSCEASGFTLDYYAIGWFRQAPGKEREGVICISRSDGSTYYADSVKGRFTISRDNAKKTVYLQMISLKPEDTAAYYCAAGADCSGYLRDYEFRGQGTQVTVSSTSTTTPAPRPPTPAPTIASQPLSLRPEACRPAAGGAVHTRGLDFACDIYIWAPLAGTCGVLLLSLVITLYCKRGRKKLLYIFKQPFMRPVQTTQEEDGCSCRFPEEEEGGCELRVKFSRSADAPAYQQGQNQLYNELNLGRREEYDVLDKRRGRDPEMGGKPRRKNPQEGLYNELQKDKMAEAYSEIGMKGERRRGKGHDGLYQGLSTATKDTYDALHMQALPPR

SEQ ID NO: 208 - protein, 494 aa, Artificial Sequence
  CD38xBCMA 38A37717 269A37346 GSI5002 CAR
MALPVTALLLPLALLLHAARPEVQLVESGGGLVQAGGSLRLSCIATGKVFSIYDMGWYRQAPGKQRELVAEITSSGTTHYDDFVSGRFTISRDNAKNTVYLQMNTLKAEDTAVYYCRANHVFGGSYWGQGTQVTVSSGGGGSGGGGSQVQLVESGGGLVQPGGSLRLSCEASGFTLDYYAIGWFRQAPGKEREGVICISRSDGSTYYADSVKGRFTISRDNAKKTVYLQMISLKPEDTAAYYCAAGADCSGYLRDYEFRGQGTQVTVSSTSTTTPAPRPPTPAPTIASQPLSLRPEACRPAAGGAVHTRGLDFACDIYIWAPLAGTCGVLLLSLVITLYCKRGRKKLLYIFKQPFMRPVQTTQEEDGCSCRFPEEEEGGCELRVKFSRSADAPAYQQGQNQLYNELNLGRREEYDVLDKRRGRDPEMGGKPRRKNPQEGLYNELQKDKMAEAYSEIGMKGERRRGKGHDGLYQGLSTATKDTYDALHMQALPPR

SEQ ID NO: 209 - protein, 500 aa, Artificial Sequence
  CD38xBCMA 38A37717 269A37346 GSI5003 CAR
MALPVTALLLPLALLLHAARPEVQLVESGGGLVQAGGSLRLSCIATGKVFSIYDMGWYRQAPGKQRELVAEITSSGTTHYDDFVSGRFTISRDNAKNTVYLQMNTLKAEDTAVYYCRANHVFGGSYWGQGTQVTVSSGGGSGGGSGGGSGGGSQVQLVESGGGLVQPGGSLRLSCEASGFTLDYYAIGWFRQAPGKEREGVICISRSDGSTYYADSVKGRFTISRDNAKKTVYLQMISLKPEDTAAYYCAAGADCSGYLRDYEFRGQGTQVTVSSTSTTTPAPRPPTPAPTIASQPLSLRPEACRPAAGGAVHTRGLDFACDIYIWAPLAGTCGVLLLSLVITLYCKRGRKKLLYIFKQPFMRPVQTTQEEDGCSCRFPEEEEGGCELRVKFSRSADAPAYQQGQNQLYNELNLGRREEYDVLDKRRGRDPEMGGKPRRKNPQEGLYNELQKDKMAEAYSEIGMKGERRRGKGHDGLYQGLSTATKDTYDALHMQALPPR

SEQ ID NO: 210 - protein, 508 aa, Artificial Sequence
  CD38xBCMA 38A37717 269A37346 GSI5004 CAR
MALPVTALLLPLALLLHAARPEVQLVESGGGLVQAGGSLRLSCIATGKVFSIYDMGWYRQAPGKQRELVAEITSSGTTHYDDFVSGRFTISRDNAKNTVYLQMNTLKAEDTAVYYCRANHVFGGSYWGQGTQVTVSSGGGGSGGGGSGGGGGGSGSGGGGSQVQLVESGGGLVQPGGSLRLSCEASGFTLDYYAIGWFRQAPGKEREGVICISRSDGSTYYADSVKGRFTISRDNAKKTVYLQMISLKPEDTAAYYCAAGADCSGYLRDYEFRGQGTQVTVSSTSTTTPAPRPPTPAPTIASQPLSLRPEACRPAAGGAVHTRGLDFACDIYIWAPLAGTCGVLLLSLVITLYCKRGRKKLLYIFKQPFMRPVQTTQEEDGCSCRFPEEEEGGCELRVKFSRSADAPAYQQGQNQLYNELNLGRREEYDVLDKRRGRDPEMGGKPRRKNPQEGLYNELQKDKMAEAYSEIGMKGERRRGKGHDGLYQGLSTATKDTYDALHMQALPPR

SEQ ID NO: 211 - protein, 518 aa, Artificial Sequence
  CD38xBCMA 38A37717 269A37346 GSI5005 CAR
MALPVTALLLPLALLLHAARPEVQLVESGGGLVQAGGSLRLSCIATGKVFSIYDMGWYRQAPGKQRELVAEITSSGTTHYDDFVSGRFTISRDNAKNTVYLQMNTLKAEDTAVYYCRANHVFGGSYWGQGTQVTVSSGGGGSGGGGSGGGGGGSGSGGGGSGGGGSGGGGSQVQLVESGGGLVQPGGSLRLSCEASGFTLDYYAIGWFRQAPGKEREGVICISRSDGSTYYADSVKGRFTISRDNAKKTVYLQMISLKPEDTAAYYCAAGADCSGYLRDYEFRGQGTQVTVSSTSTTTPAPRPPTPAPTIASQPLSLRPEACRPAAGGAVHTRGLDFACDIYIWAPLAGTCGVLLLSLVITLYCKRGRKKLLYIFKQPFMRPVQTTQEEDGCSCRFPEEEEGGCELRVKFSRSADAPAYQQGQNQLYNELNLGRREEYDVLDKRRGRDPEMGGKPRRKNPQEGLYNELQKDKMAEAYSEIGMKGERRRGKGHDGLYQGLSTATKDTYDALHMQALPPR

SEQ ID NO: 212 - protein, 489 aa, Artificial Sequence
  BCMAxCD38 269A37346 38A37717 GSI5006 CAR
MALPVTALLLPLALLLHAARPQVQLVESGGGLVQPGGSLRLSCEASGFTLDYYAIGWFRQAPGKEREGVICISRSDGSTYYADSVKGRFTISRDNAKKTVYLQMISLKPEDTAAYYCAAGADCSGYLRDYEFRGQGTQVTVSSGGGGSEVQLVESGGGLVQAGGSLRLSCIATGKVFSIYDMGWYRQAPGKQRELVAEITSSGTTHYDDFVSGRFTISRDNAKNTVYLQMNTLKAEDTAVYYCRANHVFGGSYWGQGTQVTVSSTSTTTPAPRPPTPAPTIASQPLSLRPEACRPAAGGAVHTRGLDFACDIYIWAPLAGTCGVLLLSLVITLYCKRGRKKLLYIFKQPFMRPVQTTQEEDGCSCRFPEEEEGGCELRVKFSRSADAPAYQQGQNQLYNELNLGRREEYDVLDKRRGRDPEMGGKPRRKNPQEGLYNELQKDKMAEAYSEIGMKGERRRGKGHDGLYQGLSTATKDTYDALHMQALPPR

SEQ ID NO: 213 - protein, 494 aa, Artificial Sequence
  BCMAxCD38 269A37346 38A37717 GSI5007 CAR
MALPVTALLLPLALLLHAARPQVQLVESGGGLVQPGGSLRLSCEASGFTLDYYAIGWFRQAPGKEREGVICISRSDGSTYYADSVKGRFTISRDNAKKTVYLQMISLKPEDTAAYYCAAGADCSGYLRDYEFRGQGTQVTVSSGGGGSGGGGSEVQLVESGGGLVQAGGSLRLSCIATGKVFSIYDMGWYRQAPGKQRELVAEITSSGTTHYDDFVSGRFTISRDNAKNTVYLQMNTLKAEDTAVYYCRANHVFGGSYWGQGTQVTVSSTSTTTPAPRPPTPAPTIASQPLSLRPEACRPAAGGAVHTRGLDFACDIYIWAPLAGTCGVLLLSLVITLYCKRGRKKLLYIFKQPFMRPVQTTQEEDGCSCRFPEEEEGGCELRVKFSRSADAPAYQQGQNQLYNELNLGRREEYDVLDKRRGRDPEMGGKPRRKNPQEGLYNELQKDKMAEAYSEIGMKGERRRGKGHDGLYQGLSTATKDTYDALHMQALPPR

SEQ ID NO: 214 - protein, 500 aa, Artificial Sequence
  BCMAxCD38 269A37346 38A37717 GSI5008 CAR
MALPVTALLLPLALLLHAARPQVQLVESGGGLVQPGGSLRLSCEASGFTLDYYAIGWFRQAPGKEREGVICISRSDGSTYYADSVKGRFTISRDNAKKTVYLQMISLKPEDTAAYYCAAGADCSGYLRDYEFRGQGTQVTVSSGGGSGGGSGGGSGGGSEVQLVESGGGLVQAGGSLRLSCIATGKVFSIYDMGWYRQAPGKQRELVAEITSSGTTHYDDFVSGRFTISRDNAKNTVYLQMNTLKAEDTAVYYCRANHVFGGSYWGQGTQVTVSSTSTTTPAPRPPTPAPTIASQPLSLRPEACRPAAGGAVHTRGLDFACDIYIWAPLAGTCGVLLLSLVITLYCKRGRKKLLYIFKQPFMRPVQTTQEEDGCSCRFPEEEEGGCELRVKFSRSADAPAYQQGQNQLYNELNLGRREEYDVLDKRRGRDPEMGGKPRRKNPQEGLYNELQKDKMAEAYSEIGMKGERRRGKGHDGLYQGLSTATKDTYDALHMQALPPR

SEQ ID NO: 215 - protein, 510 aa, Artificial Sequence
  BCMAxCD38 269A37346 38A37717 GSI5009 CAR
MALPVTALLLPLALLLHAARPQVQLVESGGGLVQPGGSLRLSCEASGFTLDYYAIGWFRQAPGKEREGVICISRSDGSTYYADSVKGRFTISRDNAKKTVYLQMISLKPEDTAAYYCAAGADCSGYLRDYEFRGQGTQVTVSSGGGGSGGGGSGGGGGGSGSGGGGSEVQLVESGGGLVQAGGSLRLSCIATGKVFSIYDMGWYRQAPGKQRELVAEITSSGTTHYDDFVSGRFTISRDNAKNTVYLQMNTLKAEDTAVYYCRANHVFGGSYWGQGTQVTVSSTSTSTTTPAPRPPTPAPTIASQPLSLRPEACRPAAGGAVHTRGLDFACDIYIWAPLAGTCGVLLLSLVITLYCKRGRKKLLYIFKQPFMRPVQTTQEEDGCSCRFPEEEEGGCELRVKFSRSADAPAYQQGQNQLYNELNLGRREEYDVLDKRRGRDPEMGGKPRRKNPQEGLYNELQKDKMAEAYSEIGMKGERRRGKGHDGLYQGLSTATKDTYDALHMQALPPR

SEQ ID NO: 216 - protein, 518 aa, Artificial Sequence
  BCMAxCD38 269A37346 38A37717 GSI5010 CAR
MALPVTALLLPLALLLHAARPQVQLVESGGGLVQPGGSLRLSCEASGFTLDYYAIGWFRQAPGKEREGVICISRSDGSTYYADSVKGRFTISRDNAKKTVYLQMISLKPEDTAAYYCAAGADCSGYLRDYEFRGQGTQVTVSSGGGGSGGGGSGGGGGGSGSGGGGSGGGGSGGGGSEVQLVESGGGLVQAGGSLRLSCIATGKVFSIYDMGWYRQAPGKQRELVAEITSSGTTHYDDFVSGRFTISRDNAKNTVYLQMNTLKAEDTAVYYCRANHVFGGSYWGQGTQVTVSSTSTTTPAPRPPTPAPTIASQPLSLRPEACRPAAGGAVHTRGLDFACDIYIWAPLAGTCGVLLLSLVITLYCKRGRKKLLYIFKQPFMRPVQTTQEEDGCSCRFPEEEEGGCELRVKFSRSADAPAYQQGQNQLYNELNLGRREEYDVLDKRRGRDPEMGGKPRRKNPQEGLYNELQKDKMAEAYSEIGMKGERRRGKGHDGLYQGLSTATKDTYDALHMQALPPR

SEQ ID NO: 217 - DNA, 1521 bp, Artificial Sequence
  CD19XCD20 single-domain antibody-based bispecific CAR
gccgccaccatggccttaccagtgaccgccttgctcctgccgctggccttgctgctccacgccgccaggccgcaggtaaagctggaggagtctgggggagaattggtgcagcctggggggcctctgagactctcctgtgcagcctcgggaaacatcttcagtatcaatcgcatgggctggtaccgccaggctccagggaagcagcgcgcgttcgtcgcatctattactgttcgtggtataacaaactatgcagactccgtgaagggccgattcaccatttctgtagacaagtccaaaaacacgatttatctgcagatgaacgcactcaaacctgaggacacggccgtctattattgtaatgcagtgtcttcaaacagggaccccgactactggggccaggggacccaggtcaccgtctcctcaggcggcggcagcggcggcggcagcggcggcggcagcggcggcggcagcccggtgcagctggtggagtctgggggaggcttggtgcaggctggggattctctgagactctcctgtgctgcctctggacgcaccttcggtattggtaccatgggctggttccgccaacctccagggaaggagcgtgaatttgtagcagctattaggtggagtactggtggcactcgctatgcagactccgtgaagggccgattcaccatctcccgagacaacgccaagctcacggtagatctgcaaatggacagcctgaaacctgaagacacggccgtttattactgtgcagcagatagactgtcccttgatttaagtggtcgttaccactacaaccccgccgtgtatgactattggggccaggggacccaggtcaccgtctcctcaattgaagttatgtatcctcctccttacctagacaatgagaagagcaatggaaccattatccatgtgaaagggaaacacctttgtccaagtcccctatttcccggaccttctaagcccttttgggtgctggtggtggttggtggagtcctggcttgctatagcttgctagtaacagtggcctttattattttctgggtgaggagtaagaggagcaggctcctgcacagtgactacatgaacatgactccccgccgccccgggcccacccgcaagcattaccagccctatgccccaccacgcgacttcgcagcctatcgctccagagtgaagttcagcaggagcgcagacgcccccgcgtaccagcagggccagaaccagctctataacgagctcaatctaggacgaagagaggagtacgatgttttggacaagagacgtggccgggaccctgagatggggggaaagccgagaaggaagaaccctcaggaaggcctgtacaatgaactgcagaaagataagatggcggaggcctacagtgagattgggatgaaaggcgagcgccggaggggcaaggggcacgatggcctttaccagggtctcagtacagccaccaaggacacctacgacgcccttcacatgcaggccctgccccctcgctgataa

SEQ ID NO: 218 - DNA, 1470 bp, Artificial Sequence
  CD38xBCMA 38A37717 269A37346 GSI5001 CAR
atggctctgcccgtcactgctctgctgctgcccctggctctgctgctgcacgccgcaagacccgaagtccagctggtggaatctggcggaggcctggtgcaggcaggaggcagcctgaggctgtcctgcatcgccaccggcaaggtgttctccatctacgacatgggctggtatcggcaggccccaggcaagcagagagagctggtggccgagatcacaagctccggcaccacacactacgacgatttcgtgtctggccggtttaccatcagcagagacaacgccaagaatacagtgtatctgcagatgaacaccctgaaggccgaggatacagccgtgtactattgtcgggccaatcacgtgtttggaggaagctactggggacagggaacccaggtgacagtgtctagcggaggaggaggcagccaggtgcagctggtggagtccggaggaggcctggtgcagccaggaggctctctgaggctgagctgcgaggcatccggattcaccctggactactatgccatcggctggtttaggcaggcacctggaaaggagagggagggagtgatctgtatctccagatctgacggctccacatactatgccgattctgtgaagggcaggttcaccatctctcgcgataacgccaagaagacagtctacctgcagatgatcagcctgaagcccgaggacaccgcagcatactattgcgcagcaggagcagattgtagtggctatctgagggactacgagttccgagggcaggggacacaggtgaccgtgagcagcactagtaccacgacgccagcgccgcgaccaccaacaccggcgcccaccatcgcgtcgcagcccctgtccctgcgcccagaggcgtgccggccagcggcggggggcgcagtgcacacgagggggctggacttcgcctgtgatatctacatctgggcgcccttggccgggacttgtggggtccttctcctgtcactggttatcaccctttactgcaaacggggcagaaagaaactcctgtatatattcaaacaaccatttatgagaccagtacaaactactcaagaggaagatggctgtagctgccgatttccagaagaagaagaaggaggatgtgaactgagagtgaagttcagcaggagcgcagacgcccccgcgtaccagcagggccagaaccagctctataacgagctcaatctaggacgaagagaggagtacgatgttttggacaagagacgtggccgggaccctgagatggggggaaagccgagaaggaagaaccctcaggaaggcctgtacaatgaactgcagaaagataagatggcggaggcctacagtgagattgggatgaaaggcgagcgccggaggggcaaggggcacgatggcctttaccagggtctcagtacagccaccaaggacacctacgacgcccttcacatgcaggccctgccccctcgctaa

SEQ ID NO: 219 - DNA, 1485 bp, Artificial Sequence
  CD38xBCMA 38A37717 269A37346 GSI5002 CAR
atggctctgcccgtcactgctctgctgctgcccctggctctgctgctgcacgctgctcgccctgaagtccagctggtcgaatccggcggaggcctggtgcaggcaggaggcagcctgaggctgtcctgcatcgccaccggcaaggtgttctccatctacgacatgggctggtatcggcaggccccaggcaagcagagagagctggtggccgagatcacaagctccggcaccacacactacgacgatttcgtgtccggccggtttaccatctctagagacaacgccaagaatacagtgtatctgcagatgaacaccctgaaggccgaggatacagccgtgtactattgtcgggccaatcacgtgtttggaggatcctactggggacagggaacccaggtgacagtgtctagcggaggaggaggatctggcggaggaggcagccaggtgcagctggtggagtctggaggaggcctggtgcagccaggaggctctctgaggctgagctgcgaggcatccggattcaccctggactactatgccatcggctggtttaggcaggcacctggaaaggagagggagggagtgatctgtatctccagatctgacggcagcacatactatgccgattccgtgaagggcaggttcaccatctctcgcgataacgccaagaagacagtctacctgcagatgatcagcctgaagcccgaggacaccgcagcatactattgcgcagcaggagcagattgtagcggctatctgagggattatgagtttagagggcagggaacacaggtgacagtgagcagcactagtaccacgacgccagcgccgcgaccaccaacaccggcgcccaccatcgcgtcgcagcccctgtccctgcgcccagaggcgtgccggccagcggcggggggcgcagtgcacacgagggggctggacttcgcctgtgatatctacatctgggcgcccttggccgggacttgtggggtccttctcctgtcactggttatcaccctttactgcaaacggggcagaaagaaactcctgtatatattcaaacaaccatttatgagaccagtacaaactactcaagaggaagatggctgtagctgccgatttccagaagaagaagaaggaggatgtgaactgagagtgaagttcagcaggagcgcagacgcccccgcgtaccagcagggccagaaccagctctataacgagctcaatctaggacgaagagaggagtacgatgttttggacaagagacgtggccgggaccctgagatggggggaaagccgagaaggaagaaccctcaggaaggcctgtacaatgaactgcagaaagataagatggcggaggcctacagtgagattgggatgaaaggcgagcgccggaggggcaaggggcacgatggcctttaccagggtctcagtacagccaccaaggacacctacgacgcccttcacatgcaggccctgccccctcgctaa

SEQ ID NO: 220 - DNA, 1503 bp, Artificial Sequence
  CD38xBCMA 38A37717 269A37346 GSI5003 CAR
atggccctgcctgtcaccgcactgctgctgcccctggctctgctgctgcacgccgcacgccctgaagtccagctggtcgagtccgggggaggcctggtgcaggcaggaggcagcctgaggctgtcctgcatcgccaccggcaaggtgttctccatctacgacatgggctggtatcggcaggccccaggcaagcagagagagctggtggccgagatcacaagctccggcaccacacactacgacgatttcgtgagcggccggtttaccatctccagagacaacgccaagaatacagtgtatctgcagatgaacaccctgaaggccgaggatacagccgtgtactattgtcgggccaatcacgtgtttggaggatcctactggggacagggaacccaggtgacagtgtctagcggcggcggctctggaggaggaagcggaggaggatctggaggaggctctcaggtgcagctggtggagagcggaggaggcctggtgcagccaggaggcagcctgcggctgtcctgcgaggcctctggcttcaccctggactactatgccatcggctggtttaggcaggcacctggaaaggagagggagggagtgatctgtatctccagatctgacggctctacatactatgccgatagcgtgaagggcaggttcaccatctcccgcgataacgccaagaagacagtctacctgcagatgatctctctgaagcccgaggacaccgcagcatactattgcgcagcaggagcagattgtagcgggtatctgcgggattatgagtttagaggacaggggacacaggtcacagtcagttccactagtaccacgacgccagcgccgcgaccaccaacaccggcgcccaccatcgcgtcgcagcccctgtccctgcgcccagaggcgtgccggccagcggcggggggcgcagtgcacacgagggggctggacttcgcctgtgatatctacatctgggcgcccttggccgggacttgtggggtccttctcctgtcactggttatcaccctttactgcaaacggggcagaaagaaactcctgtatatattcaaacaaccatttatgagaccagtacaaactactcaagaggaagatggctgtagctgccgatttccagaagaagaagaaggaggatgtgaactgagagtgaagttcagcaggagcgcagacgcccccgcgtaccagcagggccagaaccagctctataacgagctcaatctaggacgaagagaggagtacgatgttttggacaagagacgtggccgggaccctgagatggggggaaagccgagaaggaagaaccctcaggaaggcctgtacaatgaactgcagaaagataagatggcggaggcctacagtgagattgggatgaaaggcgagcgccggaggggcaaggggcacgatggcctttaccagggtctcagtacagccaccaaggacacctacgacgcccttcacatgcaggccctgccccctcgctaa

SEQ ID NO: 221 - DNA, 1527 bp, Artificial Sequence
  CD38xBCMA 38A37717 269A37346 GSI5004 CAR
atggctctgcctgtgaccgccctgctgctgcccctggctctgctgctgcacgccgcacgacccgaagtccagctggtggaatctgggggaggcctggtgcaggcaggaggctctctgaggctgagctgcatcgccaccggcaaggtgttctctatctacgacatgggctggtatcggcaggccccaggcaagcagagagagctggtggccgagatcacaagctccggcaccacacactacgacgatttcgtgagcggccggtttaccatctccagagacaacgccaagaatacagtgtatctgcagatgaacaccctgaaggccgaggatacagccgtgtactattgtcgggccaatcacgtgtttggaggaagctactggggacagggaacccaggtgacagtgtctagcggaggaggaggatccggaggaggaggatctggaggcggcggcggcggctccggctctggcggcggcggctcccaggtgcagctggtggagtctggaggaggcctggtgcagccaggaggctccctgcggctgtcttgcgaggccagcggcttcaccctggactactatgccatcggctggtttaggcaggcacctggaaaggagagggagggagtgatctgtatcagcagatccgacggctctacatactatgccgatagcgtgaagggcaggttcaccatcagccgcgataacgccaagaagacagtctacctgcagatgatctccctgaagcccgaggacaccgcagcatactattgcgcagcaggagcagattgtagcggctatctgcgggattacgagtttagaggacagggcacccaggtcaccgtctcaagcactagtaccacgacgccagcgccgcgaccaccaacaccggcgcccaccatcgcgtcgcagcccctgtccctgcgcccagaggcgtgccggccagcggcggggggcgcagtgcacacgagggggctggacttcgcctgtgatatctacatctgggcgcccttggccgggacttgtggggtccttctcctgtcactggttatcaccctttactgcaaacggggcagaaagaaactcctgtatatattcaaacaaccatttatgagaccagtacaaactactcaagaggaagatggctgtagctgccgatttccagaagaagaagaaggaggatgtgaactgagagtgaagttcagcaggagcgcagacgcccccgcgtaccagcagggccagaaccagctctataacgagctcaatctaggacgaagagaggagtacgatgttttggacaagagacgtggccgggaccctgagatggggggaaagccgagaaggaagaaccctcaggaaggcctgtacaatgaactgcagaaagataagatggcggaggcctacagtgagattgggatgaaaggcgagcgccggaggggcaaggggcacgatggcctttaccagggtctcagtacagccaccaaggacacctacgacgcccttcacatgcaggccctgccccctcgctaa

SEQ ID NO: 222 - DNA, 1557 bp, Artificial Sequence
  CD38xBCMA 38A37717 269A37346 GSI5005 CAR
atggctctgcctgtcactgctctgctgctgcccctggccctgctgctgcacgctgctagacccgaagtccagctggtggagtccggcggaggcctggtgcaggcaggaggctctctgaggctgagctgcatcgccaccggcaaggtgttcagcatctacgacatgggctggtatcggcaggccccaggcaagcagagagagctggtggccgagatcacaagctccggcaccacacactacgacgatttcgtgagcggccggtttaccatctccagagacaacgccaagaatacagtgtatctgcagatgaacaccctgaaggccgaggatacagccgtgtactattgtcgggccaatcacgtgtttggaggaagctactggggacagggaacccaggtgacagtgtctagcggaggaggaggatccggaggaggaggatctggaggcggcggcggcggctccggctctggcggcggcggcagtggaggcggcggctccggcggcggcggctctcaggtgcagctggtggagtccggaggaggcctggtgcagccaggaggctccctgcggctgtcttgcgaggccagcggcttcaccctggactactatgccatcggctggtttaggcaggcacctggaaaggagagggagggagtgatctgtatcagcagatccgacggctctacatactatgccgatagcgtgaagggcaggttcaccatctcccgcgataacgccaagaagacagtctacctgcagatgatctctctgaagcccgaggacaccgcagcatactattgcgcagcaggagcagattgttcaggctatctgcgggattatgagtttcggggacaggggacacaggtcacagtctccagcactagtaccacgacgccagcgccgcgaccaccaacaccggcgcccaccatcgcgtcgcagcccctgtccctgcgcccagaggcgtgccggccagcggcggggggcgcagtgcacacgagggggctggacttcgcctgtgatatctacatctgggcgcccttggccgggacttgtggggtccttctcctgtcactggttatcaccctttactgcaaacggggcagaaagaaactcctgtatatattcaaacaaccatttatgagaccagtacaaactactcaagaggaagatggctgtagctgccgatttccagaagaagaagaaggaggatgtgaactgagagtgaagttcagcaggagcgcagacgcccccgcgtaccagcagggccagaaccagctctataacgagctcaatctaggacgaagagaggagtacgatgttttggacaagagacgtggccgggaccctgagatggggggaaagccgagaaggaagaaccctcaggaaggcctgtacaatgaactgcagaaagataagatggcggaggcctacagtgagattgggatgaaaggcgagcgccggaggggcaaggggcacgatggcctttaccagggtctcagtacagccaccaaggacacctacgacgcccttcacatgcaggccctgccccctcgctaa

SEQ ID NO: 223 - DNA, 1470 bp, Artificial Sequence
  BCMAxCD38 269A37346 38A37717 GSI5006 CAR
atggctctgcccgtcaccgctctgctgctgcctctggctctgctgctgcacgccgcccgccctcaggtccagctggtcgagtcaggaggaggcctggtgcagccaggaggcagcctgaggctgtcctgcgaggcctctggcttcaccctggactactatgccatcggctggtttaggcaggcacctggaaaggagagggagggagtgatctgtatctcccgctctgacggctctacatactatgccgatagcgtgaagggccggttcaccatctctagagacaacgccaagaagacagtgtacctgcagatgatcagcctgaagccagaggataccgcagcatactattgcgcagcaggagcagactgttccggatacctgagggattatgagtttaggggacagggaacccaggtgacagtgagctccggcggcggcggcagcgaggtgcagctggtggagtccggaggaggcctggtgcaggcaggaggcagcctgcggctgtcctgcatcgccaccggcaaggtgttcagcatctacgatatgggatggtataggcaggcaccaggaaagcagagagagctggtggccgagatcacatctagcggcaccacacactacgacgatttcgtgtccggccggtttactatttccagggacaacgccaagaatacagtgtatctgcagatgaataccctgaaggccgaggatacagccgtgtactattgtagagcaaatcatgtcttcggggggtcctattgggggcagggcactcaggtcaccgtctcctcaactagtaccacgacgccagcgccgcgaccaccaacaccggcgcccaccatcgcgtcgcagcccctgtccctgcgcccagaggcgtgccggccagcggcggggggcgcagtgcacacgagggggctggacttcgcctgtgatatctacatctgggcgcccttggccgggacttgtggggtccttctcctgtcactggttatcaccctttactgcaaacggggcagaaagaaactcctgtatatattcaaacaaccatttatgagaccagtacaaactactcaagaggaagatggctgtagctgccgatttccagaagaagaagaaggaggatgtgaactgagagtgaagttcagcaggagcgcagacgcccccgcgtaccagcagggccagaaccagctctataacgagctcaatctaggacgaagagaggagtacgatgttttggacaagagacgtggccgggaccctgagatggggggaaagccgagaaggaagaaccctcaggaaggcctgtacaatgaactgcagaaagataagatggcggaggcctacagtgagattgggatgaaaggcgagcgccggaggggcaaggggcacgatggcctttaccagggtctcagtacagccaccaaggacacctacgacgcccttcacatgcaggccctgccccctcgctaa

SEQ ID NO: 224 - DNA, 1485 bp, Artificial Sequence
  BCMAxCD38 269A37346 38A37717 GSI5007 CAR
atggctctgcccgtcactgctctgctgctgcctctggctctgctgctgcacgccgctcgcccacaggtccagctggtcgaatcagggggaggcctggtgcagccaggaggcagcctgaggctgtcctgcgaggcctctggcttcaccctggactactatgccatcggctggtttaggcaggcacctggaaaggagagggagggagtgatctgtatctcccgctctgacggctccacatactatgccgattctgtgaagggccggttcaccatctctagagacaacgccaagaagacagtgtacctgcagatgatcagcctgaagccagaggataccgcagcatactattgcgcagcaggagcagactgttccggatacctgagggattatgagtttaggggacagggaacccaggtgacagtgagctccggaggaggaggatctggcggaggaggcagcgaggtgcagctggtggagtccggcggcggcctggtgcaggccggcggcagcctgcggctgtcctgcatcgccaccggcaaggtgttctctatctacgatatgggatggtataggcaggcaccaggaaagcagagagagctggtggccgagatcacatctagcggcaccacacactacgacgatttcgtgagcggccggtttaccatctccagagacaacgccaagaatacagtgtatctgcagatgaataccctgaaggccgaggatacagccgtgtactattgtagagccaaccatgtcttcggcgggtcatactgggggcagggaactcaggtcactgtcagcagcactagtaccacgacgccagcgccgcgaccaccaacaccggcgcccaccatcgcgtcgcagcccctgtccctgcgcccagaggcgtgccggccagcggcggggggcgcagtgcacacgagggggctggacttcgcctgtgatatctacatctgggcgcccttggccgggacttgtggggtccttctcctgtcactggttatcaccctttactgcaaacggggcagaaagaaactcctgtatatattcaaacaaccatttatgagaccagtacaaactactcaagaggaagatggctgtagctgccgatttccagaagaagaagaaggaggatgtgaactgagagtgaagttcagcaggagcgcagacgcccccgcgtaccagcagggccagaaccagctctataacgagctcaatctaggacgaagagaggagtacgatgttttggacaagagacgtggccgggaccctgagatggggggaaagccgagaaggaagaaccctcaggaaggcctgtacaatgaactgcagaaagataagatggcggaggcctacagtgagattgggatgaaaggcgagcgccggaggggcaaggggcacgatggcctttaccagggtctcagtacagccaccaaggacacctacgacgcccttcacatgcaggccctgccccctcgctaa

SEQ ID NO: 225 - DNA, 1503 bp, Artificial Sequence
  BCMAxCD38 269A37346 38A37717 GSI5008 CAR
atggctctgcccgtcactgctctgctgctgcctctggctctgctgctgcacgccgcaaggcctcaggtccagctggtcgaatcagggggaggcctggtgcagccaggaggcagcctgaggctgtcctgcgaggcctctggcttcaccctggactactatgccatcggctggtttaggcaggcacctggaaaggagagggagggagtgatctgtatctcccgctctgacggcagcacatactatgccgattccgtgaagggccggttcaccatctccagagacaacgccaagaagacagtgtacctgcagatgatctctctgaagccagaggataccgcagcatactattgcgcagcaggagcagactgttccggatacctgagggattatgagtttaggggacagggaacccaggtgacagtgagctccggaggaggaagcggaggaggatccggaggcggctctggcggcggcagcgaggtgcagctggtggagtccggcggcggcctggtgcaggccggcggctccctgcggctgtcttgcatcgccaccggcaaggtgttcagcatctacgatatgggatggtataggcaggcaccaggaaagcagagagagctggtggccgagatcacatctagcggcaccacacactacgacgatttcgtgtctggccggtttaccatcagtagggacaacgccaagaatacagtgtatctgcagatgaataccctgaaggccgaggatacagccgtgtactattgtagagctaaccatgtcttcggggggtcatactgggggcagggcactcaggtcactgtctcatccactagtaccacgacgccagcgccgcgaccaccaacaccggcgcccaccatcgcgtcgcagcccctgtccctgcgcccagaggcgtgccggccagcggcggggggcgcagtgcacacgagggggctggacttcgcctgtgatatctacatctgggcgcccttggccgggacttgtggggtccttctcctgtcactggttatcaccctttactgcaaacggggcagaaagaaactcctgtatatattcaaacaaccatttatgagaccagtacaaactactcaagaggaagatggctgtagctgccgatttccagaagaagaagaaggaggatgtgaactgagagtgaagttcagcaggagcgcagacgcccccgcgtaccagcagggccagaaccagctctataacgagctcaatctaggacgaagagaggagtacgatgttttggacaagagacgtggccgggaccctgagatggggggaaagccgagaaggaagaaccctcaggaaggcctgtacaatgaactgcagaaagataagatggcggaggcctacagtgagattgggatgaaaggcgagcgccggaggggcaaggggcacgatggcctttaccagggtctcagtacagccaccaaggacacctacgacgcccttcacatgcaggccctgccccctcgctaa

SEQ ID NO: 226 - DNA, 1533 bp, Artificial Sequence
  BCMAxCD38 269A37346 38A37717 GSI5009 CAR
atggctctgcccgtcaccgcactgctgctgcctctggctctgctgctgcacgccgcaaggcctcaggtccagctggtcgaatcagggggaggcctggtgcagccaggaggctctctgaggctgagctgcgaggcatccggattcaccctggactactatgccatcggctggtttaggcaggcacctggaaaggagagggagggagtgatctgtatctcccgctctgacggcagcacatactatgccgattccgtgaagggccggttcaccatcagcagagacaacgccaagaagacagtgtacctgcagatgatctccctgaagccagaggataccgcagcatactattgcgcagcaggagcagactgttctggatacctgagggattatgagtttaggggacagggaacccaggtgacagtgagctccggaggaggaggatccggcggaggaggctctggcggcggcggcggcggcagcggctccggcggcggcggctccgaggtgcagctggtggagtctggaggaggcctggtgcaggcaggaggctctctgcggctgagctgcatcgccaccggcaaggtgttcagcatctacgatatgggatggtataggcaggcaccaggaaagcagagagagctggtggccgagatcacatctagcggcaccacacactacgacgatttcgtgtctggccggtttactatttccagggacaacgccaagaatacagtgtatctgcagatgaataccctgaaggccgaggatacagccgtgtactattgtagagctaatcacgtcttcggcggctcttattgggggcagggaactcaggtcactgtgtcatccactagtactagtaccacgacgccagcgccgcgaccaccaacaccggcgcccaccatcgcgtcgcagcccctgtccctgcgcccagaggcgtgccggccagcggcggggggcgcagtgcacacgagggggctggacttcgcctgtgatatctacatctgggcgcccttggccgggacttgtggggtccttctcctgtcactggttatcaccctttactgcaaacggggcagaaagaaactcctgtatatattcaaacaaccatttatgagaccagtacaaactactcaagaggaagatggctgtagctgccgatttccagaagaagaagaaggaggatgtgaactgagagtgaagttcagcaggagcgcagacgcccccgcgtaccagcagggccagaaccagctctataacgagctcaatctaggacgaagagaggagtacgatgttttggacaagagacgtggccgggaccctgagatggggggaaagccgagaaggaagaaccctcaggaaggcctgtacaatgaactgcagaaagataagatggcggaggcctacagtgagattgggatgaaaggcgagcgccggaggggcaaggggcacgatggcctttaccagggtctcagtacagccaccaaggacacctacgacgcccttcacatgcaggccctgccccctcgctaa

SEQ ID NO: 227 - DNA, 1557 bp, Artificial Sequence
  BCMAxCD38 269A37346 38A37717 GSI5010 CAR
atggctctgcccgtcaccgctctgctgctgcccctggctctgctgctgcacgctgctcgccctcaggtccagctggtcgaatcaggaggaggcctggtgcagccaggaggctctctgaggctgagctgcgaggcatccggattcaccctggactactatgccatcggctggtttaggcaggcacctggaaaggagagggagggagtgatctgtatctcccgctctgacggcagcacatactatgccgattccgtgaagggccggttcaccatctccagagacaacgccaagaagacagtgtacctgcagatgatctctctgaagccagaggataccgcagcatactattgcgcagcaggagcagactgtagcggatacctgagggattatgagtttaggggacagggaacccaggtgacagtgagctccggaggaggaggatccggcggaggaggctctggaggcggcggcggcggcagcggctcaggaggcggaggaagcggcggcggcggctccggcggcggcggctctgaggtgcagctggtggagagcggaggaggcctggtgcaggcaggaggctctctgcggctgagctgcatcgccaccggcaaggtgttctccatctacgatatgggatggtataggcaggcaccaggaaagcagagagagctggtggccgagatcacatctagcggcaccacacactacgacgatttcgtgtctggccggtttaccatcagtagggacaacgccaagaatacagtgtatctgcagatgaataccctgaaggccgaggatacagccgtgtactattgtagagctaatcatgtgtttggagggtcatactgggggcagggaactcaggtcactgtctcatcaactagtaccacgacgccagcgccgcgaccaccaacaccggcgcccaccatcgcgtcgcagcccctgtccctgcgcccagaggcgtgccggccagcggcggggggcgcagtgcacacgagggggctggacttcgcctgtgatatctacatctgggcgcccttggccgggacttgtggggtccttctcctgtcactggttatcaccctttactgcaaacggggcagaaagaaactcctgtatatattcaaacaaccatttatgagaccagtacaaactactcaagaggaagatggctgtagctgccgatttccagaagaagaagaaggaggatgtgaactgagagtgaagttcagcaggagcgcagacgcccccgcgtaccagcagggccagaaccagctctataacgagctcaatctaggacgaagagaggagtacgatgttttggacaagagacgtggccgggaccctgagatggggggaaagccgagaaggaagaaccctcaggaaggcctgtacaatgaactgcagaaagataagatggcggaggcctacagtgagattgggatgaaaggcgagcgccggaggggcaaggggcacgatggcctttaccagggtctcagtacagccaccaaggacacctacgacgcccttcacatgcaggccctgccccctcgctaa

SEQ ID NO: 228 - DNA, 663 bp, Artificial Sequence
  CD28 TM and CD28-CD3 zeta intracellular signaling domain
attgaagttatgtatcctcctccttacctagacaatgagaagagcaatggaaccattatccatgtgaaagggaaacacctttgtccaagtcccctatttcccggaccttctaagcccttttgggtgctggtggtggttggtggagtcctggcttgctatagcttgctagtaacagtggcctttattattttctgggtgaggagtaagaggagcaggctcctgcacagtgactacatgaacatgactccccgccgccccgggcccacccgcaagcattaccagccctatgccccaccacgcgacttcgcagcctatcgctccagagtgaagttcagcaggagcgcagacgcccccgcgtaccagcagggccagaaccagctctataacgagctcaatctaggacgaagagaggagtacgatgttttggacaagagacgtggccgggaccctgagatggggggaaagccgagaaggaagaaccctcaggaaggcctgtacaatgaactgcagaaagataagatggcggaggcctacagtgagattgggatgaaaggcgagcgccggaggggcaaggggcacgatggcctttaccagggtctcagtacagccaccaaggacacctacgacgcccttcacatgcaggccctgccccctcgctgataa

SEQ ID NO: 229 - DNA, 23 bp, Artificial Sequence
  upstream primer CALL001
gtcctggctgctcttctacaagg

SEQ ID NO: 230 - DNA, 23 bp, Artificial Sequence
  downstream primer CALLOO2
ggtacgtgctgttgaactgttcc

SEQ ID NO: 231 - DNA, 29 bp, Artificial Sequence
  upstream primer BACK-1
gatgtgcagctgcaggagtctggaggagg

SEQ ID NO: 232 - DNA, 29 bp, Artificial Sequence
  downstream primer BACK-2
gatgtgcagctgcaggagtctgggggagg

SEQ ID NO: 233 - DNA, 34 bp, Artificial Sequence
  downstream primer PMCF
ctagtgcggccgctgaggagacggtgacctgggt

SEQ ID NO: 234 - DNA, 6 bp, Artificial Sequence
  EcoRI restriction site
gaattc

SEQ ID NO: 235 - DNA, 6 bp, Artificial Sequence
  SpeI restriction site
actagt

SEQ ID NO: 236 - DNA, 6 bp, Artificial Sequence
  HpaI restriction site
gttaac

SEQ ID NO: 237 - DNA, 6 bp, Artificial Sequence
  MluI restriction site
acgcgt

SEQ ID NO: 238 - DNA, 6 bp, Artificial Sequence
  NsiI restriction site
atgcat

SEQ ID NO: 239 - DNA, 2307 bp, Artificial Sequence
  tandem BCMA, CD38 269A37346 38A37717 GSI5013 CAR
atggccttaccagtgaccgccttgctcctgccgctggccttgctgctccacgccgccaggccggttaacgaggtgcagctggtggaaagcggggggggactggtgcaggcaggcgggtcactgagactgtcatgtatcgcaactgggaaggtgtttagcatctacgacatgggctggtataggcaggcaccaggaaagcagagggagctggtggccgagatcaccagctccggcaccacacactacgacgatttcgtgtctggccggtttaccatcagcagagacaacgccaagaatacagtgtatctgcagatgaacaccctgaaggccgaggatacagccgtgtactattgccgggctaatcacgtcttcggcggctcctactgggggcagggaactcaggtcactgtgtcatccacgcgtcgcatgcatactagtaccacgacgccagcgccgcgaccaccaacaccggcgcccaccatcgcgtcgcagcccctgtccctgcgcccagaggcgtgccggccagcggcggggggcgcagtgcacacgagggggctggacttcgcctgtgatatctacatctgggcgcccttggccgggacttgtggggtccttctcctgtcactggttatcaccctttactgcaaacggggcagaaagaaactcctgtatatattcaaacaaccatttatgagaccagtacaaactactcaagaggaagatggctgtagctgccgatttccagaagaagaagaaggaggatgtgaactgagagtgaagttcagcaggagcgcagacgcccccgcgtaccagcagggccagaaccagctctataacgagctcaatctaggacgaagagaggagtacgatgttttggacaagagacgtggccgggaccctgagatggggggaaagccgagaaggaagaaccctcaggaaggcctgtacaatgaactgcagaaagataagatggcggaggcctacagtgagattgggatgaaaggcgagcgccggaggggcaaggggcacgatggcctttaccagggtctcagtacagccaccaaggacacctacgacgcccttcacatgcaggccctgccccctcgcggcagtggagagggcagaggaagtctgctaacatgcggtgacgtcgaggagaatcctggcccaggatccatggccttaccagtgaccgccttgctcctgccgctggccttgctgctccacgccgccaggccggttaaccgcacgcgtcgcatgcatcaggtgcagctggtggagtctgggggaggcttggtgcagcctgggggttctctgaggctctcctgtgaagcctctggattcactttggattattatgccataggctggttccgccaggccccagggaaggagcgcgagggggtcatatgtattagtagaagtgatggtagcacatactatgcagactccgtgaagggccgattcaccatctccagagacaacgccaagaaaacggtgtatctgcaaatgatcagcctgaaacctgaggacacggccgcttattactgtgcagcaggggccgattgttcggggtacctacgagattatgagttccgggggcaggggacccaggtcaccgtctcctcaactagtaccacgacgccagcgccgcgaccaccaacaccggcgcccaccatcgcgtcgcagcccctgtccctgcgcccagaggcgtgccggccagcggcggggggcgcagtgcacacgagggggctggacttcgcctgtgatatctacatctgggcgcccttggccgggacttgtggggtccttctcctgtcactggttatcaccctttactgcaaacggggcagaaagaaactcctgtatatattcaaacaaccatttatgagaccagtacaaactactcaagaggaagatggctgtagctgccgatttccagaagaagaagaaggaggatgtgaactgagagtgaagttcagcaggagcgcagacgcccccgcgtaccagcagggccagaaccagctctataacgagctcaatctaggacgaagagaggagtacgatgttttggacaagagacgtggccgggaccctgagatggggggaaagccgagaaggaagaaccctcaggaaggcctgtacaatgaactgcagaaagataagatggcggaggcctacagtgagattgggatgaaaggcgagcgccggaggggcaaggggcacgatggcctttaccagggtctcagtacagccaccaaggacacctacgacgcccttcacatgcaggccctgccccctcgctaa

SEQ ID NO: 240 - protein, 30 aa, Artificial Sequence
  CD19 VHH FR1
QVKLEESGGELVQPGGPLRLSCAASGNIFS

SEQ ID NO: 241 - protein, 14 aa, Artificial Sequence
  CD19 VHH FR2
WYRQAPGKQRAFVA

SEQ ID NO: 242 - protein, 32 aa, Artificial Sequence
  CD19 VHH FR3
RFTISVDKSKNTIYLQMNALKPEDTAVYYCNA

SEQ ID NO: 243 - protein, 11 aa, Artificial Sequence
  CD19 VHH FR4
WGQGTQVTVSS

SEQ ID NO: 244 - protein, 30 aa, Artificial Sequence
  CD20 VHH FR1
PVQLVESGGGLVQAGDSLRLSCAASGRTFG

SEQ ID NO: 245 - protein, 14 aa, Artificial Sequence
  CD20 VHH FR2
WFRQPPGKEREFVA

SEQ ID NO: 246 - protein, 32 aa, Artificial Sequence
  CD20 VHH FR3
RFTISRDNAKLTVDLQMDSLKPEDTAVYYCAA

SEQ ID NO: 247 - protein, 11 aa, Artificial Sequence
  CD20 VHH FR4
WGQGTQVTVSS

SEQ ID NO: 248 - protein, 357 aa, Artificial Sequence
  CD19 CAR
MALPVTALLLPLALLLHAARPQVKLEESGGELVQPGGPLRLSCAASGNIFSINRMGWYRQAPGKQRAFVASITVRGITNYADSVKGRFTISVDKSKNTIYLQMNALKPEDTAVYYCNAVSSNRDPDYWGQGTQVTVSSIEVMYPPPYLDNEKSNGTIIHVKGKHLCPSPLFPGPSKPFWVLVVVGGVLACYSLLVTVAFIIFWVRSKRSRLLHSDYMNMTPRRPGPTRKHYQPYAPPRDFAAYRSRVKFSRSADAPAYQQGQNQLYNELNLGRREEYDVLDKRRGRDPEMGGKPRRKNPQEGLYNELQKDKMAEAYSEIGMKGERRRGKGHDGLYQGLSTATKDTYDALHMQALPPR

SEQ ID NO: 249 - protein, 369 aa, Artificial Sequence
  CD20 CAR
MALPVTALLLPLALLLHAARPPVQLVESGGGLVQAGDSLRLSCAASGRTFGIGTMGWFRQPPGKEREFVAAIRWSTGGTRYADSVKGRFTISRDNAKLTVDLQMDSLKPEDTAVYYCAADRLSLDLSGRYHYNPAVYDYWGQGTQVTVSSIEVMYPPPYLDNEKSNGTIIHVKGKHLCPSPLFPGPSKPFWVLVVVGGVLACYSLLVTVAFIIFWVRSKRSRLLHSDYMNMTPRRPGPTRKHYQPYAPPRDFAAYRSRVKFSRSADAPAYQQGQNQLYNELNLGRREEYDVLDKRRGRDPEMGGKPRRKNPQEGLYNELQKDKMAEAYSEIGMKGERRRGKGHDGLYQGLSTATKDTYDALHMQALPPR

SEQ ID NO: 250 - DNA, 1077 bp, Artificial Sequence
  CD19 CAR
atggccttaccagtgaccgccttgctcctgccgctggccttgctgctccacgccgccaggccgcaggtaaagctggaggagtctgggggagaattggtgcagcctggggggcctctgagactctcctgtgcagcctcgggaaacatcttcagtatcaatcgcatgggctggtaccgccaggctccagggaagcagcgcgcgttcgtcgcatctattactgttcgtggtataacaaactatgcagactccgtgaagggccgattcaccatttctgtagacaagtccaaaaacacgatttatctgcagatgaacgcactcaaacctgaggacacggccgtctattattgtaatgcagtgtcttcaaacagggaccccgactactggggccaggggacccaggtcaccgtctcctcaattgaagttatgtatcctcctccttacctagacaatgagaagagcaatggaaccattatccatgtgaaagggaaacacctttgtccaagtcccctatttcccggaccttctaagcccttttgggtgctggtggtggttggtggagtcctggcttgctatagcttgctagtaacagtggcctttattattttctgggtgaggagtaagaggagcaggctcctgcacagtgactacatgaacatgactccccgccgccccgggcccacccgcaagcattaccagccctatgccccaccacgcgacttcgcagcctatcgctccagagtgaagttcagcaggagcgcagacgcccccgcgtaccagcagggccagaaccagctctataacgagctcaatctaggacgaagagaggagtacgatgttttggacaagagacgtggccgggaccctgagatggggggaaagccgagaaggaagaaccctcaggaaggcctgtacaatgaactgcagaaagataagatggcggaggcctacagtgagattgggatgaaaggcgagcgccggaggggcaaggggcacgatggcctttaccagggtctcagtacagccaccaaggacacctacgacgcccttcacatgcaggccctgccccctcgctgataa

SEQ ID NO: 251 - DNA, 1113 bp, Artificial Sequence
  CD20 CAR
atggccttaccagtgaccgccttgctcctgccgctggccttgctgctccacgccgccaggccgccggtgcagctggtggagtctgggggaggcttggtgcaggctggggattctctgagactctcctgtgctgcctctggacgcaccttcggtattggtaccatgggctggttccgccaacctccagggaaggagcgtgaatttgtagcagctattaggtggagtactggtggcactcgctatgcagactccgtgaagggccgattcaccatctcccgagacaacgccaagctcacggtagatctgcaaatggacagcctgaaacctgaagacacggccgtttattactgtgcagcagatagactgtcccttgatttaagtggtcgttaccactacaaccccgccgtgtatgactattggggccaggggacccaggtcaccgtctcctcaattgaagttatgtatcctcctccttacctagacaatgagaagagcaatggaaccattatccatgtgaaagggaaacacctttgtccaagtcccctatttcccggaccttctaagcccttttgggtgctggtggtggttggtggagtcctggcttgctatagcttgctagtaacagtggcctttattattttctgggtgaggagtaagaggagcaggctcctgcacagtgactacatgaacatgactccccgccgccccgggcccacccgcaagcattaccagccctatgccccaccacgcgacttcgcagcctatcgctccagagtgaagttcagcaggagcgcagacgcccccgcgtaccagcagggccagaaccagctctataacgagctcaatctaggacgaagagaggagtacgatgttttggacaagagacgtggccgggaccctgagatggggggaaagccgagaaggaagaaccctcaggaaggcctgtacaatgaactgcagaaagataagatggcggaggcctacagtgagattgggatgaaaggcgagcgccggaggggcaaggggcacgatggcctttaccagggtctcagtacagccaccaaggacacctacgacgcccttcacatgcaggccctgccccctcgctgataa

SEQ ID NO: 252 - DNA, 23 bp, Artificial Sequence
  137P2F primer
gtccttctcctgtcactggttat

SEQ ID NO: 253 - DNA, 23 bp, Artificial Sequence
  137P2R primer
tcttcttcttctggaaatcggca

SEQ ID NO: 254 - DNA, 48 bp, Artificial Sequence
  Linker sequence 3
ggcggcggcagcggcggcggcagcggcggcggcagcggcggcggcagc

SEQ ID NO: 255 - protein, 21 aa, Artificial Sequence
  T2A
GSGEGRGSLLTCGDVEENPGP

SEQ ID NO: 256 - DNA, 63 bp, Artificial Sequence
  T2A
ggcagtggagagggcagaggaagtctgctaacatgcggtgacgtcgaggagaatcctggccca

SEQ ID NO: 257 - protein, 376 aa, Artificial Sequence
  GSI5011 CAR 269A37346
MALPVTALLLPLALLLHAARPVNRTRRMHQVQLVESGGGLVQPGGSLRLSCEASGFTLDYYAIGWFRQAPGKEREGVICISRSDGSTYYADSVKGRFTISRDNAKKTVYLQMISLKPEDTAAYYCAAGADCSGYLRDYEFRGQGTQVTVSSTSTTTPAPRPPTPAPTIASQPLSLRPEACRPAAGGAVHTRGLDFACDIYIWAPLAGTCGVLLLSLVITLYCKRGRKKLLYIFKQPFMRPVQTTQEEDGCSCRFPEEEEGGCELRVKFSRSADAPAYQQGQNQLYNELNLGRREEYDVLDKRRGRDPEMGGKPRRKNPQEGLYNELQKDKMAEAYSEIGMKGERRRGKGHDGLYQGLSTATKDTYDALHMQALPPR

SEQ ID NO: 258 - protein, 373 aa, Artificial Sequence
  GSI5019 CAR 269A37353
MALPVTALLLPLALLLHAARPVNRTRRMHQVKLEESGGGLVQAGRSLRLSCAASEHTFSSHVMGWFRQAPGKERESVAVIGWRDISTSYADSVKGRFTISRDNAKKTLYLQMNSLKPEDTAVYYCAARRIDAADFDSWGQGTQVTVSSTSTTTPAPRPPTPAPTIASQPLSLRPEACRPAAGGAVHTRGLDFACDIYIWAPLAGTCGVLLLSLVITLYCKRGRKKLLYIFKQPFMRPVQTTQEEDGCSCRFPEEEEGGCELRVKFSRSADAPAYQQGQNQLYNELNLGRREEYDVLDKRRGRDPEMGGKPRRKNPQEGLYNELQKDKMAEAYSEIGMKGERRRGKGHDGLYQGLSTATKDTYDALHMQALPPR

SEQ ID NO: 259 - protein, 372 aa, Artificial Sequence
  GSI5020 CAR 269A37917
MALPVTALLLPLALLLHAARPVNRTRRMHEVQLVESGGGLVQAGGSLRLSCAASGRTFTMGWFRQAPGKEREFVAAISLSPTLAYYAESVKGRFTISRDNAKNTVVLQMNSLKPEDTALYYCAADRKSVMSIRPDYWGQGTQVTVSSTSTTTPAPRPPTPAPTIASQPLSLRPEACRPAAGGAVHTRGLDFACDIYIWAPLAGTCGVLLLSLVITLYCKRGRKKLLYIFKQPFMRPVQTTQEEDGCSCRFPEEEEGGCELRVKFSRSADAPAYQQGQNQLYNELNLGRREEYDVLDKRRGRDPEMGGKPRRKNPQEGLYNELQKDKMAEAYSEIGMKGERRRGKGHDGLYQGLSTATKDTYDALHMQALPPR

SEQ ID NO: 260 - protein, 369 aa, Artificial Sequence
  GSI5012 CAR 38A37717
MALPVTALLLPLALLLHAARPVNEVQLVESGGGLVQAGGSLRLSCIATGKVFSIYDMGWYRQAPGKQRELVAEITSSGTTHYDDFVSGRFTISRDNAKNTVYLQMNTLKAEDTAVYYCRANHVFGGSYWGQGTQVTVSSTRRMHTSTTTPAPRPPTPAPTIASQPLSLRPEACRPAAGGAVHTRGLDFACDIYIWAPLAGTCGVLLLSLVITLYCKRGRKKLLYIFKQPFMRPVQTTQEEDGCSCRFPEEEEGGCELRVKFSRSADAPAYQQGQNQLYNELNLGRREEYDVLDKRRGRDPEMGGKPRRKNPQEGLYNELQKDKMAEAYSEIGMKGERRRGKGHDGLYQGLSTATKDTYDALHMQALPPR

SEQ ID NO: 261 - DNA, 1131 bp, Artificial Sequence
  GSI5011 CAR 269A37346
atggccttaccagtgaccgccttgctcctgccgctggccttgctgctccacgccgccaggccggttaaccgcacgcgtcgcatgcatcaggtgcagctggtggagtctgggggaggcttggtgcagcctgggggttctctgaggctctcctgtgaagcctctggattcactttggattattatgccataggctggttccgccaggccccagggaaggagcgcgagggggtcatatgtattagtagaagtgatggtagcacatactatgcagactccgtgaagggccgattcaccatctccagagacaacgccaagaaaacggtgtatctgcaaatgatcagcctgaaacctgaggacacggccgcttattactgtgcagcaggggccgattgttcggggtacctacgagattatgagttccgggggcaggggacccaggtcaccgtctcctcaactagtaccacgacgccagcgccgcgaccaccaacaccggcgcccaccatcgcgtcgcagcccctgtccctgcgcccagaggcgtgccggccagcggcggggggcgcagtgcacacgagggggctggacttcgcctgtgatatctacatctgggcgcccttggccgggacttgtggggtccttctcctgtcactggttatcaccctttactgcaaacggggcagaaagaaactcctgtatatattcaaacaaccatttatgagaccagtacaaactactcaagaggaagatggctgtagctgccgatttccagaagaagaagaaggaggatgtgaactgagagtgaagttcagcaggagcgcagacgcccccgcgtaccagcagggccagaaccagctctataacgagctcaatctaggacgaagagaggagtacgatgttttggacaagagacgtggccgggaccctgagatggggggaaagccgagaaggaagaaccctcaggaaggcctgtacaatgaactgcagaaagataagatggcggaggcctacagtgagattgggatgaaaggcgagcgccggaggggcaaggggcacgatggcctttaccagggtctcagtacagccaccaaggacacctacgacgcccttcacatgcaggccctgccccctcgctaa

SEQ ID NO: 262 - DNA, 1122 bp, Artificial Sequence
  GSI5019 CAR 269A37353
atggccttaccagtgaccgccttgctcctgccgctggccttgctgctccacgccgccaggccggttaaccgcacgcgtcgcatgcatcaggtaaagctggaggagtctgggggaggcttggtgcaggctgggcggtctctgagactctcctgtgcagcctctgaacacaccttcagtagccatgtcatgggctggttccgccaggctccagggaaggagcgtgagtctgttgcagttattggctggagagatattagcacaagctatgcagactccgtgaagggccgattcaccatctccagagacaacgccaagaagacgctgtatctgcaaatgaatagcctgaaacctgaggacacggccgtttactactgtgcagcacgtcggatcgacgcagctgactttgattcctgggggcaggggacccaggtcaccgtctcctcgactagtaccacgacgccagcgccgcgaccaccaacaccggcgcccaccatcgcgtcgcagcccctgtccctgcgcccagaggcgtgccggccagcggcggggggcgcagtgcacacgagggggctggacttcgcctgtgatatctacatctgggcgcccttggccgggacttgtggggtccttctcctgtcactggttatcaccctttactgcaaacggggcagaaagaaactcctgtatatattcaaacaaccatttatgagaccagtacaaactactcaagaggaagatggctgtagctgccgatttccagaagaagaagaaggaggatgtgaactgagagtgaagttcagcaggagcgcagacgcccccgcgtaccagcagggccagaaccagctctataacgagctcaatctaggacgaagagaggagtacgatgttttggacaagagacgtggccgggaccctgagatggggggaaagccgagaaggaagaaccctcaggaaggcctgtacaatgaactgcagaaagataagatggcggaggcctacagtgagattgggatgaaaggcgagcgccggaggggcaaggggcacgatggcctttaccagggtctcagtacagccaccaaggacacctacgacgcccttcacatgcaggccctgccccctcgctaa

SEQ ID NO: 263 - DNA, 1119 bp, Artificial Sequence
  GSI5020 CAR 269A37917
atggccttaccagtgaccgccttgctcctgccgctggccttgctgctccacgccgccaggccggttaaccgcacgcgtcgcatgcatgaggtgcagctggtggagtctgggggaggcttggtgcaggctggggggtctctgagactctcctgtgcagcctctggacgcaccttcaccatggggtggttccgtcaggctccagggaaggagcgtgagtttgtagcagctattagtttgagtcctactttagcatattatgcagagtccgtgaagggccgattcaccatcagccgagacaacgccaagaacacggtggttttgcaaatgaacagcctgaaacctgaggacacggccctttattactgtgcagcagaccggaaatcagtaatgtctattcggcccgactactggggccaggggacccaggtcaccgtctcctcaactagtaccacgacgccagcgccgcgaccaccaacaccggcgcccaccatcgcgtcgcagcccctgtccctgcgcccagaggcgtgccggccagcggcggggggcgcagtgcacacgagggggctggacttcgcctgtgatatctacatctgggcgcccttggccgggacttgtggggtccttctcctgtcactggttatcaccctttactgcaaacggggcagaaagaaactcctgtatatattcaaacaaccatttatgagaccagtacaaactactcaagaggaagatggctgtagctgccgatttccagaagaagaagaaggaggatgtgaactgagagtgaagttcagcaggagcgcagacgcccccgcgtaccagcagggccagaaccagctctataacgagctcaatctaggacgaagagaggagtacgatgttttggacaagagacgtggccgggaccctgagatggggggaaagccgagaaggaagaaccctcaggaaggcctgtacaatgaactgcagaaagataagatggcggaggcctacagtgagattgggatgaaaggcgagcgccggaggggcaaggggcacgatggcctttaccagggtctcagtacagccaccaaggacacctacgacgcccttcacatgcaggccctgccccctcgctaa

SEQ ID NO: 264 - DNA, 1110 bp, Artificial Sequence
  GSI5012 CAR 38A37717
atggccttaccagtgaccgccttgctcctgccgctggccttgctgctccacgccgccaggccggttaacgaggtgcagctggtggaaagcggggggggactggtgcaggcaggcgggtcactgagactgtcatgtatcgcaactgggaaggtgtttagcatctacgacatgggctggtataggcaggcaccaggaaagcagagggagctggtggccgagatcaccagctccggcaccacacactacgacgatttcgtgtctggccggtttaccatcagcagagacaacgccaagaatacagtgtatctgcagatgaacaccctgaaggccgaggatacagccgtgtactattgccgggctaatcacgtcttcggcggctcctactgggggcagggaactcaggtcactgtgtcatccacgcgtcgcatgcatactagtaccacgacgccagcgccgcgaccaccaacaccggcgcccaccatcgcgtcgcagcccctgtccctgcgcccagaggcgtgccggccagcggcggggggcgcagtgcacacgagggggctggacttcgcctgtgatatctacatctgggcgcccttggccgggacttgtggggtccttctcctgtcactggttatcaccctttactgcaaacggggcagaaagaaactcctgtatatattcaaacaaccatttatgagaccagtacaaactactcaagaggaagatggctgtagctgccgatttccagaagaagaagaaggaggatgtgaactgagagtgaagttcagcaggagcgcagacgcccccgcgtaccagcagggccagaaccagctctataacgagctcaatctaggacgaagagaggagtacgatgttttggacaagagacgtggccgggaccctgagatggggggaaagccgagaaggaagaaccctcaggaaggcctgtacaatgaactgcagaaagataagatggcggaggcctacagtgagattgggatgaaaggcgagcgccggaggggcaaggggcacgatggcctttaccagggtctcagtacagccaccaaggacacctacgacgcccttcacatgcaggccctgccccctcgctaa

SEQ ID NO: 265 - protein, 488 aa, Artificial Sequence
  GSI5021 CAR
MALPVTALLLPLALLLHAARPQVKLEESGGGLVQAGRSLRLSCAASEHTFSSHVMGWFRQAPGKERESVAVIGWRDISTSYADSVKGRFTISRDNAKKTLYLQMNSLKPEDTAVYYCAARRIDAADFDSWGQGTQVTVSSGGGGSEVQLVESGGGLVQAGGSLRLSCAASGRTFTMGWFRQAPGKEREFVAAISLSPTLAYYAESVKGRFTISRDNAKNTVVLQMNSLKPEDTALYYCAADRKSVMSIRPDYWGQGTQVTVSSTSTTTPAPRPPTPAPTIASQPLSLRPEACRPAAGGAVHTRGLDFACDIYIWAPLAGTCGVLLLSLVITLYCKRGRKKLLYIFKQPFMRPVQTTQEEDGCSCRFPEEEEGGCELRVKFSRSADAPAYQQGQNQLYNELNLGRREEYDVLDKRRGRDPEMGGKPRRKNPQEGLYNELQKDKMAEAYSEIGMKGERRRGKGHDGLYQGLSTATKDTYDALHMQALPPR

SEQ ID NO: 266 - protein, 498 aa, Artificial Sequence
  GSI5022 CAR
MALPVTALLLPLALLLHAARPQVKLEESGGGLVQAGRSLRLSCAASEHTFSSHVMGWFRQAPGKERESVAVIGWRDISTSYADSVKGRFTISRDNAKKTLYLQMNSLKPEDTAVYYCAARRIDAADFDSWGQGTQVTVSSGGGGSGGGGSGGGGSEVQLVESGGGLVQAGGSLRLSCAASGRTFTMGWFRQAPGKEREFVAAISLSPTLAYYAESVKGRFTISRDNAKNTVVLQMNSLKPEDTALYYCAADRKSVMSIRPDYWGQGTQVTVSSTSTTTPAPRPPTPAPTIASQPLSLRPEACRPAAGGAVHTRGLDFACDIYIWAPLAGTCGVLLLSLVITLYCKRGRKKLLYIFKQPFMRPVQTTQEEDGCSCRFPEEEEGGCELRVKFSRSADAPAYQQGQNQLYNELNLGRREEYDVLDKRRGRDPEMGGKPRRKNPQEGLYNELQKDKMAEAYSEIGMKGERRRGKGHDGLYQGLSTATKDTYDALHMQALPPR

SEQ ID NO: 267 - protein, 508 aa, Artificial Sequence
  GSI5023 CAR
MALPVTALLLPLALLLHAARPQVKLEESGGGLVQAGRSLRLSCAASEHTFSSHVMGWFRQAPGKERESVAVIGWRDISTSYADSVKGRFTISRDNAKKTLYLQMNSLKPEDTAVYYCAARRIDAADFDSWGQGTQVTVSSGGGGSGGGGSGGGGSGGGGSGGGGSEVQLVESGGGLVQAGGSLRLSCAASGRTFTMGWFRQAPGKEREFVAAISLSPTLAYYAESVKGRFTISRDNAKNTVVLQMNSLKPEDTALYYCAADRKSVMSIRPDYWGQGTQVTVSSTSTTTPAPRPPTPAPTIASQPLSLRPEACRPAAGGAVHTRGLDFACDIYIWAPLAGTCGVLLLSLVITLYCKRGRKKLLYIFKQPFMRPVQTTQEEDGCSCRFPEEEEGGCELRVKFSRSADAPAYQQGQNQLYNELNLGRREEYDVLDKRRGRDPEMGGKPRRKNPQEGLYNELQKDKMAEAYSEIGMKGERRRGKGHDGLYQGLSTATKDTYDALHMQALPPR

SEQ ID NO: 268 - protein, 493 aa, Artificial Sequence
  GSI5024 CAR
MALPVTALLLPLALLLHAARPEVQLVESGGGLVQAGGSLRLSCAASGRTFTMGWFRQAPGKEREFVAAISLSPTLAYYAESVKGRFTISRDNAKNTVVLQMNSLKPEDTALYYCAADRKSVMSIRPDYWGQGTQVTVSSGGGGSGGGGSQVKLEESGGGLVQAGRSLRLSCAASEHTFSSHVMGWFRQAPGKERESVAVIGWRDISTSYADSVKGRFTISRDNAKKTLYLQMNSLKPEDTAVYYCAARRIDAADFDSWGQGTQVTVSSTSTTTPAPRPPTPAPTIASQPLSLRPEACRPAAGGAVHTRGLDFACDIYIWAPLAGTCGVLLLSLVITLYCKRGRKKLLYIFKQPFMRPVQTTQEEDGCSCRFPEEEEGGCELRVKFSRSADAPAYQQGQNQLYNELNLGRREEYDVLDKRRGRDPEMGGKPRRKNPQEGLYNELQKDKMAEAYSEIGMKGERRRGKGHDGLYQGLSTATKDTYDALHMQALPPR

SEQ ID NO: 269 - protein, 498 aa, Artificial Sequence
  GSI5025 CAR
MALPVTALLLPLALLLHAARPEVQLVESGGGLVQAGGSLRLSCAASGRTFTMGWFRQAPGKEREFVAAISLSPTLAYYAESVKGRFTISRDNAKNTVVLQMNSLKPEDTALYYCAADRKSVMSIRPDYWGQGTQVTVSSGGGGSGGGGSGGGGSQVKLEESGGGLVQAGRSLRLSCAASEHTFSSHVMGWFRQAPGKERESVAVIGWRDISTSYADSVKGRFTISRDNAKKTLYLQMNSLKPEDTAVYYCAARRIDAADFDSWGQGTQVTVSSTSTTTPAPRPPTPAPTIASQPLSLRPEACRPAAGGAVHTRGLDFACDIYIWAPLAGTCGVLLLSLVITLYCKRGRKKLLYIFKQPFMRPVQTTQEEDGCSCRFPEEEEGGCELRVKFSRSADAPAYQQGQNQLYNELNLGRREEYDVLDKRRGRDPEMGGKPRRKNPQEGLYNELQKDKMAEAYSEIGMKGERRRGKGHDGLYQGLSTATKDTYDALHMQALPPR

SEQ ID NO: 270 - protein, 503 aa, Artificial Sequence
  GSI5026 CAR
MALPVTALLLPLALLLHAARPEVQLVESGGGLVQAGGSLRLSCAASGRTFTMGWFRQAPGKEREFVAAISLSPTLAYYAESVKGRFTISRDNAKNTVVLQMNSLKPEDTALYYCAADRKSVMSIRPDYWGQGTQVTVSSGGGGSGGGGSGGGGSGGGGSQVKLEESGGGLVQAGRSLRLSCAASEHTFSSHVMGWFRQAPGKERESVAVIGWRDISTSYADSVKGRFTISRDNAKKTLYLQMNSLKPEDTAVYYCAARRIDAADFDSWGQGTQVTVSSTSTTTPAPRPPTPAPTIASQPLSLRPEACRPAAGGAVHTRGLDFACDIYIWAPLAGTCGVLLLSLVITLYCKRGRKKLLYIFKQPFMRPVQTTQEEDGCSCRFPEEEEGGCELRVKFSRSADAPAYQQGQNQLYNELNLGRREEYDVLDKRRGRDPEMGGKPRRKNPQEGLYNELQKDKMAEAYSEIGMKGERRRGKGHDGLYQGLSTATKDTYDALHMQALPPR

SEQ ID NO: 271 - DNA, 1467 bp, Artificial Sequence
  GSI5021 CAR
atggctctgcccgtcaccgctctgctgctgcctctggctctgctgctgcacgctgctcgccctcaggtcaaactggaagaatctggcggaggcctggtgcaggcaggacggagcctgcgcctgagctgcgcagcatccgagcacaccttcagctcccacgtgatgggctggtttcggcaggccccaggcaaggagagagagagcgtggccgtgatcggctggagggacatctccacatcttacgccgattccgtgaagggccggttcaccatcagccgggacaacgccaagaagacactgtatctgcagatgaacagcctgaagcccgaggacaccgccgtgtactattgcgcagcaaggagaatcgacgcagcagactttgattcctggggccagggcacccaggtgacagtgtctagcggaggaggaggatctgaggtgcagctggtggagagcggaggcggcctggtgcaggccggaggctctctgaggctgagctgtgcagcatccggaagaaccttcacaatgggctggtttaggcaggcaccaggaaaggagagggagttcgtggcagcaatcagcctgtcccctaccctggcctactatgccgagagcgtgaagggcaggtttaccatctcccgcgataacgccaagaatacagtggtgctgcagatgaactccctgaaacctgaggacacagccctgtactattgtgccgccgatcggaagagcgtgatgagcattagaccagactattgggggcagggaacacaggtgaccgtgagcagcactagtaccacgacgccagcgccgcgaccaccaacaccggcgcccaccatcgcgtcgcagcccctgtccctgcgcccagaggcgtgccggccagcggcggggggcgcagtgcacacgagggggctggacttcgcctgtgatatctacatctgggcgcccttggccgggacttgtggggtccttctcctgtcactggttatcaccctttactgcaaacggggcagaaagaaactcctgtatatattcaaacaaccatttatgagaccagtacaaactactcaagaggaagatggctgtagctgccgatttccagaagaagaagaaggaggatgtgaactgagagtgaagttcagcaggagcgcagacgcccccgcgtaccagcagggccagaaccagctctataacgagctcaatctaggacgaagagaggagtacgatgttttggacaagagacgtggccgggaccctgagatggggggaaagccgagaaggaagaaccctcaggaaggcctgtacaatgaactgcagaaagataagatggcggaggcctacagtgagattgggatgaaaggcgagcgccggaggggcaaggggcacgatggcctttaccagggtctcagtacagccaccaaggacacctacgacgcccttcacatgcaggccctgccccctcgctaa

SEQ ID NO: 272 - DNA, 1497 bp, Artificial Sequence
  GSI5022 CAR
atggctctgcctgtcaccgctctgctgctgcctctggctctgctgctgcacgctgctcgccctcaggtcaaactggaagaaagtgggggaggcctggtgcaggcaggacggagcctgcgcctgagctgcgcagcatccgagcacaccttcagctcccacgtgatgggctggtttcggcaggccccaggcaaggagagagagtccgtggccgtgatcggctggagggacatctccacatcttacgccgattctgtgaagggccggttcaccatcagcagagacaacgccaagaagacactgtatctgcagatgaatagcctgaagcccgaggacaccgccgtgtactattgcgcagcaaggagaatcgacgcagcagactttgattcctggggccagggcacccaggtgacagtgtctagcggaggaggaggatctggaggaggaggaagcggaggaggaggatccgaggtgcagctggtggagtctggaggcggcctggtgcaggccggaggctctctgaggctgagctgtgcagcatccggaagaaccttcacaatgggctggtttaggcaggcaccaggaaaggagagggagttcgtggcagcaatcagcctgtcccctaccctggcctactatgccgagtccgtgaagggcaggtttaccatctctcgcgataacgccaagaatacagtggtgctgcagatgaacagcctgaaacctgaggacacagccctgtactattgtgccgccgatcggaagagcgtgatgagcattagacccgattattggggacagggcacacaggtgacagtgagtagcactagtaccacgacgccagcgccgcgaccaccaacaccggcgcccaccatcgcgtcgcagcccctgtccctgcgcccagaggcgtgccggccagcggcggggggcgcagtgcacacgagggggctggacttcgcctgtgatatctacatctgggcgcccttggccgggacttgtggggtccttctcctgtcactggttatcaccctttactgcaaacggggcagaaagaaactcctgtatatattcaaacaaccatttatgagaccagtacaaactactcaagaggaagatggctgtagctgccgatttccagaagaagaagaaggaggatgtgaactgagagtgaagttcagcaggagcgcagacgcccccgcgtaccagcagggccagaaccagctctataacgagctcaatctaggacgaagagaggagtacgatgttttggacaagagacgtggccgggaccctgagatggggggaaagccgagaaggaagaaccctcaggaaggcctgtacaatgaactgcagaaagataagatggcggaggcctacagtgagattgggatgaaaggcgagcgccggaggggcaaggggcacgatggcctttaccagggtctcagtacagccaccaaggacacctacgacgcccttcacatgcaggccctgccccctcgctaa

SEQ ID NO: 273 - DNA, 1527 bp, Artificial Sequence
  GSI5023 CAR
atggctctgcccgtcaccgcactgctgctgcctctggctctgctgctgcacgccgcaagaccacaggtcaaactggaagaatcaggaggaggcctggtgcaggcaggacggagcctgcgcctgagctgcgcagcatccgagcacaccttcagctcccacgtgatgggctggtttcggcaggccccaggcaaggagagagagtccgtggccgtgatcggctggagggacatctccacatcttacgccgattccgtgaagggccggttcaccatcagccgggacaacgccaagaagacactgtatctgcagatgaacagcctgaagcccgaggacaccgccgtgtactattgcgcagcaaggagaatcgacgcagcagactttgatagctggggccagggcacccaggtgacagtgtctagcggaggaggaggatctggaggaggaggaagcggaggaggaggaagcggcggcggcggctctggcggcggcggcagcgaggtgcagctggtggagagcggcggcggcctggtgcaggccggcggctctctgaggctgagctgtgcagcatccggaagaaccttcacaatgggctggtttaggcaggcaccaggaaaggagagggagttcgtggcagcaatcagcctgtcccctaccctggcctactatgccgagagcgtgaagggcaggtttaccatctcccgcgataacgccaagaatacagtggtgttacaaatgaacagcctgaaacctgaggacacagccctgtactattgtgccgccgatcggaagagcgtgatgagcattagacccgattattgggggcaggggacacaggtgaccgtgagcagcactagtaccacgacgccagcgccgcgaccaccaacaccggcgcccaccatcgcgtcgcagcccctgtccctgcgcccagaggcgtgccggccagcggcggggggcgcagtgcacacgagggggctggacttcgcctgtgatatctacatctgggcgcccttggccgggacttgtggggtccttctcctgtcactggttatcaccctttactgcaaacggggcagaaagaaactcctgtatatattcaaacaaccatttatgagaccagtacaaactactcaagaggaagatggctgtagctgccgatttccagaagaagaagaaggaggatgtgaactgagagtgaagttcagcaggagcgcagacgcccccgcgtaccagcagggccagaaccagctctataacgagctcaatctaggacgaagagaggagtacgatgttttggacaagagacgtggccgggaccctgagatggggggaaagccgagaaggaagaaccctcaggaaggcctgtacaatgaactgcagaaagataagatggcggaggcctacagtgagattgggatgaaaggcgagcgccggaggggcaaggggcacgatggcctttaccagggtctcagtacagccaccaaggacacctacgacgcccttcacatgcaggccctgccccctcgctaa

SEQ ID NO: 274 - DNA, 1482 bp, Artificial Sequence
  GSI5024 CAR
atggctctgcctgtgaccgcactgctgctgcctctggctctgctgctgcacgccgcacgacctgaagtccagctggtggaatccgggggaggcctggtgcaggcaggaggctccctgaggctgtcttgcgcagcaagcggaagaaccttcacaatgggctggtttaggcaggcaccaggaaaggagagggagttcgtggccgccatctccctgtctcctaccctggcctactatgccgagagcgtgaagggcaggtttaccatctcccgcgacaacgccaagaatacagtggtgctgcagatgaacagcctgaagccagaggacacagccctgtactattgcgccgccgatcggaagtctgtgatgagcatcagacccgattactggggccagggcacccaggtgacagtgagctccggaggaggaggatccggcggaggaggctctcaggtgaagctggaggagtccggaggcggcctggtgcaggccggacggtccctgagactgtcttgtgccgccagcgagcacaccttctctagccacgtgatgggatggttcaggcaggcacctggaaaggagagggagtccgtggcagtgatcggatggagggacatcagcacatcctacgccgattctgtgaagggccggttcaccatcagcagagacaacgccaagaagacactgtatttacaaatgaacagcctgaagcccgaggataccgccgtgtactattgtgccgcccggcggattgacgccgcagactttgactcatgggggcagggaactcaggtgaccgtgtcctcaactagtaccacgacgccagcgccgcgaccaccaacaccggcgcccaccatcgcgtcgcagcccctgtccctgcgcccagaggcgtgccggccagcggcggggggcgcagtgcacacgagggggctggacttcgcctgtgatatctacatctgggcgcccttggccgggacttgtggggtccttctcctgtcactggttatcaccctttactgcaaacggggcagaaagaaactcctgtatatattcaaacaaccatttatgagaccagtacaaactactcaagaggaagatggctgtagctgccgatttccagaagaagaagaaggaggatgtgaactgagagtgaagttcagcaggagcgcagacgcccccgcgtaccagcagggccagaaccagctctataacgagctcaatctaggacgaagagaggagtacgatgttttggacaagagacgtggccgggaccctgagatggggggaaagccgagaaggaagaaccctcaggaaggcctgtacaatgaactgcagaaagataagatggcggaggcctacagtgagattgggatgaaaggcgagcgccggaggggcaaggggcacgatggcctttaccagggtctcagtacagccaccaaggacacctacgacgcccttcacatgcaggccctgccccctcgctaa

SEQ ID NO: 275 - DNA, 1497 bp, Artificial Sequence
  GSI5025 CAR
atggccctgcctgtcaccgctctgctgctgcccctggccctgctgctgcacgccgcacgccctgaggtccagctggtcgagtccgggggaggcctggtgcaggcaggaggctccctgaggctgtcttgcgcagcaagcggaagaaccttcacaatgggctggtttaggcaggcaccaggaaaggagagggagttcgtggccgccatctccctgtctcctaccctggcctactatgccgagtccgtgaagggcaggtttaccatctctcgcgacaacgccaagaatacagtggtgctgcagatgaactccctgaagccagaggacacagccctgtactattgcgccgccgatcggaagtctgtgatgagcatcagacccgattactggggccagggcacccaggtgacagtgagctccggaggaggaggatccggcggaggaggctctggcggcggcggcagccaggtgaagctggaggagagcggaggcggcctggtgcaggccggacggtccctgagactgtcttgtgccgccagcgagcacaccttctctagccacgtgatgggatggttcaggcaggcacctggaaaggagagggagtctgtggccgtgatcggctggagggacatcagcacatcctacgccgatagcgtgaagggccggttcaccatctccagagacaacgccaagaagacactgtatctgcagatgaatagcctgaagcccgaggataccgccgtgtactattgtgccgcccggcggattgacgccgcagattttgattcttgggggcagggaactcaggtgaccgtgtcctcaactagtaccacgacgccagcgccgcgaccaccaacaccggcgcccaccatcgcgtcgcagcccctgtccctgcgcccagaggcgtgccggccagcggcggggggcgcagtgcacacgagggggctggacttcgcctgtgatatctacatctgggcgcccttggccgggacttgtggggtccttctcctgtcactggttatcaccctttactgcaaacggggcagaaagaaactcctgtatatattcaaacaaccatttatgagaccagtacaaactactcaagaggaagatggctgtagctgccgatttccagaagaagaagaaggaggatgtgaactgagagtgaagttcagcaggagcgcagacgcccccgcgtaccagcagggccagaaccagctctataacgagctcaatctaggacgaagagaggagtacgatgttttggacaagagacgtggccgggaccctgagatggggggaaagccgagaaggaagaaccctcaggaaggcctgtacaatgaactgcagaaagataagatggcggaggcctacagtgagattgggatgaaaggcgagcgccggaggggcaaggggcacgatggcctttaccagggtctcagtacagccaccaaggacacctacgacgcccttcacatgcaggccctgccccctcgctaa

SEQ ID NO: 276 - DNA, 1512 bp, Artificial Sequence
  GSI5026 CAR
atggctctgcctgtgaccgccctgctgctgcccctggccctgctgctgcacgccgcacgacctgaagtccagctggtggaatctggcggaggcctggtgcaggcaggaggctccctgaggctgtcttgcgcagcaagcggaagaaccttcacaatgggctggtttaggcaggcaccaggaaaggagagggagttcgtggccgccatctccctgtctcctaccctggcctactatgccgagtctgtgaagggcaggtttaccatcagccgcgacaacgccaagaatacagtggtgctgcagatgaacagcctgaagccagaggacacagccctgtactattgcgccgccgatcggaagtctgtgatgagcatcagacccgattactggggccagggcacccaggtgacagtgagctccggaggaggaggatccggcggaggaggctctggcggcggcggctccggcggcggcggctcccaggtgaagctggaggagtccggaggcggcctggtgcaggccggacggtccctgagactgtcttgtgccgccagcgagcacaccttctctagccacgtgatgggatggttcaggcaggcacctggaaaggagagggagagcgtggcagtgatcggatggagggacatcagcacatcctacgccgattccgtgaagggccggttcaccatcagccgggacaacgccaagaagacactgtatttacaaatgaacagcctgaagcccgaggataccgccgtgtactattgtgccgcccggcggattgatgccgcagactttgatagttggggacaggggactcaggtcaccgtcagcagcactagtaccacgacgccagcgccgcgaccaccaacaccggcgcccaccatcgcgtcgcagcccctgtccctgcgcccagaggcgtgccggccagcggcggggggcgcagtgcacacgagggggctggacttcgcctgtgatatctacatctgggcgcccttggccgggacttgtggggtccttctcctgtcactggttatcaccctttactgcaaacggggcagaaagaaactcctgtatatattcaaacaaccatttatgagaccagtacaaactactcaagaggaagatggctgtagctgccgatttccagaagaagaagaaggaggatgtgaactgagagtgaagttcagcaggagcgcagacgcccccgcgtaccagcagggccagaaccagctctataacgagctcaatctaggacgaagagaggagtacgatgttttggacaagagacgtggccgggaccctgagatggggggaaagccgagaaggaagaaccctcaggaaggcctgtacaatgaactgcagaaagataagatggcggaggcctacagtgagattgggatgaaaggcgagcgccggaggggcaaggggcacgatggcctttaccagggtctcagtacagccaccaaggacacctacgacgcccttcacatgcaggccctgccccctcgctaa

SEQ ID NO: 277 - protein, 768 aa, Artificial Sequence
  tandem BCMA, CD38 269A37346 38A37717 GSI5013 CARs
MALPVTALLLPLALLLHAARPVNEVQLVESGGGLVQAGGSLRLSCIATGKVFSIYDMGWYRQAPGKQRELVAEITSSGTTHYDDFVSGRFTISRDNAKNTVYLQMNTLKAEDTAVYYCRANHVFGGSYWGQGTQVTVSSTRRMHTSTTTPAPRPPTPAPTIASQPLSLRPEACRPAAGGAVHTRGLDFACDIYIWAPLAGTCGVLLLSLVITLYCKRGRKKLLYIFKQPFMRPVQTTQEEDGCSCRFPEEEEGGCELRVKFSRSADAPAYQQGQNQLYNELNLGRREEYDVLDKRRGRDPEMGGKPRRKNPQEGLYNELQKDKMAEAYSEIGMKGERRRGKGHDGLYQGLSTATKDTYDALHMQALPPRGSGEGRGSLLTCGDVEENPGPGSMALPVTALLLPLALLLHAARPVNRTRRMHQVQLVESGGGLVQPGGSLRLSCEASGFTLDYYAIGWFRQAPGKEREGVICISRSDGSTYYADSVKGRFTISRDNAKKTVYLQMISLKPEDTAAYYCAAGADCSGYLRDYEFRGQGTQVTVSSTSTTTPAPRPPTPAPTIASQPLSLRPEACRPAAGGAVHTRGLDFACDIYIWAPLAGTCGVLLLSLVITLYCKRGRKKLLYIFKQPFMRPVQTTQEEDGCSCRFPEEEEGGCELRVKFSRSADAPAYQQGQNQLYNELNLGRREEYDVLDKRRGRDPEMGGKPRRKNPQEGLYNELQKDKMAEAYSEIGMKGERRRGKGHDGLYQGLSTATKDTYDALHMQALPPR